European Patent Specification EP 3 630 964 B1, published August 13, 2025. Title: THERAPEUTICS FOR GLYCOGEN STORAGE DISEASE TYPE III. Applicant: Ultragenyx Pharmaceutical Inc. Tachikawa, Kiyoshi Perez-Garcia, Carlos Gustavo Chivukula, Padmanabh Bhaskaran, Hari Prakash Cobaugh, Christian W. Daugherty, Sean Christopher. The sequence listing filed with the application follows.

SEQUENCE LISTING (45 sequences)

SEQ ID NO: 1 - RNA, 4599 nt, Artificial Sequence
  Consensus Human AGL Coding Sequence
augggacacaguaaacagauucgaauuuuacuucugaacgaaauggagaaacuggaaaagacccucuucagacuugaacaaggguaugagcuacaguuccgauuaggcccaacuuuacagggaaaagcaguuaccguguauacaaauuacccauuuccuggagaaacauuuaauagagaaaaauuccguucucuggauugggaaaauccaacagaaagagaagaugauucugauaaauacuguaaacuuaaucugcaacaaucugguucauuucaguauuauuuccuucaaggaaaugagaaaagugguggagguuacauaguuguggaccccauuuuacguguuggugcugauaaucaugugcuacccuuggacuguguuacucuucagacauuuuuagcuaaguguuugggaccuuuugaugaaugggaaagcagacuuaggguugcaaaagaaucaggcuacaacaugauucauuuuaccccauugcagacucuuggacuaucuaggucaugcuacucccuugccaaucaguuagaauuaaauccugacuuuucaagaccuaauagaaaguauaccuggaaugauguuggacagcuaguggaaaaauuaaaaaaggaauggaauguuauuuguauuacugauguugucuacaaucauacugcugcuaauaguaaauggauccaggaacauccagaaugugccuauaaucuugugaauucuccacacuuaaaaccugccugggucuuagacagagcacuuuggcguuucuccugugauguugcagaagggaaauacaaagaaaagggaauaccugcuuugauugaaaaugaucaccauaugaauuccauccgaaaaauaauuugggaggauauuuuuccaaagcuuaaacucugggaauuuuuccaaguagaugucaacaaagcgguugagcaauuuagaagacuucuuacacaagaaaauaggcgaguaaccaagucugauccaaaccaacaccuuacgauuauucaagauccugaauacagacgguuuggcuguacuguagauaugaacauugcacuaacgacuuucauaccacaugacaaggggccagcagcaauugaagaaugcuguaauugguuucauaaaagaauggaggaauuaaauucagagaagcaucgacucauuaacuaucaucaggaacaggcaguuaauugccuuuugggaaauguguuuuaugaacgacuggcuggccaugguccaaaacuaggaccugucacuagaaagcauccuuuaguuaccagguauuuuacuuucccauuugaagagauagacuucuccauggaagaaucuaugauucaucugccaaauaaagcuuguuuucugauggcacacaauggauggguaaugggagaugauccucuucgaaacuuugcugaaccggguucagaaguuuaccuaaggagagaacuuauuugcuggggagacaguguuaaauuacgcuaugggaauaaaccagaggacuguccuuaucucugggcacacaugaaaaaauacacugaaauaacugcaacuuauuuccagggaguacgucuugauaacugccacucaacaccucuucacguagcugaguacauguuggaugcugcuaggaauuugcaacccaauuuauauguaguagcugaacuguucacaggaagugaagaucuggacaaugucuuuguuacuagacugggcauuaguuccuuaauaagagaggcaaugagugcauauaauagucaugaagagggcagauuaguuuaccgauauggaggagaaccuguuggauccuuuguucagcccuguuugaggccuuuaaugccagcuauugcacaugcccuguuuauggauauuacgcaugauaaugaguguccuauugugcauagaucagcguaugaugcucuaccaaguacuacaauuguuucuauggcauguugugcuaguggaaguacaagaggcuaugaugaauuagugccucaucagauuucagugguuucugaagaacgguuuuacacuaaguggaauccugaagcauugccuucaaacacaggugaaguuaauuuccaaagcggcauuauugcagccaggugugcuaucaguaaacuucaucaggagcuuggagccaaggguuuuauucagguguauguggaucaaguugaugaagacauaguggcaguaacaagacacucaccuagcauccaucagucuguuguggcuguaucuagaacugcuuucaggaaucccaagacuucauuuuacagcaaggaagugccucaaaugugcaucccuggcaaaauugaagaaguaguucuugaagcuagaacuauugagagaaacacgaaaccuuauaggaaggaugagaauucaaucaauggaacaccagauaucacaguagaaauuagagaacauauucagcuuaaugaaaguaaaauuguuaaacaagcuggaguugccacaaaagggcccaaugaauauauucaagaaauagaauuugaaaacuugucuccaggaaguguuauuauauucagaguuagucuugauccacaugcacaagucgcuguuggaauucuucgaaaucaucugacacaauucaguccucacuuuaaaucuggcagccuagcuguugacaaugcagauccuauauuaaaaauuccuuuugcuucucuugccuccagauuaacuuuggcugagcuaaaucagauccuuuaccgaugugaaucagaagaaaaggaagaugguggagggugcuaugacauaccaaacuggucagcccuuaaauaugcaggucuucaagguuuaaugucuguauuggcagaaauaagaccaaagaaugacuuggggcauccuuuuuguaauaauuugagaucuggagauuggaugauugacuaugucaguaaccggcuuauuucacgaucaggaacuauugcugaaguugguaaaugguugcaggcuauguucuucuaccugaagcagaucccacguuaccuuaucccauguuacuuugaugcuauauuaauuggugcauauaccacucuucuggauacagcauggaagcagaugucaagcuuuguucagaaugguucaaccuuugugaaacaccuuucauuggguucaguucaacuguguggaguaggaaaauucccuucccugccaauucuuucaccugcccuaauggauguaccuuauagguuaaaugagaucacaaaagaaaaggagcaauguuguguuucucuagcugcaggcuuaccucauuuuucuucugguauuuuccgcugcuggggaagggauacuuuuauugcacuuagagguauacugcugauuacuggacgcuauguagaagccaggaauauuauuuuagcauuugcggguacccugaggcauggacucauuccuaaucuacugggugaaggaauuuaugccagauacaauugucgggaugcuguguggugguggcugcaguguauccaggauuacuguaaaaugguuccaaauggucuagacauucucaagugcccaguuuccagaauguauccuacagaugauucugcuccuuugccugcuggcacacuggaucagccauuguuugaagucauacaggaagcaaugcaaaaacacaugcagggcauacaguuccgagaaaggaaugcugguccccagauagaucgaaacaugaaggacgaagguuuuaauauaacugcaggaguugaugaagaaacaggauuuguuuauggaggaaaucguuucaauuguggcacauggauggauaaaaugggagaaagugacagagcuagaaacagaggaaucccagccacaccaagagaugggucugcuguggaaauugugggccugaguaaaucugcuguucgcugguugcuggaauuauccaaaaaaaauauuuucccuuaucaugaagucacaguaaaaagacauggaaaggcuauaaagguaucauaugaugaguggaacagaaaaauacaagacaacuuugaaaagcuauuucauguuuccgaagacccuucagauuuaaaugaaaagcauccaaaucugguucacaaacguggcauauacaaagauaguuauggagcuucaaguccuuggugugacuaucagcucaggccuaauuuuaccauagcaaugguuguggccccugagcucuuuacuacagaaaaagcauggaaagcuuuggagauugcagaaaaaaaauugcuugguccccuuggcaugaaaacuuuagauccagaugauaugguuuacuguggaauuuaugacaaugcauuagacaaugacaacuacaaucuugcuaaagguuucaauuaucaccaaggaccugaguggcuguggccuauuggguauuuucuucgugcaaaauuauauuuuuccagauugaugggcccggagacuacugcaaagacuauaguuuugguuaaaaauguucuuucccgacauuauguucaucuugagagauccccuuggaaaggacuuccagaacugaccaaugagaaugcccaguacuguccuuucagcugugaaacacaagccuggucaauugcuacuauucuugagacacuuuaugauuuauag

SEQ ID NO: 2 - protein, 1532 aa, Artificial Sequence
  Consensus Human AGL Amino Acid Sequence
MGHSKQIRILLLNEMEKLEKTLFRLEQGYELQFRLGPTLQGKAVTVYTNYPFPGETFNREKFRSLDWENPTEREDDSDKYCKLNLQQSGSFQYYFLQGNEKSGGGYIVVDPILRVGADNHVLPLDCVTLQTFLAKCLGPFDEWESRLRVAKESGYNMIHFTPLQTLGLSRSCYSLANQLELNPDFSRPNRKYTWNDVGQLVEKLKKEWNVICITDVVYNHTAANSKWIQEHPECAYNLVNSPHLKPAWVLDRALWRFSCDVAEGKYKEKGIPALIENDHHMNSIRKIIWEDIFPKLKLWEFFQVDVNKAVEQFRRLLTQENRRVTKSDPNQHLTIIQDPEYRRFGCTVDMNIALTTFIPHDKGPAAIEECCNWFHKRMEELNSEKHRLINYHQEQAVNCLLGNVFYERLAGHGPKLGPVTRKHPLVTRYFTFPFEEIDFSMEESMIHLPNKACFLMAHNGWVMGDDPLRNFAEPGSEVYLRRELICWGDSVKLRYGNKPEDCPYLWAHMKKYTEITATYFQGVRLDNCHSTPLHVAEYMLDAARNLQPNLYVVAELFTGSEDLDNVFVTRLGISSLIREAMSAYNSHEEGRLVYRYGGEPVGSFVQPCLRPLMPAIAHALFMDITHDNECPIVHRSAYDALPSTTIVSMACCASGSTRGYDELVPHQISVVSEERFYTKWNPEALPSNTGEVNFQSGIIAARCAISKLHQELGAKGFIQVYVDQVDEDIVAVTRHSPSIHQSVVAVSRTAFRNPKTSFYSKEVPQMCIPGKIEEVVLEARTIERNTKPYRKDENSINGTPDITVEIREHIQLNESKIVKQAGVATKGPNEYIQEIEFENLSPGSVIIFRVSLDPHAQVAVGILRNHLTQFSPHFKSGSLAVDNADPILKIPFASLASRLTLAELNQILYRCESEEKEDGGGCYDIPNWSALKYAGLQGLMSVLAEIRPKNDLGHPFCNNLRSGDWMIDYVSNRLISRSGTIAEVGKWLQAMFFYLKQIPRYLIPCYFDAILIGAYTTLLDTAWKQMSSFVQNGSTFVKHLSLGSVQLCGVGKFPSLPILSPALMDVPYRLNEITKEKEQCCVSLAAGLPHFSSGIFRCWGRDTFIALRGILLITGRYVEARNIILAFAGTLRHGLIPNLLGEGIYARYNCRDAVWWWLQCIQDYCKMVPNGLDILKCPVSRMYPTDDSAPLPAGTLDQPLFEVIQEAMQKHMQGIQFRERNAGPQIDRNMKDEGFNITAGVDEETGFVYGGNRFNCGTWMDKMGESDRARNRGIPATPRDGSAVEIVGLSKSAVRWLLELSKKNIFPYHEVTVKRHGKAIKVSYDEWNRKIQDNFEKLFHVSEDPSDLNEKHPNLVHKRGIYKDSYGASSPWCDYQLRPNFTIAMVVAPELFTTEKAWKALEIAEKKLLGPLGMKTLDPDDMVYCGIYDNALDNDNYNLAKGFNYHQGPEWLWPIGYFLRAKLYFSRLMGPETTAKTIVLVKNVLSRHYVHLERSPWKGLPELTNENAQYCPFSCETQAWSIATILETLYDL

SEQ ID NO: 3 - RNA, 129 nt, Tobacco Etch Virus
ucaacacaacauauacaaaacaaacgaaucucaagcaaucaagcauucuacuucuauugcagcaauuuaaaucauuucuuuuaaagcaaaagcaauuuucugaaaauuuucaccauuuacgaacgauag

SEQ ID NO: 4 - RNA, 6 nt, Unknown
  Kozak Sequence
gccacc

SEQ ID NO: 5 - RNA, 158 nt, Xenopus sp.
cuagugacugacuaggaucugguuaccacuaaaccagccucaagaacacccgaauggagucucuaagcuacauaauaccaacuuacacuuacaaaauguugucccccaaaauguagccauucguaucugcuccuaauaaaaagaaaguuucuucacau

SEQ ID NO: 6 - RNA, 114 nt, Unknown
  Poly(A) 114 Tail
aaaaaaaaaaaaaaaaaaaaaaaaaaaaaaaaaaaaaaaaaaaaaaaaaaaaaaaaaaaaaaaaaaaaaaaaaaaaaaaaaaaaaaaaaaaaaaaaaaaaaaaaaaaaaaaaaa

SEQ ID NO: 7 - RNA, 4599 nt, Artificial Sequence
  Codon-Optimized AGL Coding Sequence
augggacacuccaaacagauccggauacugcugcugaacgagauggaaaagcuggaaaagacucuauuccggcucgagcagggauacgagcugcaguuccgccugggccccacccuacaagggaaggccgugaccgucuacaccaacuacccuuucccgggcgaaacuuucaaccgggagaaguuccggucccuugacugggaaaacccgacugagcgcgaggacgacucggacaaauacugcaagcugaaccuccagcagucgggcucuuuccaauauuacuucuugcaagggaacgagaaguccgguggcggcuacaucgugguggacccaauuuugcgcgugggggcugacaaccacgugcugccacuggauugugugacccugcaaaccuuccuggccaagugccucggccccuucgacgaaugggagucgcgccugagaguggcgaaagagagcggauacaacaugauucacuucacgccgcuccaaacgcugggucugagccggucaugcuacucacuggcgaaccagcucgaacugaaccccgauuucucccggccaaacaggaaguacaccuggaacgacgugggacagcuggucgagaaguugaagaaggaguggaacgugaucuguaucaccgacgucguguacaaccacaccgcugcaaacucgaaguggauccaggaacauccggaaugugccuacaaccucgugaacagcccgcaccugaagccugccuggguguuggauagggcacuguggagguucuccugugacguggcagagggaaaguacaaggagaaggguauucccgcacucaucgaaaacgaucaccacaugaauucgaucagaaagauuaucugggaggauaucuucccuaagcugaagcugugggaguucuuucaaguugaugugaacaaggcagucgaacaguuucggcggcuguuaacccaagaaaaccgccgcgugaccaaguccgauccgaaucagcaucugaccauaauccaggacccggaauaccgccgguuuggcugcaccguggacaugaacauugcccugacuaccuuuaucccgcaugauaagggccccgccgcuaucgaagaaugcugcaacugguuccacaagaggauggaggaacugaacuccgaaaagcauaggcucauuaacuaccaccaggaacaggcagugaacugccugcuggggaacguguucuacgagcgacuggcuggacacggaccgaaguuaggacccgugacaaggaagcacccacuggucacuagauacuucaccuucccauuugaggaaaucgacuucucaauggaggagucgaugauccacuugccuaacaaggccugcuuucucauggcacauaacggaugggucaugggcgacgauccccuacggaauuuugcagaaccaggcagcgaggucuaccuucggcgggaacugauuugcuggggcgacuccgucaagcugcgcuacggcaacaagccugaggacugucccuaccuuugggcacacaugaagaaguacacugaaauuacugcgacauacuuccaaggaguccgcuuagauaauugucacuccaccccgcugcauguggcggaguacaugcuggaugccgcaagaaaccuccagccgaaucucuacgugguagcagagcuguucaccgggagcgaggaccuggacaauguguuugucacccggcuggggaucuccucccugauccgggaggccauguccgccuacaacucacacgaggaggggagacugguguaccgcuacggaggagaacccgugggcagcuuugugcagccuugccuccggccgcugaugcccgcgauugcgcaugcucuguucauggauaucacucacgauaacgagugccccauugugcacagauccgccuacgacgcccuuccuuccacaaccaucguguccauggcaugcugcgccuccggcuccacucgggguuacgaugagcuggugccacaccagauuuccgugguguccgaagaacgcuucuacaccaaguggaacccggaagcucugccgucaaacaccggagaagugaacuuccaguccgggaucaucgcagcgcgcugugcuauuagcaagcugcaccaggagcugggagccaagggguucauccaggucuauguggaccaggucgaugaggauaucgucgcugucacgagacacagcccgucuauccaucaaagcgucguggccgugucccggacugcguuccggaacccuaaaaccucauucuauuccaaagaggugccccagaugugcaucccuggaaagaucgaagaagucgugcuggaagcccggaccaucgagcggaacaccaagccguacaggaaggacgaaaacuccaucaaugguaccccugacauuaccguggaaaucagagaacauauccagcugaacgaguccaagaucgugaagcaggccggcguggcgaccaagggucccaacgaguacauucaggaaaucgaguuugaaaaccugucccccggaagcgugaucauuuuccgggugucccuggacccgcaugcgcaagucgcugucggaauucugcggaaucaccucacccaauucucgccgcauuucaagagugguucccuggcgguggauaaugccgauccgauccugaagauucccuucgcgucccuggcaucgagacucacccuggcggaguugaaccagauucuguaccgcugcgaauccgaggaaaaggaggacggaggcgguugcuacgacauccccaacugguccgcacuuaaguacgcagggcugcagggucuuaugagcgugcuggcagaaauucgcccuaagaacgauuugggacaccccuucugcaacaaccuccgguccggagacuggaugaucgauuacgugucgaacagacugauuucgagauccggcaccauugccgaggucggaaaguggcuucaggccauguucuucuaccugaagcagaucccgagauaccugauucccugcuacuucgacgcaauccugaucggggcguauaccacucuucuggacacugccuggaagcagauguccagcuucgugcaaaacggauccaccuucgucaagcaucuuagccugggcucagugcaguugugcggagugggaaaauucccuagccucccuauucuuucaccggcgcugauggacgugccuuaccgccugaacgaaaucaccaaagagaaggagcaguguugcgugucgcuggccgcgggucugccgcauuucuccuccggcaucuuccggugcuggggaagggacaccuucaucgcucugaggggaauccugcugauuaccgggcgcuacguggaagcucggaacaucauccuggccuucgcgggaacucugcgccacggccugauuccaaacuugcuuggcgaaggcaucuacgcgcgcuacaacugccgcgacgcggucuggugguggcuccagugcauucaagacuacugcaagauggugccaaacggccuggacauccugaagugcccggugucgagaauguaccccaccgacgauucugcgccccugccggccgguacucuugaccaaccucuguucgaagugauccaggaagcaaugcagaagcacaugcagggcauucaguuccgggagcgcaacgcagggccgcaaaucgacaggaacaugaaggacgaaggauucaacaucaccgcgggaguggacgaagagacuggcuucgucuacgguggaaaucgguucaacugcgggaccuggauggacaagaugggcgaaucagaccgagcccgcaaccgcggaaucccugccaccccccgggaugggagcgccguggagauugugggacugagcaagagcgcugugcgcuggcugcuggaguugagcaagaagaacauuuuccccuaucacgaagugaccgugaagcggcacggaaaagcuaucaaaguguccuacgacgaguggaacagaaagauccaggacaacuucgagaagcuguuccacguguccgaggacccgucggacuugaaugagaagcacccuaaccucgugcacaagcggggaaucuacaaggacagcuacggagcauccucgccuuggugcgacuaucagcugaggcccaacuucacuaucgcaauggugguggccccagaacuguucacuaccgaaaaggccuggaaggcacuggagaucgcagagaaaaagcugcugggcccucugggcaugaaaacccuggaccccgacgacaugguguacugcgggaucuacgauaacgcucuugacaaugacaacuacaaccuggcuaagggauucaacuaucaccagggccccgaguggcuguggccgaucgguuacuuccugcgcgccaagcuguacuuuucccggcugaugggcccugagacuaccgcaaagacgaucgugcuggucaagaacgugcugucacggcacuacgugcaucuggaacggagcccguggaagggguugcccgaacugaccaacgaaaacgcgcaguacuguccguucucgugcgaaacucaggccugguccaucgccacuauccucgaaacucucuacgaccuguag

SEQ ID NO: 8 - RNA, 4599 nt, Artificial Sequence
  Codon-Optimized AGL Coding Sequence
augggacauagcaaacaaauuaggauccuccugcugaacgaaauggaaaaacuggaaaagacgcuguuucggcuggaacagggcuacgaacuccaguuucgccucgggccaacgcugcaagggaaagcagugaccguguauacaaacuacccauucccuggagagacauucaauagggagaaguuuagaagcuuagacugggaaaauccaaccgaacgagaagaugacagcgauaaguauugcaagcugaaucugcaacaguccggaaguuuucaguacuacuuuuugcaagggaacgaaaagagcggcggagguuauauugugguggauccaauuuugagaguuggggccgacaaccauguacugccucuugacugugugacacugcaaacguuccuggccaagugccugggcccguuugaugagugggaaagccguuugcgcguggccaaggaauccggguacaacaugauccauuuuaccccacugcaaaccuuaggccugucaaggagcuguuacagucuggccaaccagcuggaacugaaucccgacuucucccggccaaauaggaaguacacguggaacgacguuggccagcuaguggagaaguugaagaaggaguggaacguuauuugcaucacugacgucguguauaaucacacugccgcuaauagcaaauggauccaggaacauccagagugugccuauaaccuggucaacagcccgcaucugaagccagcaugggugcuggaccgggcguuguggcgguucucgugugacguggccgaaggaaaguauaaggagaaggguauuccggcucugauagagaacgaccaucauaugaauuccaucaggaagaucauuugggaggacaucuuuccaaaguugaagcugugggaguucuuucaaguggaugugaacaaggccguagaacaguuucgccgccuacuaacccaggaaaauaggagagucacaaaguccgaucccaaccaacaucugaccauaauucaggaccccgaauaucgucgauuuggcugcaccguggauaugaacaucgcuuugacaacuuucauaccacacgacaaggguccagccgccauugaagaguguuguaacugguuucacaaacgaauggaggaguugaacagugaaaagcaccgccugaucaauuaucaucaggagcaggccgugaacuguuugcuggggaauguguucuaugagaggcucgcuggucauggcccuaagcuggguccuguaacaagaaagcauccauuagugacgcgcuacuuuacauucccauuugaggagaucgacuuuucgauggaagaguccaugauucaucuccccaacaaggccuguuuucugauggcccacaacggcuggguuaugggggaugauccguugagaaauuuugcggaaccagguucagaaguguaucugcgucgggagcugauuuguuggggcgacuccgugaagcuccgcuaugggaacaagccugaggauuguccuuaucugugggcgcauaugaagaaguauacagagaucacugccacauauuuucagggcgucaggcuggacaauugucauagcaccccgcuucauguggcugaguauaugcuggacgcagcaaggaaucugcagcccaaucuguaugugguggcggaacuguuuaccggguccgaggaccuggacaauguauuuguaacccgauugggcaucuccagccugauuagggaagcaaugagugcauacaacucacacgaggaggggcggcugguuuaucgauaugggggggaaccugugggcagcuuuguacagccaugucuccggccguugaugccugccauugcucaugcgcucuuuauggauauaacacaugacaacgaauguccaaucguucauaggagugcuuacgacgcccugccgagcacaacgaucguguccauggccuguugugcaaguggcagcacacguggcuaugacgaauugguaccccaccaaauuagcgugguuuccgaggagagguucuauacaaaguggaauccagaggcuuugcccucgaacaccggagaggucaacuuucaaucuggcauaauugccgcucgcugcgccauaucuaaguugcaucaggaacugggcgcgaagggguuuauacaagucuacguugaccaaguggaugaggacaucguugcugucacgcggcacucaccuaguauucaucaauccgugguagcagugucucggacggccuuuagaaacccaaagacaucauuuuacucgaaagaagugccucaaauguguauaccuggcaaaauugaagaggugguccuggaagcccgcacgauagagaggaauacuaagccguauagaaaggaugaaaauucuaucaacggcacuccggauauuacaguagaaaucagagagcacauucaacuuaaugagucuaagauuguuaagcaggcugguguugcaaccaaagggccaaacgaguacauccaggagauugaauuugaaaaucugucaccgggcuccgugaucaucuuuagaguaucuuuggauccacaugcucaagucgcuguuggaauccugagaaaccaucugacacaauuuuccccacauuuuaagagcggcagccuggccguggacaacgcagacccaauccugaagaucccauuugcaucccuggcuucccgccugacucuggcugagcugaaccagaucuuguaucgcugugaaucugaagaaaaagaggauggcggaggcuguuaugacaucccaaauuggagcgcccugaaauaugccggacuccaaggccugauguccguucuggccgagauuaggccaaagaaugaucugggacacccauuuuguaacaacuugcggucuggagacuggaugaucgacuaugucagcaaccgccugauaagcagauccgguacuaucgcugaagucggaaaauggcugcaggcuauguuuuucuauuugaagcagauuccgagauauuugauccccuguuauuuugaugccauucugauuggugcuuauacuacccugcuggauaccgcuuggaaacagaugaguagcuuuguccaaaauggcuccaccuucguaaagcaucugucgcugggcuccgugcaauuguguggcgucgggaaguucccuagccugccaauccuguccccugcucugauggacgugccuuaucgccugaacgagauuacgaaggaaaaggaacaguguugcgugucacucgcugcugggcugccacacuuuucuucuggaauuuuucgguguugggggcgggacaccuuuauugcccugaggggcauucugcugauuaccggccgcuaugucgaggcuaggaacauuauccuggcuuucgcggguacccuucggcacggacucauacccaaccuccugggagaaggaaucuaugcacgguauaacugucgggacgcaguuugguggugguugcaguguauucaagauuauugcaagauggucccgaacggacuggacauacugaagugcccagugucccggauguauccaacugacgacuccgcaccacugcccgcugggacacuugaccagccauuguuugaaguuauucaggaagcuaugcagaagcauaugcagggaauucaguuuagggagagaaacgcuggaccccagauugaccguaacaugaaggaugagggguuuaacauuaccgcgggaguggacgaagagacuggcuucgucuaugguggcaaucgguucaacugcggcaccuggauggacaaaaugggcgaaagcgauagagcucgaaauaggggcaucccagcaacaccacgggauggcucugccguggagauugugggccugucuaagagcgcaguucggugguuguuggaacucagcaagaagaacauuuuuccauaccaugaaguuacagugaagcggcaugggaaggccaucaagguuucuuacgacgaauggaaucggaagauccaggauaacuucgagaaacuguuucauguauccgaggacccuucugaccugaacgaaaagcauccaaauuugguacacaaaaggggaaucuauaaggauaguuauggagccagcagcccuuggugcgacuaucagcuacgaccaaacuucacuauugccaugguaguagcaccagaacucuuuacuaccgaaaaggcuuggaaggcacuggagaucgccgagaagaagcuguuagguccacugggcaugaaaacccuggaccccgacgacaugguuuacuguggcaucuaugacaacgcucuggacaaugacaacuauaaucuggccaagggcuucaacuaccaccagggcccagaguggcuauggccaauuggcuauuuucugcgggcgaagcuguacuuuucacgauugaugggcccagagacaaccgcuaagaccauaguauuggucaagaacgugcugagucggcacuauguccaccuggaaaggagccccuggaaggggcugcccgagcugaccaacgaaaaugcacaguauuguccguuuucaugcgaaacccaggcuugguccaucgcgacgauccuggaaacccucuaugaucuguag

SEQ ID NO: 9 - RNA, 4599 nt, Artificial Sequence
  Codon-Optimized AGL Coding Sequence
augggacacucaaaacagauaaggauccugcugcugaacgaaauggagaaacuggaaaagacccuguuccggcucgaacagggauaugaacuccaguuuaggcugggcccaacucugcaaggaaaagcugugaccgucuauacuaacuauccauuucccggggaaacguuuaaccgagagaaguuccgauccuuggacugggaaaaucccacagagcgggaggaugauucggacaaguauugcaagcugaaucugcaacaaucgggcagcuuucaguacuauuuucuacaaggaaacgaaaagagcggcgggggauacauugugguggacccaauccugaggguuggggcagacaaucacguacugccuuuggacugugugacauugcaaacauuccuggcaaagugccugggccccuucgaugaaugggagucacggcugcgaguggcuaaggaaucuggcuauaauaugauucacuuuacaccauuacaaacgcugggccugagcagaaguugcuacucgcuggcuaaucaguuggaguugaacccggacuuuagccgucccaaccggaaguauacauggaaugauguuggccaacucguggagaagcugaagaaggaguggaacgugaucuguauuaccgaugucguguauaaucauacagccgcgaacuccaaguggauucaggagcacccagaaugugcauauaacuuggucaauagcccccaccugaagccggccuggguacuggaucgggcccuguggcgguuuucuugugacguggcagaaggaaaguauaaggaaaaggggaucccagcacugauagagaacgaccaucauaugaacagcauuaggaagaucauuugggaggacauuuucccaaaguugaagcucugggaguuuuuccaaguugacgucaacaaggccguggaacaauuucgaaggcugcugacacaggaaaacagacguguaacgaaguccgaccccaaucagcauuugacgaucauacaggauccugaguauaggcgcuuuggcuguacggucgacaugaauauugcucugaccaccuuuaucccucaugacaaggggccagccgccaucgaagaguguuguaauugguuccacaagcgcauggaagaguugaauuccgaaaagcauagguugaucaacuaccaccaggaacaggcagugaacugucugcugggcaacguguuuuaugagcggcuggccggucauggcccuaagcugggaccagugaccaggaagcauccacucguaaccagauauuuuaccuucccguuugaggagauagauuuuagcauggaagaauccaugauucaccuaccgaacaaggcuuguuuucugauggcucacaacgguuggguuaugggcgaugauccccugcgcaacuuugcggaaccgggcucugagguguacuugagaagggagcugauauguuggggggacuccgucaaacugcgcuaugggaauaagccugaagauugcccuuaucugugggcccauaugaagaaguauaccgagauuaccgcgacauauuuucaaggagugcggcuggacaacugccacagcacgccgcugcauguggcagaguauaugcuggacgcagcccgcaaucugcagccaaaucuguauguuguggcugagcuguuuacgggcuccgaggaccucgacaacguuuucguaacccggcugggcaucagcagccugauccgggaagcuaugucagcguauaauagccaugaggagggcagacugguguacagauaugguggcgaaccaguuggcagcuuugugcagcccuguuugcgcccucugaugcccgccaucgcacaugcuuuguucauggacaucacgcaugauaacgaaugucccauuguacaucgcuccgccuaugacgcuuugccauccacaacaaucguguccauggcuuguugugcaagcggcagcaccaggggauaugacgaauugguuccgcaucaaaucagcgugguaucagaggaaagguuuuauacaaaguggaauccugaagcccugccauccaacaccggcgaagugaacuuucagucggguaucauugccgcgcguugcgcuauuagcaaacugcaucaggagcugggugcuaaaggcuuuauccaaguuuauguggaucaaguagacgaagauauuguugccguaaccagacauagccccagcauucaucaauccgugguugcugugucccggacggccuucaggaacccuaaaacauccuuuuauuccaaggaagucccacagauguguauuccgggaaagauagaggaagugguuuuggaggcucgcacgauugagcggaacaccaagccauauaggaaggacgagaacucgaucaacggcacgcccgacauuaccguugaaauucgcgagcacauucagcugaacgaaucgaaaauugucaagcaggccggcguagcgaccaaggguccaaacgaguauauccaggaaaucgaguuugagaaucugucgccuggguccguaaucauuuuuagagucagccuagacccucacgcucaaguggccguagggauccugaggaaucaucugacgcaguuuucaccccauuuuaaguccggcagccuggcaguggauaacgccgaccccauccugaaaauucccuuugcuucccuggccucgcgccugacacuggcagaauugaaucagauacuguaucguugcgagagcgaggagaaggaggacggagggggguguuaugauaucccgaacugguccgcucugaaauaugcgggauugcagggcuugaugaguguacuggccgaaauuagacccaagaacgaucugggccauccguucuguaacaaucugcgauccggcgauuggaugauugauuaugucagcaaccgguugauaagccggagugggacaauugcagaagucggaaagugguugcaagccauguucuuuuaccugaagcagaucccucgauaucugauaccauguuauuucgaugccauucugaucggggccuauacaacucuguuagacacugcuuggaaacagaugucuagcuucgugcaaaacggcucaacauuuguuaagcacuugagccuggggucugugcaguuguguggcguaggaaaguuucccucacugcccauccugucgcccgcccugauggacgugcccuaccgccucaacgaaauuaccaaggagaaagagcaguguuguguuagcuuggcugccgguuugccgcauuuuucaagcggaaucuuccgaugcuggggacgcgauacguucauagcccugagggguauucugcugauuacgggcagauacguagaggcucggaauauuauccuggccuucgccggcacgcugcggcaugggcugauuccgaacuugcugggagagggcaucuacgcccgguacaacugcagggacgcuguguggugguggcugcagugcauccaggacuauugcaaaauggugccaaacggccuugacauacugaaguguccugucucucggauguauccaacggaugacuccgcaccccugcccgcuggaacccuggaucaaccccuguuugaagugauacaggaagcaaugcagaagcacaugcagggaauucaguuuagagagagaaaugcaggcccccaaaucgacagaaacaugaaagaugaaggcuuuaacaucacggcuggaguggacgaagaaacuggguuuguguauggcgggaauagguuuaacugugggacguggauggacaagaugggcgaauccgauagagcgcggaacaggggaaucccggcuacaccccgggacgguagugcuguggagauugucggcuuauccaaauccgccgugcgcuggcugcuggagcuguccaagaagaacaucuuuccuuaccaugaagugaccgugaagcggcauggaaaggccaucaaagucuccuacgacgaauggaauaggaagauucaggacaauuuugagaagcuguuucauguguccgaggaucccagcgaccugaacgagaagcacccuaauuuggugcauaagcggggcaucuauaaggacuccuacggcgcuaguucgccuuggugcgacuaucagcugcggccaaacuuuacgauugcgauggugguagcccccgaauuguuuacgacggaaaaggcuuggaaggcccuggagaucgcagaaaagaagcugcuggggcccuugggcaugaaaacgcuggaccccgacgauaugguuuauuguggcaucuacgacaacgcccucgacaaugacaauuacaaccuggcaaaggguuuuaacuaucaucaggguccugaauggcuguggccaauuggcuacuuuuugcgggccaagcuguacuuuucacggcugaugggaccugaaaccaccgcuaagaccauuguacuggucaagaacgugcugagcaggcauuacgugcaucuggaaagaagcccguggaagggucugccagaguugacgaacgagaacgcgcaguauuguccuuucucuugugaaacgcaggcuuggaguauugcaaccauucuggaaacucuuuaugaccuguag

SEQ ID NO: 10 - RNA, 4599 nt, Artificial Sequence
  Codon-Optimized AGL Coding Sequence
augggccacucaaagcagauuagaaucuuacuccugaacgagauggaaaagcuggaaaagacccuguuccgccuggaacagggauaugagcugcaguuccggcuuggaccaacccuccaaggaaaggccgugaccguguacacgaacuacccauucccgggcgaaaccuucaacagagagaaguuccggagccuggacugggaaaacccgaccgaaagggaagaugauagcgacaaguacugcaagcugaacuugcaacaguccggaucauuccaguacuacuuucugcaagggaacgagaagucgggcggcgguuacaucgugguggacccuauucugcgcgugggagccgacaaccacguguugccucuggacugugucacccugcaaacuuuccuggccaagugccuggggccauucgaugagugggaaucgcggcugcggguggcaaaagaguccgguuacaacaugauccacuucaccccacuccaaacccugggccuguccaggucgugcuacucgcuggccaaccagcuggaacugaacccggauuucucgcggccuaacagaaaguauaccuggaaugacgucggacagcucgucgaaaagcugaagaaggaauggaacguaaucuguaucaccgaugucguguauaaccacaccgcugccaacuccaaguggauccaggaacaccccgagugcgcuuacaacuuggugaacucgccccaccugaaaccggcuugggugcuggaccgggcccuguggcgguucagcugcgauguggcugagggaaaguauaaggagaaggguaucccagcgcucauugaaaacgaccaccauaugaacucgauccgcaagaucauuugggaggauauuuucccaaaguugaaacugugggaguuuuuccaaguggacgugaacaaggcggucgaacaguucagacggcuguugacucaggaaaaucggagggucaccaagucggaucccaaccagcaccugaccauaauccaggauccagaauaccggcgguucggcugcacuguggacaugaacauugcccugaccacuuuuaucccacacgacaagggcccggccgccaucgaagagugcugcaacugguuccacaagcggauggaggaacugaacucggagaagcaccgccugaucaacuaccaccaggagcaggcgguuaacugucuguugggaaacguguucuacgagcgguuggccggccacggcccuaagcugggcccggucacccggaagcacccccuggucacccgcuacuucaccuuuccauucgaggagaucgacuucagcauggaagaaucgaugauccaucugccgaacaaggccugcuuccugauggcucacaacggaugggugaugggcgacgauccucugagaaacuuugccgagccgggcucggagguguaccugaggagggagcugaucuguuggggggacagcgugaagcugagauacggaaacaagccagaggacugcccguaccugugggcccauaugaagaaguacaccgagauuaccgcaacauacuuccaagggguccggcuggacaauugccacucgacuccccugcacguggcggaguacaugcuggacgcggccaggaaccuccagcccaaccucuacgucguggccgagcuguucacugguuccgaggaccuggauaacguguucgugaccagacuggggaucuccucacugauucgcgaagccauguccgcguauaacucgcaugaagagggccgccugguguaccgcuacggaggcgaaccugugggcagcuucgugcaaccgugucugcggccucugaugccugccauugcgcacgcccuguucauggacaucacccacgacaacgaaugccccaucgugcaccgguccgccuacgaugcccucccuucgacuacuaucguguccauggcuugcugcgcguccggcucgacccgcggcuacgaugagcucgugccgcaucagauuagcgugguguccgaggaaagguucuacaccaaguggaauccagaagcgcugccgagcaacaccggggaggucaacuuccagucgggaaucaucgccgcccgcugugccaucuccaagcugcaccaggaacugggcgcgaaggguuucauccaagucuacgucgaucaggucgacgaggacaucguggccgugacucggcauuccccgagcauucaccaguccgugguggccgugucgcgcaccgccuuccgcaacccuaagaccagcuucuauucaaaagaagugccgcagaugugcaucccuggaaagaucgaggaggugguccuggaagcgcggacuaucgaaaggaacaccaagccauaccgcaaggacgagaacuccaucaacgguaccccggacaucacuguggagauccgcgagcauauucaacugaacgaguccaagaucgugaaacaggccggaguggcaaccaagggaccgaacgaguauauccaggaaauugaguucgagaaccucuccccgggaagcgugauuaucuuccgcgugucccuggacccacacgcccaaguggccgucggcaucuugcggaaccaccugacucaguucuccccgcauuucaaguccggaagccuggcgguggacaacgcggacccaauccugaagauacccuucgccucacuggccucgcgccugacuuuggccgaguugaaucagauccuguaccgcugcgaauccgaagaaaaggaggacgguggaggcuguuacgacaucccuaacugguccgcacugaaauacgcaggacugcagggacugauguccguccucgcugaaaucagaccgaagaacgaucucggccacccauucugcaacaaccugagauccggcgauuggaugauugauuacgugucgaaccgacugaucucccgcucggguacuauugcggaagucggaaaauggcugcaggccauguucuucuaccugaagcagaucccacgauaccuuaucccuugcuacuuugacgcgauucugauuggugccuacacgacccugcuggacacggccuggaagcaaauguccagcuuugugcagaacggcagcaccuucgugaaacaccugucgcugggaucggugcagcucugcggcguggggaaguuuccgucacugccgauccuguccccggccuugauggaugugcccuaccggcugaacgaaaucaccaaggagaaggagcagugcugcgugucgcuggccgccgggcugccucacuucuccuccggaauuuuucgaugcugggguagagacacuuucauugcgcugagggggauucugcuuauuaccggccgcuacguggaagccaggaacaucauccuggcauucgccggaacccugcggcacgggcugauucccaaccuccucggagaaggaaucuacgcucgguacaauugccgggacgcaguguggugguggcuccagugcauccaggacuacugcaagauggucccuaacggacuggacauucugaagugcccagugucccggauguaccccacugacgauucggcaccgcugccggcugguacccuggaccagccgcuguucgaagugauccaggaagccaugcaaaagcauaugcaggggauucaguuccgcgaaagaaaugccggaccucagaucgaccgcaacaugaaggaugaaggcuuuaacaucacugccggaguggacgaagagacuggauucgucuacgggggaaacagauucaauugcgguacauggauggauaagaugggagaaagcgacagagcucggaauagaggaauuccggccacaccucgggacggcucagccguggagaucguggggcuauccaagucugccgugcgcuggcuguuggaacugucgaagaagaacauuuucccauaccacgaggucaccgugaagcgccacggaaaggccaucaaagugucauacgaugaauggaaccgcaagauucaggacaacuucgagaagcuguuccaugugucggaggacccuuccgaccugaacgaaaagcauccaaaccuggugcacaagcgggggaucuacaaggacuccuacggagcguccuccccuuggugcgacuaccaacuccggccaaauuucacgaucgcgauggugguggccccugaauuguuuaccaccgaaaaggccuggaaggcccucgagaucgcagagaagaaacugcugggaccccugggcaugaaaacccuggacccggacgauaugguguacugcggaaucuacgacaacgcccucgauaaugacaacuauaacuuggccaaggguuucaauuaccaccaggggccagaguggcuguggccaaucgguuacuuucugcgggccaagcuguacuucucgagauugauggggcccgaaaccaccgcuaagacuaucgugcucgucaagaacgugcugucacggcauuacgugcaccuggaacgcagcccauggaagggccugccggaacugaccaacgagaacgcacaguacuguccguucucgugugaaacucaggccuggagcauugcgaccauccuggaaacucucuaugaucuguag

SEQ ID NO: 11 - RNA, 4599 nt, Artificial Sequence
  Codon-Optimized AGL Coding Sequence
augggccauucuaagcaaauucggauacugcugcugaacgaaauggagaaacuugaaaagacccuguuccggcuggagcagggcuaugagcugcaguuuagauugggcccgacacugcaggggaaggcagucaccguuuauaccaauuauccuuuuccuggggaaacguucaaucgugaaaaguuucggagccucgacugggaaaacccuaccgagcgagaggaugauagcgacaaguauuguaaacucaaucugcagcagucaggcucauuccaauauuauuuucugcaagggaacgagaagucuggcggaggcuacauugucguugauccgauacugcggguuggcgccgacaaccacguguugccucuggacugcgugacacugcaaacauuucucgcgaaaugcuuaggccccuuugaugagugggaaagccgccugagagucgccaaggagagcggcuauaauaugauccauuuuacgccgcugcaaacacugggucugucuaggucauguuacucauuggcuaaccagcuggagcugaacccggacuuuaguaggccuaacaggaaguauacauggaaugauguugggcaacugguggagaagcugaagaaggaauggaaugucauuuguauuaccgaugucguguacaaccacacggcagcaaauucaaaguggauucaggaacauccggaaugcgcuuauaaccucguaaacucaccgcaccugaagccggccuggguacuggacagggcacuguggagauucucuugugauguagccgaggggaaguacaaggagaaaggcauucccgcucuuauugaaaaugaccaccauaugaauagcauuaggaagaucaucugggaagauauuuuuccaaaacugaagcugugggaauucuuucaaguugacgugaacaaggcugucgagcaguucaggcggcuguugacccaggagaacagacggguuacuaagagugaccccaaccaacaucugacgaucauccaggacccagaguaucggcgcuuuggcugcacaguggacaugaacaucgcccugaccacguuuaucccccaugauaagggcccggccgcuauugaagaguguuguaacugguuucauaagcgcauggaagaacucaacagcgaaaagcauagacugaucaacuaucaucaagaacaggcugugaauugucugcugggcaacguguuuuaugagcgguuggcuggccauggccccaaguugggccccgugacgcgaaaacauccccucgugacaagauauuucaccuuuccauuugaagagaucgacuucucaauggaggaaagcaugauucaucugccaaacaaggcuuguuuucugauggcucauaauggcuggguuaugggcgacgacccccugagaaacuuugcggaaccagggucugaaguguaucugcggagggaauugauuugcuggggagacucuguaaagcugcgauaugggaacaagccggaggauuguccguaucugugggcccauaugaagaaguauacagaaauuaccgcaacguauuuucagggcguacgccuggauaauugucauucaacgccacugcauguggcagaguacaugcuagacgcggcuaggaaucugcagccgaaucuguaugucguggccgagcuguucaccggcuccgaagauuuggacaauguguuugugacccgccucgguauuagcucacugauuagagaagcaaugucggcuuacaauucgcaugaggaaggucgccugguguaccguuacggcggcgaacccgugggcaguuuugugcaacccugucugaggccacuaaugcccgcuauugcacaugcccuguuuauggauauaacacaugauaacgaauguccaaucguacaccggagugcuuaugaugcucugcccucaacgaccaucguaucaauggcaugcugugccuccggcucaacacggggcuaugaugaacugguaccacaccagaucagcgugguuucugaggaacgguuuuacacaaaguggaauccugaggcguugccauccaacacuggcgaagugaacuuucagagcggcauuauugcugcccgaugugcuauuucaaagcuacaccaggaguugggcgcaaagggguuuauccagguuuauguggaccagguugacgaagauaucguagcugugacgcggcacucuccgucuauccaucaauccgugguagccgugucuaggacggcuuuucgcaaccccaagacaaguuucuauuccaaagaaguaccccagauguguaucccggggaagauugaggaagugguccuggaggccaggacgauagaacggaacacgaagccguaucgcaaggacgaaaacagcauaaacgggacgccugacaucacgguggagauucgcgagcacauccaguugaacgaaucaaagauagugaaacaggcugggguggcuaccaagggcccaaaugaguacauucaggagaucgaguucgaaaaccuguccccgggcagugugaucaucuuuagagucucuuuggauccgcaugcccaggucgcugugggcaucuugcgaaaucaccugacgcaguuuucuccacauuuuaagaguggcucccuggcuguggacaacgccgacccaaucuugaagauuccguucgcuucccuggcuucacgucugacucucgcugaauugaaucaaauucuguauagaugcgaaucagaggagaaggaagauggaggcgguuguuacgacaucccgaauuggucggcacugaaauacgccggucugcaaggcuugaugagcguacuggccgagauaagaccaaagaacgaucugggccacccauuuugcaacaacuugcgguccggcgauuggaugauugacuaugucucuaaccgacucaucaguagaagcggaaccauagcugaggucggcaaauggcugcaagccauguucuucuauuugaagcagaucccccgauaucugauccccuguuauuuugacgcaauccucauuggcgccuauaccacacuccucgacaccgcuuggaagcagauguccucauuugugcaaaacgguagcaccuuugugaagcaucugucgcuggguagugugcagcucugcggcguagggaaguuccccaguuugccgauccugaguccagcucuaauggacgugccauauaggcugaacgagauuaccaaggaaaaggagcaguguugugucucccuugcugccggucugccccauuuuuccucgggcauuuuuagauguugggggcgggacaccuucaucgcucugcggggcauccugcugaucaccggcagauauguggaggcucggaauauuauucuggcuuuugcugggacgcugcgccauggacugauucccaaucuauugggcgaaggcauauacgcuagguauaacugucgggacgcuguuuggugguggcugcaguguauccaagauuauugcaagaugguccccaacggccuggacauacugaaauguccaguaucuaggauguacccgacugacgacagugcuccccugcccgcuggaacuuuggaucaaccccuguuugagguuauucaagaggcuaugcagaagcacaugcagggcauucaguuucgcgaaaggaacgccggcccccaaauugaccguaacaugaaggacgaaggcuucaauauuacggcuggcguagaugaagaaacaggcuuuguguacggcggcaaccgcuucaacugugggacauggauggacaagaugggcgaaagcgacagggcucggaacaggggaauuccagccacgccccgcgauggcagugcuguugaaauugucggcuugucaaaaucagccguacgcugguuauuagagcucuccaagaagaacaucuuuccguaucaugaagucacgguuaagcggcauggaaaagcaaucaaagugucuuacgacgaauggaauaggaaaauucaggacaacuuugagaagcuguuccaugugucugaggacccguccgaucuuaacgagaagcaucccaauuuggugcacaagaggggcaucuauaaggacucauacggggcuagcucaccuuggugugacuaucagcugcgaccgaauuucacaauagcuauggucguggcuccggagcuuuuuaccaccgagaaggcuuggaaggcccuggagauugccgagaagaagcuguuaggcccguugggcaugaaaacguuggauccagacgacauggucuauuguggcaucuaugacaacgcucucgacaaugacaacuauaaccuagcuaagggcuucaauuaccaucagggcccggaguggcuguggccaauuggauauuuccugagggcaaagcuguauuucucccggcugaugggccccgagacaacggcaaaaaccauagucuugguuaagaacgugcugucccgccacuaugugcaccuugaaaggaguccguggaagggccugccggagcugacaaacgaaaaugcccaguacugcccauuuucuugcgaaacucaggcuuggagcaucgccacaaucuuggaaacccuguaugacuuguag

SEQ ID NO: 12 - RNA, 4599 nt, Artificial Sequence
  Codon-Optimized AGL Coding Sequence
augggacacucgaagcagauccgcauccuccugcugaacgaaauggaaaaacuggaaaagacacucuuccggcuggaacagggauaugagcugcaguuuagacuggggcccaccuuacaaggaaaggccgugacugucuauaccaacuacccguuccccggagaaacuuucaaccgggaaaaguuccggucacuggacugggaaaacccgaccgagcgggaggacgauagcgacaaguacugcaagcugaaccuucagcaguccggaucguuccaguacuacuuccugcaagggaacgagaagucgggcggaggauacauuguggucgauccuauccugcgcgugggagcugacaaucacgugcucccucuggacugcgugacgcugcaaaccuuccucgcaaagugccucggaccuuucgacgaaugggaauccagacuccgcguggccaaggagucaggauacaacaugauccacuucacgccgcugcagaccuugggacucucucggagcuguuacucccuggccaaccagcuggaacugaacccagacuucucacgcccgaauagaaaguacaccuggaacgacgugggacagcuuguggagaagcucaagaaggaauggaacgucaucugcauaaccgacgucguguacaaccacaccgcagccaauucuaaguggauucaggaacaccccgaaugcgccuacaaucugguuaacucaccccaccuuaagcccgccuggguccuagacagagcccucuggcgguucucgugugacguggccgagggaaaguacaaggagaagggaauccccgcucugauugaaaacgaccaccacaugaacuccauccgcaagauuaucugggaggacaucuucccgaagcucaagcugugggaauucuuccaaguggacgugaacaaggcggucgagcaguucagacgccugcugacccaggaaaaucggagagugaccaagagcgauccuaaccagcaccugaccaucauccaagacccagaguaccggcgguucggaugcacuguggauaugaacaucgcccugaccacuuucaucccucacgacaagggaccggccgcaauugaggaaugcugcaacugguuccauaagcggauggaggaacugaacagcgagaagcaucgacugaucaauuaucaucaagagcaggcugugaauugccugcugggaaacguguucuacgaacggcuggccggacauggcccuaagcuggggccugugacccggaagcacccucuugugacccgauacuucaccuucccguuugaagaaauugauuucuccauggaagaauccaugauccaucugccaaacaaggccugcuuccuuauggcccacaauggcugggucaugggggacgacccucuucggaacuucgccgaaccagggagcgagguguaccucagaagggagcucaucuguuggggggauuccgugaagcucagauacggaaacaagccagaagauugccccuaccuuugggcccacaugaagaaguacaccgaaaucaccgccacauacuuccaaggagugcggcuggacaacugccauucaacuccccugcacgucgccgaguacaugcuggacgcugcgagaaacuugcagcccaaccuuuacgugguggccgagcuguucaccgggagcgaggaccuggacaacguguuugugaccaggcucggaaucucgucgcugauucgcgaagccaugagcgccuacaacucccacgaagaggguagacugguguacagauacggaggagagccagugggauccuucguccaaccgugccugcggccgcucaugccugcgaucgcacacgcgcuguucauggacaucacccacgauaacgaauguccuaucgugcauaggagcgccuaugaugcccuucccuccaccaccaucguguccauggcgugcugugccucggguagcaccaggggauacgacgagcuggugccgcaccagaucucggugguguccgaagaacgguuuuacacuaaguggaacccugaggcgcugccuuccaacaccggagaagugaacuuccaguccgguaucauugccgcucgcugcgcaaucagcaaacugcaccaggagcuuggugccaaaggauucauccaaguuuacgucgaucaaguggacgaggauauuguggccgucacuaggcacucuccaagcauucaccaguccguaguggcagugucgaggaccgccuuccggaaccccaagacuucauuuuacucgaaagaggucccacagaugugcaucccuggaaagaucgaagaaguggugcuggaagcccggaccaucgagaggaacacaaagcccuaccggaaggacgagaacuccaucaacggaacccccgacauuaccguggaaauuagagagcacauccaguugaacgagucgaagaucgugaagcaggccggaguggccacuaagggaccaaacgaguacauccaggagaucgaguuugaaaaccuguccccgggcuccgugaucaucuuccgggugucccuugacccccaugcccaaguggccgucggaauccuuaggaaccaccugacccaguuuucgccccauuucaaguccggauccuuggcugucgacaaugccgaucccauccugaaaauuccguucgccucccucgcuucccggcucacccuugccgaacucaaccagauucuguaccgcugcgagucagaagaaaaggaagauggagggggaugcuacgacaucccgaacugguccgcccuuaaauacgccgggcugcaaggccugauguccgugcuggcggagauuagaccgaagaacgacuugggucacccuuuuugcaacaacuugcggagcggagacuggaugaucgacuacgugucgaaccggcugauuagucgguccggaaccaucgccgaagucggaaaguggcuccaagccauguucuucuaccugaagcaaauuccccgcuaccugauaccgugcuacuucgacgccauccucauuggagccuacaccacgcugcuggacaccgccuggaagcaaaugagcuccuucgugcaaaacggaucaaccuucgugaagcaccugucccuggguagcguccagcucuguggcgugggaaaguuuccgucccugccaauucugagcccggcucugauggaugugccguaucgccugaacgagaucacgaaggagaaggagcaguguugcgugucgcuggcugcgggacugccucacuucucguccggaaucuuccgcuguuggggacgcgacacguuuaucgcguugagggguauucuccucauuaccggacgcuacguggaagcgcggaacauuauccuggcguucgccggaacccugcgccacggucugauuccuaaucugcugggagagggaaucuacgcgcgguacaacugccgggaugcugugugguggugguugcagugcauccaggacuauuguaaaauggugccgaacggccuggacauccugaagugcccggugucccggauguacccgaccgaugauucagcaccacugcccgccgggacccuggaccagccccuguucgaagucauucaggaagcgaugcagaagcauaugcagggaauccaguuccgcgaaagaaacgccggaccucagaucgaccgcaacaugaaggaugagggcuucaacaucaccgcgggaguggaugaggaaaccggcuucgucuacggagggaaccgguucaacugcggaaccuggauggacaagaugggagaguccgaccgcgcaagaaaccgcgguauuccugccaccccgcgggacggaagcgcgguggagaucgucggacugagcaagagcgcagugcgcuggcugcuggaguuguccaagaagaauaucuuccccuaucacgaggucaccgugaaacgccacgggaaggccaucaaaguguccuacgaugaguggaaccgcaagauucaggauaacuucgaaaagcuguuucauguguccgaggaucccuccgaccucaacgaaaagcacccgaaccucgugcauaagagggggaucuacaaggacagcuacggugccuccucaccuuggugcgauuaucagcuccgcccgaacuucaccauugccaugguggucgccccugaacuguuuacuaccgagaaggccuggaaggcgcuggagauugccgaaaagaagcuguugggaccccugggcaugaaaacccucgaccccgacgacaugguguacugcggaaucuacgacaacgcccucgacaacgacaacuacaaccucgcgaagggguucaacuaccaccagggccccgaauggcuguggcccaucggauacuuccuccgggcgaaguuguacuucucccgccugaugggcccugaaaccacggccaaaacgaucgugcucgugaagaacgugcugucgaggcauuacgugcaccucgagcggagcccguggaaggggcugccggaacugaccaacgagaaugcacaguacugccccuucuccugcgaaacgcaggcuugguccauugccacuauuuuggaaacgcuguacgaccuguag

SEQ ID NO: 13 - RNA, 4599 nt, Artificial Sequence
  Codon-Optimized AGL Coding Sequence
augggacacucgaaacagaucagaauccuguugcucaacgaaauggagaagcuggaaaagacccucuuucggcucgagcagggcuacgagcugcaguuccgccuggguccgacacuacaaggaaaggcagugacuguguacaccaacuacccauuucccggagaaaccuucaaccgggagaaguuccggucccuggacugggaaaacccaaccgaacgagaggaugacuccgacaaguacugcaagcugaaccuccaacaguccgguucauuccaguacuacuuucugcaagggaacgagaaguccggaggcggcuacaucguggucgacccgauacuuagagugggagccgacaaucauguccugccucuggacugcgugacccugcaaaccuucuuggccaaaugucugggcccguucgaugagugggaaagccgccucagagucgcaaaggaguccggauacaacaugauucacuucacuccgcugcaaacccucggucugucccggucgugcuauucucuggcgaaccagcuggagcuuaaccccgacuucucgcgcccaaaccggaaguacaccuggaacgacgucgggcagcuuguggaaaagcugaagaaggaguggaacgugaucugcaucacugacgugguguacaaccauacggccgccaacucgaaguggauccaagagcaucccgagugcgcguacaaccucgugaacagcccgcaucugaagccugcuugggugcuggauagagcccucuggagauucagcugcgacguggccgaggggaaguacaaagaaaagggaauuccggccuugauugagaacgaccaucacaugaacucaauccgcaagaucaucugggaggauaucuucccuaagcuuaaguugugggaguucuuccaaguggacguaaacaaggcaguggagcaguucagaagguugcugacucaagaaaacagacgcgucacuaaguccgauccuaaccagcaccuuaccaucauucaagacccugaguaccgccgguuuggcugcaccgucgacaugaacaucgcccugaccacuuucaucccgcaugacaagggcccggcggcaaucgaggaaugcuguaacugguuucauaagaggauggaggaacugaauuccgagaagcaccggcugauuaacuaccaccaggaacaggcagugaauugccuccugggcaacguguucuacgaacggcuggcuggacacggaccgaagcugggucccgugacucgcaagcauccgcucgugacucgcuacuucaccuucccguuugaggagauugacuucuccauggaagaauccaugauccaccucccgaacaaggcuugcuuccugauggcgcacaacggaugggucaugggcgacgacccacugcgcaacuucgcugagccuggcucggaggucuaccugagaagggaauugauuugcuggggagacuccgucaagcugcgcuauggaaacaagcccgaagauugccccuaccugugggcucacaugaagaaguacacggaaaucacugccacguacuuccagggaguccggcuggacaauugccacuccaccccccuccauguggccgaguacaugcucgaugcagcgaggaaucugcagcccaaucuguacgugguugcagaacuguucacuggcuccgaggaccucgacaacguguucgugaccagacuggggaucuccucccugauccgggaagccaugucggccuacaacucccaugaagagggccgccugguguaccgcuacggcggagaacccgugggaagcuucgugcagccuugccuccggccgcugaugccugcgaucgcccacgcccuguucauggauaucacucacgacaacgaaugccccauugugcaucgcucggccuacgacgcacugccuucgaccacuaucguguccauggccugcugcgccuccgggagcacccgcggauacgaugaacucgugccgcaccagaucagcgugguguccgaagaaagauucuauaccaaguggaaccccgaagcccugccgagcaauaccggggaagugaacuuccaguccgguauuaucgccgcucgcugugccaucagcaaacuccaccaagagcucggugccaagggauucauucaagucuacguggaucaggucgacgaagauauuguggccgugaccaggcacucaccuuccauccaccaauccgucgucgccgugucccggacugcguuucggaaccccaagacuucguucuacucgaaagaagugccacagauguguaucccgggaaaaaucgaagaggucgugcucgaagcccggaccauugagaggaacaccaagccuuaccggaaagacgagaacucuaucaacgguaccccugauauuacuguggagauccgcgaacacauccagcugaacgaaucaaagaucgucaagcaggcuggaguggccaccaagggacccaacgaguacauccaggagaucgaauuugaaaaccucuccccuggcuccgugauuaucuuccgggugucccuggacccucacgcccaaguggccgugggaauucucagaaaccaccugacccaguucucaccccacuuuaaguccgguucccuggcgguggacaacgccgauccgaucuugaagauccccuucgcaucgcuggccucccgccugacucucgcggaacugaaccagauccuguaccgcugugaaucagaggaaaaggaggacggcggcggcuguuacgauauccccaauuggucggcuuugaaauacgcgggacuucaggggcugaugucugugcuggcggaaauccggccgaagaacgaccugggacacccauucugcaacaacuugcggagcggagacuggaugaucgauuacgucagcaacagauugaucagccggagcggcacuaucgccgaggucggaaaguggcuccaggccauguucuucuaccugaagcagaucccccgauaccucauccccuguuacuucgacgccauucugaucggggccuacaccacccugcuggacaccgccuggaagcagaugagcaguuuugugcaaaacggguccaccuucgugaagcaccuuucacugggcucagugcagcucugcggcgugggaaaguuccccucgcugcccauucugagcccggcccugauggacgucccuuaccggcugaacgagaucaccaaggagaaggagcagugcuguguuucccuggcugccgggcugccacacuucucguccggcaucuuccggugcuggggccgggauaccuucauugcccugcggggaauccugcuuaucaccggucgcuacguggaggcucggaacauuauucuggcguucgccggcacccuuagacacggucugauuccgaaucuuuugggcgaaggaaucuacgccagauacaacugucgggacgccguguggugguggcuccagugcauucaggacuauugcaagauggugccgaacggccuggacauccugaagugcccagugucgaggauguauccaaccgacgacagcgcaccucugccggccgggacccucgaccaaccccuguucgaagucauucaagaggcuaugcagaagcacaugcaggguauucaguuccgggagcggaacgcggggccccagauugauaggaacaugaaagacgagggcuucaacaucacugccggcguggacgaagaaaccgguuuuguguacggaggaaacagauucaacugcgguaccuggauggacaagaugggagaguccgaucgcgcgcgcaacagagggaucccggcaaccccgcgggacggauccgcgguggaaauugugggacugagcaagagcgccgugcgguggcuccuggaacugagcaaaaagaacaucuuccccuaccacgaagugaccgugaagcggcacggaaaggccaucaaagucucauacgaugaauggaauaggaagauccaggauaacuucgagaagcuguuucacguguccgaggaucccuccgaucugaacgaaaagcauccgaaucucgugcacaagcgcgggaucuacaaggacucguacggagcguccuccccuuggugcgacuaucagcugcggccuaacuucaccauugccauggucguggccccggagcuguucacaacugagaaggccuggaaggcccuugaaauugccgagaagaagcugcuggggccuuuggggaugaaaacccuggauccggacgacaugguguacugcggaaucuacgacaacgcccuggacaacgauaacuacaaucuggcgaagggcuucaauuaccaccagggcccggaauggcucuggccuauuggguacuuccugcgcgccaagcuguacuucucacggcugaugggaccagagacuaccgccaagacuaucguccucgugaagaacgugcugucccggcacuacgugcaucuggagaggagcccuuggaagggacuuccugagcugacgaacgaaaacgcgcaguacugccccuucuccugcgaaacccaggcuugguccauugccacuauacuggaaaccuuauaugaccuguag

SEQ ID NO: 14 - RNA, 4599 nt, Artificial Sequence
  Codon-Optimized AGL Coding Sequence
augggucacuccaagcaaaucagaaucuuacuccuuaacgaaauggaaaagcuugaaaagacacucuuccgcuuggagcagggcuacgagcugcaguuccggcuggguccgacacuucaggggaaagccgugaccguguauaccaacuaccccuuuccgggagaaacauucaaucgcgagaaguuccggucgcuggacugggagaacccuaccgagagggaggacgacucugauaaguacugcaagcugaaucuccagcaaucagguucuuuccaauauuacuuccuucaaggaaacgaaaaguccgggggcggcuacauuguaguggaccccauccuucgggucggcgcggauaaccaugugcuuccccucgacugcgugacucuccaaacuuuccucgccaagugccugggaccauucgaugaaugggaaucccgccugcgcguggccaaggagagcggcuacaacaugauucacuucacuccgcuucaaacccuugggcugucccgcuccugcuauucccuugcgaaccagcuggaacuuaacccggacuucucucggccgaacagaaaguacacuuggaacgacgugggccagcuugucgagaagcugaagaaggaauggaacgugaucugcaucaccgacgugguguacaaccacaccgcggcaaacuccaaguggauccaggaacauccugagugcgcauacaaccucgugaacaguccgcaucugaagccugccugggugcuggauagagcccuguggcgcuucuccugcgacguggcugagggaaaguacaaggaaaagggcaucccugcgcucauugaaaacgaucaccacaugaacagcauccgcaagauuauuugggaggacaucuucccuaagcucaagcucugggaguuuuuccaaguugacgugaacaaggccguggagcaguucagacggcuccugacucaagaaaacagacgcgucaccaaguccgacccuaaccaacaccucaccaucauccaggaucccgaauaccgccgguuuggcugcacuguggacaugaacauugcccugaccaccuucauuccgcacgacaaaggcccggccgcgauugaagagugcuguaacugguuccacaagagaauggaggagcugaacuccgaaaagcauagacuuaucaacuaccaccaggaacaggccgugaacugccugcugggaaacguguuuuacgagagacucgccggacacgguccaaaguuggguccugugacccgcaaacacccgcucgucacccgcuacuuuaccuucccguucgaggagaucgacuucaguauggaggagagcaugauccaucuccccaacaaggccuguuuccucauggcccacaacggcugggucaugggcgacgacccccugcgcaacuucgcugaacccggcucggaaguguaccuucggagggagcuuaucuguuggggcgacagcgugaagcuuagauacggcaacaagccagaagauuguccguaccugugggcgcacaugaagaaguacaccgagaucaccgcgacguacuuucaaggagugcggcucgauaacugccacuccaccccucugcacguggcagaguacaugcuagacgcggcccggaaccuccagcccaaccuuuacgugguggccgaacucuucacugguucugaggaucuugauaacguguucgugacuaggcucggcauuuccucccucauccgggaagccaugucggccuauaacucccacgaggaggggcggcugguguaccgcuacggaggcgaaccggucggcagcuucgugcagccgugccuccgcccucugaugcccgcuauugcucacgcccuuuucauggauaucacucacgauaaugagugcccuaucgugcaucggagcgccuacgacgcucucccuuccaccaccaucguguccauggcgugcugcgccuccgguucaaccaggggcuacgaugaacuugugccgcaccagaucucagucgucagcgaggaaagguucuacacuaaguggaacccugaagcccugcccucuaacacgggcgaagugaacuuucagagcgguaucauugccgcuagaugcgcaaucuccaaguugcaccaggaacugggagccaagggguucauccaggucuacguggaccaggucgacgaggacaucgucgccgugacccggcauuccccgagcauccaucaguccguggucgccgugucacggaccgccuuccgcaaccccaagaccuccuucuacuccaaggaagugccgcaaauguguaucccuggcaaaaucgaggaaguggugcucgaagcgcggacgauugagaggaauacuaagccguacagaaaggacgaaaacuccaucaacggcaccccggacaucacuguggagauccgggagcacauccagcucaacgagagcaaaauugugaagcaggccggcgucgcuacuaagggcccaaacgaguacauccaggagauugaguucgaaaaccuuagcccugggucugugaucaucuuucgcgugucccucgacccgcacgcacaggucgcagucgggauucuccggaaccaucugacucaguucagcccccacuucaagagcggcagccuugccgucgacaacgccgaucccauccucaaaaucccuuucgcaucccuugcgucgaggcuuacccuggcggaauugaaccagauucuguaccgcugcgagucggaagaaaaagaggauggcggcggcugcuacgacauuccgaacugguccgcccugaaauacgcgggccuucagggccuuaugagcgucuuggccgagauccgccccaagaacgaccuggggcaccccuuuugcaacaaccucagaagcggcgauuggaugaucgacuacgugucgaacaggcucaucagccgauccggcacuauagccgaggucggaaaguggcugcaggccauguucuuuuaccucaaacagaucccgcgguaccugaucccgugcuacuucgacgcuauucucauuggcgccuacacuacccugcucgauaccgcuuggaagcagaugagcucauucgugcaaaacggaagcaccuucgugaagcaccucucccugggaucagugcagcugugcggcgugggaaaguucccauccuuaccaauucucucgccugcccugauggacgucccuuaucgccugaacgaaaucacgaaggagaaggaacaguguugugucucacuggcugccggccucccgcacuucucauccggcaucuuccggugcugggguagagacacuuucauugcgcuccggggaauucugcuuaucacuggccgcuacguggaagcccgcaacaucauccuugccuuugccgggacccugcggcacggccugaucccuaaccuucucggggagggcaucuaugcgcgauacaauugccgggacgccgucuggugguggcugcagugcauucaggacuauugcaagauggugccaaauggucuggacauucugaaguguccagugucccggauguacccuaccgacgauagcgccccacugcccgccggaacccucgaucagccccuguucgaagucauucaggaagcgaugcagaagcauaugcaggguauccaauuccgcgaaaggaaugccggcccacaaaucgacagaaauaugaaggaugagggcuuuaacaucaccgccggcguggacgaggagacugguuucgucuacggcggcaaucgguucaauugcgggaccuggauggacaagaugggcgaaagcgaccgggccagaaaccggggcauuccggcuaccccccgcgauggcucggccguggaaaucgugggccucuccaagucugccgugcgguggcuuuuggagcucuccaagaaaaacaucuucccguaccacgaagugaccgugaagagacacgggaaggccaucaaaguguccuacgacgaauggaaccggaagauccaggacaacuucgaaaagcuguuccacguguccgaggaucccuccgacuugaacgaaaagcaccccaaccucgugcacaagcgcggcaucuacaaggauuccuacggagcguccucaccuuggugcgacuaucagcugaggcccaacuucaccaucgcaauggugguggccccugaguuguucaccacugagaaggcuuggaaggcccuugagaucgccgaaaagaagcugcucggcccgcuggggaugaaaacccucgaccccgaugacaugguguacugcgggauauacgacaaugcacuagacaacgacaacuacaaccuggccaagggcuucaauuaccaucagggcccggaguggcuuuggccuaucggcuacuuccugcgggccaagcuguacuucucacggcuuaugggaccggagacuacugcaaagaccauugugcuugugaagaacgugcuuucgcgccacuacgugcaucuggaacggagccccuggaaggggcuccccgagcugaccaacgagaacgcccaguacugucccuucuccugugaaacccaggcuugguccauugccaccauucuggaaacccuguacgaccucuag

SEQ ID NO: 15 - RNA, 4599 nt, Artificial Sequence
  Codon-Optimized AGL Coding Sequence
augggacacucaaagcaaauucggauccuccugcucaacgagauggaaaagcucgagaaaacccucuuucgccuggagcaggguuaugagcuccaguuccgccuggguccgacccuccaagggaaggccgucacuguguacacuaacuauccauuccccggagagacuuucaaccgggaaaaguuccgcagccucgauugggagaacccuacugaacgggaggacgauucggacaaguacuguaaacugaaccuccagcagagcggcucauuucaauacuacuuucugcaagggaacgagaaguccggagggggguacaucgucguggauccuauccuucgcgugggcgccgacaaccaugugcugccguuggacugcgugacccugcaaaccuuccucgccaaaugccucggaccuuucgaugagugggaauccaggcugagaguggccaaggaaucgggguacaacaugauucacuucaccccucuccaaacccugggccugucucggagcugcuacucccuggccaaccagcuggagcugaaucccgacuucucccggcccaaccggaaguacacuuggaaugacgugggccaacugguggagaagcucaagaaggaguggaacgugaucugcauuaccgacgugguguacaaccauaccgccgccaacuccaaguggauccaggaacacccagaaugugccuacaaccucgucaacucaccccaccugaaaccagcaugggugcuggaucgcgcccucuggcgguucucgugugacguggccgaaggaaaguacaaagagaagggcaucccugcccugaucgaaaaugaccaccacaugaauuccauuagaaagaucauuugggaggacauuuucccuaaguugaagcucugggaguucuuccaaguggacgucaacaaggccguggaacaguuucgccggcuccugacccaagaaaaccgccgcgugaccaaguccgacccuaaccagcaccugaccauaauccaggacccugaguacagacgguucgguugcacugucgacaugaacaucgccuugacuacuuucaucccgcacgacaaggguccugccgccauugaggagugcugcaacugguuccacaagcggauggaagaacugaacuccgaaaagcaccgccucaucaacuaccaccaggagcaggccgugaacugccugcuggggaacguauucuacgagaggcuggccggacacggacccaagcugggacccgugaccagaaagcauccucucgucacccgcuacuuuacuuucccguuugaagagaucgacuucucaauggaagagucgaugauccaucucccuaacaaggccugcuuccugauggcccacaacggcugggugaugggcgacgauccucugagaaacuucgcugagcccgguucggaaguguaccuuagacgggaacuuauuugcuggggcgauuccgugaaguuacgcuacggaaacaagccugaggacugcccuuaccugugggcccauaugaagaaguacaccgagauuaccgccaccuacuuccaagggguccggcuggacaacugccacucaacuccucugcacguggcugaguacaugcuggaugcggcccggaauuugcagccuaaccuuuacguggucgccgaacucuuuaccggguccgaggaccuggacaacguguucgugacucggcucggaaucuccucacugauuagagaggccauguccgcauacaacucgcacgaagaaggccggcuggucuaucgauacggcggcgaaccugucggaagcuucguccagcccugccugcggccgcugaugccagcgaucgcccacgcccucuucauggacaucacccaugacaacgaaugucccaucgugcaccgcuccgccuacgaugccuugccaagcaccaccaucguguccauggcgugcugcgccagcgguagcacuaggggcuacgaugaacuugugccgcaccagaucagcgugguguccgaggaaagguuuuacacgaaguggaaccccgaagcccugcccuccaacacuggggaagugaacuuccaguccgggaucauugcggcccgcugcgcgaucucgaagcuccaccaggaacucggcgcgaaaggauucauucaaguuuacguggaccaggucgacgaggacaucgucgccgugacucgccacuccccuucaauccaucaauccgugguggcggugucgcggaccgcuuuccggaacccuaagacuucguucuacucgaaagaagugccucagauguguauccccggaaagaucgaggaaguggugcucgaggccaggacuauugagaggaauaccaagccuuaccggaaggaugagaacuccauuaacgguacuccugacaucaccgucgagauccgggaacacauccagcucaacgaaagcaaaaucgugaagcaggccggcguggccacuaaggguccgaacgaguacauccaggaaaucgaauuugagaaccugucgcccggaagcgugauuauuuuucgggugucccuggacccgcacgcccaagucgccguggguauccugcgcaaucaucugacucaguucagcccucacuucaaguccggcagccuugccguggacaacgccgauccgauccugaagaucccauucgccucacucgccucacggcucacacuggccgaacucaaucagauccucuaucgcugugaauccgaagagaaggaggacggcggagguugcuacgauauuccgaauugguccgcacugaaauacgccggacugcagggccucauguccguguuggccgaaauccgcccuaagaacgaccucggccacccguucugcaacaaccucagaucuggagacuggaugaucgauuacgugucaaaccgccugaucucgagguccggcacuaucgccgaagucggaaaguggcuccaagcaauguucuucuaccugaagcagaucccucgcuaccugauaccuuguuacuucgacgccauccucauuggcgccuacacuacucugcuggauacugccuggaagcaaaugagcagcuucgugcagaacggaagcacuuucgucaagcaucugucgcucgggagcgugcagcugugcggcgucggaaaguuuccuucccugcccauucuguccccugcccucauggaugugccguaccgccuuaacgagaucacuaaggagaaggagcaguguugcgugagccuggcugccgggcucccucacuucucguccggaaucuucagaugcuggggccgcgacaccuucauugcccugcgagggauccuguugauuacuggccgcuacguggaggccaggaauaucauucucgccuucgcgggaacccugcggcacggccugaucccuaaccuccugggagaaggaaucuaugcgagauauaacugcagggacgccguguggugguggcuccagugcauccaggacuacugcaagauggugcccaacgggcuggacauccucaagugccccgugucacggauguacccaacugaugacagugcuccucugccggccgguacucucgaccagccacucuuugaagucauccaggaggccaugcagaagcacaugcagggcauucaauuccgggagaggaacgccggaccucagauugaccggaacaugaaggacgaggguuucaauaucacugccggcguggacgaagaaaccggcuucgucuacggaggaaacagauucaacugcggaaccuggauggauaagaugggagaaagcgacagagcgcggaacagggguaucccugccacuccccgggacggaucggccguggaaauugugggacuuuccaaguccgccgugcgguggcuccuggagcuuuccaagaagaacaucuucccuuaccaugaagugaccgugaagcggcacgggaaggccaucaaagucuccuacgaugaauggaaccgcaagauucaggacaauuucgagaagcuguuccaugucuccgaggacccuucugaccugaaugagaagcaucccaaccuggugcacaagagaggcaucuacaaggacagcuacggagcuuccuccccuuggugcgauuaccagcuccggccaaacuucacuaucgccauggugguggcgccugaacuguucaccacugaaaaggccuggaaggcgcucgaaaucgcggagaagaagcugcucgggccucucgggaugaaaacccucgacccugaugauaugguguacugcggaaucuacgauaacgcccuagacaacgacaacuacaaccuggccaagggauucaacuaccaucaggggcccgagugguuguggccuauuggcuacuuccugagagccaagcucuacuucucccgccucaugggccccgaaaccacugccaagaccaucgugcucgugaagaacgugcucucccggcacuaugugcaccuugagcgcucgccauggaagggacugcccgaacugacuaacgagaacgcccaguacugccccuucuccugugaaacucaggccugguccaucgccacaauuuuggaaacccucuacgaucuguag

SEQ ID NO: 16 - RNA, 4599 nt, Artificial Sequence
  Codon-Optimized AGL Coding Sequence
augggacauucaaagcaaauccggauucuguuacuuaaugagauggagaaguuggagaaaacauuguuuagacucgagcagggcuacgaacugcaguuucgccugggcccuacacuacaagggaaagccgucaccgucuauacaaacuaucccuuccccggcgaaacguuuaaucgggagaaguucagaucucuggauugggagaaccccaccgaacgggaggaugauagcgacaaguauugcaaacugaacuugcagcagucuggcaguuuucaguauuauuuucugcaagggaacgagaaguccggcggcggcuauauaguggucgaccccauccuucgugugggagcugacaaccauguguugccccuggacuguguuacacugcaaaccuuucuggcuaagugucucgguccuuuugaugaaugggaaucgcggcucaggguggcaaaagaauccggcuauaacaugauucauuuuacaccccugcaaacccugggccucucaaggaguuguuacagccuugccaaucagcuggagcugaaccccgacuuuucccgucccaaccggaaguauacuuggaacgacgugggccagcucguagaaaagcugaaaaaggaguggaacgugaucuguauaaccgauguggucuauaaccacaccgccgccaauucgaaguggauccaggagcaucccgagugugcuuacaaccucgugaacagcccccaucuuaagcccgcuuggguacuugaccgcgcacuuuggagguuuuccugugacguggcugaggggaaguauaaggaaaagggcauccccgcccugaucgaaaacgaccaucacaugaacaguauacggaagaucauuugggaggauauuuuucccaaacugaagcugugggaguuuuuucaaguggaugugaacaaggcugucgaacaguuuaggaggcugcugacccaagaaaauagacgcgugacuaagagcgacccaaaucagcauuugacaauuauacaggaccccgaauaucgccgauucggcuguaccguggauaugaauaucgcauugacuacuuucaucccccacgacaagggccccgccgcuauugaggaaugcuguaauugguuucauaagcgaauggaggagcugaacucugagaagcacaggcugauuaacuaucaucaggaacaggccguuaacuguuugcugggcaacguguuuuaugaacggcuugccggccauggcccgaaguugggcccgguuacaagaaagcauccacuugugacccgcuacuucaccuuuccguucgaagaaauugacuuuagcauggaggagucaaugauccaccuccccaacaaggcuugcuuucuuauggcucacaacggcugggugaugggcgacgacccccugcggaacuuugcggaaccgggcucagaggucuaucuaagaagggaacugauuugcuggggcgacuccgugaagcugagauacgggaacaagccugaggauugccccuaccucugggcucacaugaaaaaguauacagaaauuacugcuacguauuuccaaggcguacggcuugacaacugucacuccaccccacugcaugucgccgaguauauguuagaugcugcucgaaacuugcagcccaauuuguauguggucgcugaacuguuuacggggagugaagaucucgacaacgucuuuguaacccgacugggcaucagcucgcuaauucgggaggccauguccgcuuacaacucccaugaggaaggccgccuuguauaucguuauggcggcgaacccguggggagcuuuguucaaccgugucuacgcccccugaugcccgccaucgcucaugcccuauucauggauaucacucaugacaaugaguguccuauugugcauaggagugcuuaugacgcccucccaagcacaacgaucguguccauggcuuguugugcuaguggcuccacaagaggcuaugacgaacuggugccccaucaaaucuccguagugucugaagagagauuuuacaccaaguggaaccccgaggcucucccuucaaacacuggagagguuaacuuucaauccgggauuauugcugcuagaugugcuaucagcaagcuccaucaggaacugggcgcaaagggcuucauucaaguuuauguagaccagguugacgaggacauaguugcaguaacucggcauuccccuucgauacaucagucugucguggccguguccaggacagcauuucgcaaucccaagacuagcuuuuacuccaaagaaguaccacaaauguguauccccgggaagaucgaggaagugguacuggaagcccggacuauugagagaaacaccaagccguaucggaaggacgagaauucuaucaacggcacaccugauauaacaguggaaauacgcgaacacauucaguugaaugaguccaagaucgugaagcaggccggcgucgccaccaagggccccaacgaguauauccaggagaucgaauuugaaaaccugagccccggcucuguuauuauauuucggguuucauuagauccucaugcucaaguggcuguaggcauccuccggaaucaucugacucaguucucuccccacuucaagagcggcagccuggcugucgauaaugccgaccccauacuuaagauucccuuugcuucccuggcuucaaggcugacccuggcugaacuuaaucaaauccuauaccgaugcgaaagcgaagagaaggaagauggcggcggcuguuacgauaucccgaacuggagcgcacugaaauaugcuggcuuacaaggccucaugaguguguuggcugagauuagacccaagaaugacuugggccauccauuuuguaacaaccugagaagcggcgacuggaugaucgauuacgugucuaaccgacucaucucccgaagcggcaccauugcugagguuggcaaauggcugcaggcuauguucuuuuaucugaaacagauuccucgguaccugauucccuguuauuucgacgcuauucugauuggcgcauauaccacgcucuuggacacugcauggaagcaaaugagcucuuuuguccaaaauggcuccacuuuuguuaaacaucugaguuugggcagcgugcaguuauguggcguuggcaaauuuccaagccugcccauacugucccccgcucugauggacguccccuaccgacugaacgagaucaccaaggaaaaggaacagugcugugugucuuuagcugccggcuugccgcauuuuucaagcggcauuuuccgguguuggggucgggacaccuucaucgcacugagaggcauucugcugaucacuggccgcuauguggaagcuaggaauaucauuuuagccuuugcggguacccuucggcacgggcugauccccaaucuuuugggcgaaggcaucuacgcacguuacaauugccgggaugccguauggugguggcuccaauguauccaggacuauugcaagaugguucccaacggccucgauauccugaagugccccgugucaaggauguauccuaccgaugacagugcuccccuuccugcuggcacccuggaucagccgcucuuugaaguuauucaggaagcaaugcaaaagcauaugcagggcauccaguuucgggaaagaaacgcuggcccgcaaauagacaggaacaugaaggaugaaggcuucaauauuacugcuggcguagacgaagagacaggguucgucuacggcggcaauagguuuaacuguggcacuuggauggacaagaugggcgaaucugaccgcgcgaggaacagaggcaucccagcaacaccgagggacggcagcgcuguggagauugugggccugucuaagucugccgugcgcuggcuacucgaacuguccaagaagaauaucuuucccuaucaugaagucaccguaaagcggcauggcaaagcuauuaagguuuccuaugacgaguggaacaggaagauucaggacaauuuugagaagcuguuccaugugucggaggacccuagcgaucucaacgagaagcaccccaacuuaguacauaagaggggcaucuauaaggauagcuauggcgcuagcagcccuuggugugacuaucagcuccgucccaacuuuaccauugcuaugguaguggcgcccgaguuguuuaccacugagaaggcuuggaaggcucuugaaauagccgagaagaaauugcugggcccccugggcaugaaaacucuggaucccgaugacaugguauacuguggcaucuaugacaaugcccuggacaaugacaauuacaaucuggccaaggguuuuaacuaucaccagggcccugaauggcuguggccuauuggcuauuuucuucgcgccaagcuauauuuuaguaggcugauggguccagaaacaacugcaaagacaauugugcucgugaagaacgugcuuucccggcacuaugugcaucuggaaaggaguccauggaagggcuugccggaauugacuaacgagaacgcccaguauugucccuuuucuugugaaacucaggccugguccauugcuacuauucuggagacucuauaugacuuguag

SEQ ID NO: 17 - RNA, 4599 nt, Artificial Sequence
  Codon-Optimized AGL Coding Sequence
augggccauuccaagcaaauucgaauucugcugcugaacgaaauggaaaaguuggaaaagacauuguuccgucuggagcagggcuaugagcugcaguuuaggcuuggcccgacguugcagggcaaagccgugaccguauauacuaacuaucccuucccuggcgaaacguuuaaccgggagaaguuucgcucacuggacugggagaaucccacggaaagggaggacgauagcgauaaguacuguaaacugaaucugcaacagucuggcucuuuccaauauuauuuucugcaagggaacgagaaguccgggggcggcuauauuguaguggaccccaucuugagagugggcgcugacaaccauguauuaccccuugauugcgugacgcugcagaccuuucuggcuaaguguuugggcccuuucgaugagugggaaagccggcugaggguggccaaggagagcggcuauaauaugauucauuuuaccccuuugcaaacucuggggcucucuaggagcuguuauuccuuggcuaaucagcuggaacugaaccccgauuuuagccggcccaaccgaaaguauacauggaaugacguugggcaauugguugagaagcugaagaaggaauggaauguuauauguauaacagacgugguguauaaccauaccgcugcuaauucgaaauggauucaggaacauccugagugcgccuacaaccucguaaauaguccucaucugaagccggcuugggugcuggacagggcucucuggagguuuagcugugauguggccgaagggaaguauaaggagaaggguaucccggcucugauugagaacgaccaccauaugaacaguauaaggaagauaaucugggaggacauuuuucccaaacugaagcugugggaauucuuucaaguggacgugaacaaggccguugagcaguuuagacgcuugcugacacaagagaaccgaagggucaccaagagugacccuaaccagcaucuuacaauuauccaagaccccgaguaucgucgguuuggcuguacuguggacaugaacauugcucugaccaccuuuauaccccacgauaagggccccgcugcuaucgaagaguguuguaacugguuccacaagaggauggaagaguugaacucugaaaagcaucggcugauuaacuaucaucaggaacaggcugugaacugccugcucggcaacguauucuacgagagauuggcuggccauggaccuaagcugggcccgguuacgagaaagcauccccugguuacgcgguauuucaccuucccguuugaggagauugauuuuagcauggaagaauccaugauccaccuccccaacaaggcuugcuuccugauggcacauaacggauggguuaugggcgacgacccccugaggaauuuugcugaacccggcuccgaagucuaucugagaagggaacugaucuguuggggcgacuccgucaaguugcgcuauggcaauaagccugaggacuguccauaucugugggcucacaugaagaaguacacagagaucaccgcuacauacuuucagggcgucaggcucgacaauugucacuccacaccccugcacguggcugaguauaugcuggaugccgcuaggaaucuccagccuaaccuauauguggucgcugaacuguucaccggcucugaggaucuggauaauguguuugugacacgccugggcaucagcucccugauccgcgaggcuaugagugccuacaauagucacgaggaaggccggcuuguguaccgcuauggcggcgaacccgugggcagcuuuguacaaccuugucugcggccucugaugcccgcuauugcucacgcuuuguuuauggacaucacccaugacaacgaaugucccauuguacaccggucugcuuacgacgcucugcccuccacaacuauugucaguauggcuuguugugcaucuggcucaacucggggcuacgacgaauuaguuccgcaucaaaucucuguaguguccgaagaacgguuuuauacaaaauggaaccccgaagcgcugcccuccaauaccggcgaagugaacuuucagucugggaucaucgccgcuagaugugcuauuucuaaacugcaucaggaacugggcgcuaagggcuuuauucaaguauauguggaccaggucgacgaggacaucguagcuguaacccggcacagccccagcauacaucagagugucguggcugugucuagaacagcuuuuaggaacccaaagaccucuuuuuacuccaaagagguuccacagauguguaucccgggcaaaauugaggaaguggucuuggaggccaggacaauugagcguaauacgaagcccuauagaaaggaugagaauagcaucaacggcacuccugauaucacuguggaaauccgggagcauauacaguugaacgagucuaagaucguuaagcaggcugguguagcuaccaagggucccaaugaguauauucaggaaauugaguuugaaaaccuguccccgggcagcguaauuaucuuuagagucagucucgacccccaugcucaaguggcaguggggauccugcggaaccauuugacucaguucuccccccauuuuaagucuggcagucuggccguugacaacgcugaccccauauugaagauucccuuugcuucccuggcuucacgguugacccuggccgaacugaaccagauuuuauaucgcugcgaguccgaggaaaaggaggauggcggcggcuguuaugacauucccaacuggucugcucuaaaauacgcugggcugcagggucugaugagugugcuggcugaaauucgccccaagaacgaccugggccauccauuuugcaacaaucugcgcaguggcgacuggaugauugauuauguguccaaccggcugauuagucggagcggcacgaucgcagaagucggcaaauggcuccaggcuauguuuuuuuaccuaaagcagauacccagauaccugaucccuuguuauuuugacgcuauacugauuggcgcuuacacaaccuugcuggacaccgccuggaagcagaugagcagcuuuguccaaaauggcagcacauucgugaagcauuugucucugggcagugugcagcuguguggcgugggcaaauuuccaaguuugccgauccugucucccgcuuugauggaugugccauaucgacugaacgagauaaccaaggaaaaggaacaguguuguguuucacucgcugcuggcuugccccauuuuuccucuggcauuuuccgauguugggggagggacacauucauugcccugcgugggauccugcugauuaccggccgcuacguugaggcuagaaacauuauuuuggcuuucgccggcacauugagacauggucugauacccaaucugcugggcgaaggcauauaugcuagguauaacugucgcgacgcaguguggugguggcugcaaugcauccaggauuauugcaagaugguuccuaacggccuagacauccugaagugcccagugucccggauguauccaaccgaugauucagcuccccugcccgccgguacacuggaccaaccccuguucgaaguuauucaagaagccaugcagaagcacaugcaggguauccaguuucgagagaggaaugcaggcccccaaauugaccggaacaugaaggaugaaggcuucaacauuacugcuggcgucgacgaagaaacaggguuuguguacggcggcaaccgguuuaacugcggcacauggauggacaagaugggcgaaagcgaucgcgcacggaaccggggcauccccgccacgccgcgugauggcucugcuguggagaucgucggccucagcaaauccgcuguccgauggcuguuagagcugucgaagaagaacaucuuucccuaccaugagguuaccguuaagagacacggcaaagcuaucaaagugucuuaugacgaauggaauagaaagauucaagacaacuucgagaaacuguuucauguguccgaggaucccagcgaccucaacgaaaagcaucccaaucucguacauaagaggggcaucuauaaggacucauauggcgcaucaaguccuuggugcgacuaucagcuucggcccaauuucacgaucgcaauggucguggcacccgagcuguuuacuacggagaaggcuuggaaggcucuggaaaucgcugagaagaagcugcugggccccuugggcaugaaaacccuggaucccgacgacaugguauacuguggcauauaugacaacgcucuggauaacgauaacuauaauuuggcuaaaggcuuuaauuaucaccagggcccagaauggcuauggcccauuggcuacuuucugcgagcuaagcuauauuuuucucgccugaugggcccugaaaccaccgcuaagacuaucgugcucgucaagaacguacugaguaggcauuacgugcacuuggagcgcagcccauggaagggcuugccggaacugacgaacgaaaacgcucaguauuguccguuuucuugugaaacacaggcuuggaguauugcuacuauccuggaaacucuguacgaucuguag

SEQ ID NO: 18 - RNA, 4599 nt, Artificial Sequence
  Codon-Optimized AGL Coding Sequence
augggucauuccaaacaaauuaggauccugcuguugaacgaaauggaaaagcucgaaaagaccuuauuucgccuggagcagggcuaugaguugcaguuucggcugggaccaacucugcaaggaaaggcuguaaccguguacacaaauuauccuuuucccggcgaaacguuuaacagggagaaguuucgaucucuggauugggagaaccccacugaaagggaggacgauagcgacaaguauugcaaacugaaucugcaacaguccggcagcuuucaauauuauuuucugcaagggaacgaaaagagcggcgggggcuauauuguaguagacccuauacugagagucggagcugacaaccauguucugcccuuggacugcgugacacugcagaccuuuuuggcuaagugucugggccccuuugaugaaugggagagucggcuccguguggcuaaggagagcggguacaauaugauucacuuuaccccccugcaaacuuugggacuuucccggagcuguuauagccuggcaaaccagcuggaguugaauccugacuuuucccgcccaaauaggaaguauaccuggaacgacgugggccaacugguggagaagcugaagaaggaguggaacgugaucugcauuaccgacgucguguauaaucauaccgccgccaacuccaaguggauacaggaacauccugagugugcuuacaaccucguaaacuccccgcaucugaagccagcuuggguucuggauagagcuuuguggcgguucagcugugacgucgcugagggaaaguacaaggaaaaagggauuccugcucucaucgagaaugaccaccacaugaacaguauuaggaagauuaucugggaggacaucuucccgaagcuaaagcugugggaauucuuccaaguggacgugaacaaggccguggagcaguuccgacggcuguuaacucaagagaaccguagggucacaaaaucggauccuaaccagcaccugaccauuauccaagacccggaauaucggcgguucggcuguacuguggacaugaacauugcuuugacaacuuucauuccccacgacaaggguccagcagcuaucgaggaauguuguaauugguuucauaagcggauggaggaacucaacuccgagaagcauaggcugauuaauuaucaucaggaacaggcugugaauugucuguugggcaauguuuucuacgaacggcuggcuggccauggccccaaacucggaccuguuacaaggaagcauccacugguuacccgauacuuuaccuuuccauuugaagaaauugauuuuagcauggaagaauccaugauccaucuaccuaacaaggccuguuuucugauggcccauaacggcuggguuaugggagaugaucccuugcggaacuuugcugaacccggaucugaaguauaucugcggagagaguugauuuguuggggcgacuccguaaagcugcgcuauggcaacaagccagaggacugucccuauuugugggcucauaugaagaaguauaccgagaucaccgcuacguauuuucaaggcgucaggcucgauaauugucauuccacuccgcugcauguugcugaguauauguuggacgcugcucgaaaucugcagcccaauuuguauguuguggccgagcuguuuaccggcuccgaggaccucgauaacguguucgucacgcgacuaggcaucagcagcuugauccgggaagccauguccgcuuauaacucccacgaggagggccgacuggucuaccgcuauggcggcgaaccagugggcaguuuuguacagccuugucugaggccccucaugcccgcuauugcucaugcucuguucauggacauuacucaugauaacgagugcccuauagugcaucgguccgccuacgacgcccugccgagcacuacaauaguguccauggcuuguugugcaagcgggagcacccgcggcuaugacgagcuggugccgcaucaaauaucuguagucagcgaagaaagguuuuauaccaaguggaacccggaagcuuuaccuuccaauacuggggaagugaacuuucagagcggcauuaucgcugcgagaugugcuauauccaaguugcaucaggaacugggggcaaagggguuuauucaaguauauguagaccagguugacgaagauauaguggcugugacacgccacagcccaagcauccaccaguccgugguggcugucagccggacugcuuuucgcaacccaaagacaagcuuuuauagcaaagaagugccgcagaugugcauucccggcaaaauugaggaggucgugcuggaggcuaggacuaucgaaaggaacaccaagccguacaggaaggacgagaauuccaucaacgggacuccagauauuacaguugagauccgggaacauauucaguugaaugagucgaagauuguuaagcaggcuggcguagcuacaaaggggccaaacgaguauauucaagagauagaauucgaaaaccugagccccgguuccgugaucauuuuucgagugucccuggauccucaugcucaaguggccguuggcauucugagaaaccaucucacacaauuuuccccucacuuuaaaaguggcagccuggcuguggacaacgccgauccgauccugaagauuccauucgcuucccuggcuagucgccugacacuggcugaacuaaaccagauucuuuaccgcugugaaucugaagagaaggaggacggcggcgguugcuaugacaucccaaauuggagcgcucugaaauacgcugggcugcagggccucaugagcguacuggcagaaaucagacccaagaacgaccugggccaccccuucuguaacaaccugagguccggcgauuggaugaucgacuaugugucgaacagacucaucucaagaagcggcacuauagcugaggucggcaaaugguugcaggcuauguucuuuuaucugaagcaaauuccgcgguaucugaucccgugcuauuuugacgcuauauugaucggcgcuuauacgacuuugcuggacacagccuggaagcagauguccagcuucgugcagaacggcagcacuuuugugaagcaccugagucugggcucaguacagcuguguggcgugggcaaauuccccagccuaccaauucugucccccgcucugauggauguucccuaucggcugaacgagauuaccaaggaaaaggagcaauguugcgugagccuggcagccggccugccccacuuuucuuccggcauuuuucgcuguuggggucgggacaccuucauugcacugcggggcauccuguuaaucaccggccgcuauguggaagcuagaaauauuaucuuggcuuuugcuggcacucugcgacacggccugauccccaaccuucugggcgaaggcaucuaugcucgcuacaauugucgcgacgccgucuggugguggcugcaguguauacaggacuauugcaagauggugccaaauggccuggacauccuuaaauguccaguuucccggauguacccaacugacgacagcgcuccuuugccugccggcacacuggaucagccgcuguuugaagugauccaggaagcuaugcagaagcauaugcagggcauucaguuucgggaacgaaaugcuggcccacaaauugacagaaacaugaaggaugaggguuuuaacauuacugcuggcgucgaugaagagacaggguuuguguacggcggcaacagguucaacugcggcacauggauggacaagaugggcgaaucugaccgugcuaggaacaggggaauccccgcuaccccccgggacggcagcgcuguggaaaucguaggccuguccaaguccgccguucgcuggcuucuggagcugagcaagaaaaacaucuuucccuaucacgaggucacagugaagagacauggcaaagcuaucaaagucucuuacgaugaguggaauagaaagauucaagauaacuuugaaaaguuguuccacguuucggaggaccccagcgaucugaaugagaagcaucccaacuuggugcacaagaggggcauauacaaggacucuuauggugcuagcagcccuuggugcgacuaucagcugaggcccaacuuuacuaucgccauggugguggcaccggaacuguuuacaacggagaaggcuuggaaggcucuggaaauugcugagaagaaguugcuggggccccuggggaugaaaacgcuggauccagacgacauggucuacuguggcauauaugauaaugcucuggauaacgauaauuacaaucuggcuaaggguuucaacuaucaucaggggccagaguggcucuggccuauuggcuauuuccuccgugcuaagcuguacuuuucucgccugauggggccagaaacuaccgcaaagaccauuguauuggucaagaacgugcugagccggcauuauguacauuuggaacgguccccuuggaaaggccugcccgaacucacuaacgagaacgcucaguauuguccguuuuccugcgaaacccaggcuugguccaucgcaacuauuuuggaaacccuguacgaccuguag

SEQ ID NO: 19 - RNA, 4599 nt, Artificial Sequence
  Codon-Optimized AGL Coding Sequence
augggccacagcaagcaaaucagaauccuccugcucaacgagauggaaaagcucgaaaagacccuguucagacuggagcagggauacgagcugcaguuccgccucggaccaacccuccaagggaaggccgugaccguguacaccaacuacccauucccgggagaaaccuucaaccgggaaaaguucaggagccuggacugggaaaaccccaccgagagagaggacgacagcgacaaauacugcaagcugaaccuccaacagagcggcagcuuccaguacuacuuccuccaaggaaacgaaaagagcgggggcggcuacaucgugguggacccaauccugcgggucggggcagacaaccacgugcugccacuggacugcgugacacugcagaccuuccuggccaagugccugggaccguucgacgaaugggagagccggcugcggguggccaaggagagcggcuacaacaugauccacuucacaccgcuccaaacccucggccugagcagaagcugcuacagccuagccaaccagcuggagcucaacccggacuucagcaggcccaacagaaaguacaccuggaacgacgugggacagcucguggaaaagcugaaaaaggaauggaacgugaucugcaucaccgacgugguguacaaccacaccgccgccaacagcaaauggauccaggaacacccggaaugcgcguacaaccucgugaacagcccccaccugaagccggccuggguacuggacagggcacuguggcgcuucagcugcgacguggccgaaggaaaguacaaggagaagggcauccccgcccugaucgagaacgaccaccacaugaacagcauccggaagaucaucugggaggacaucuucccaaagcugaagcugugggaguucuuccaagucgacgugaacaaggccguggaacaguucagacgccugcugacgcaggagaaccggagggucaccaagagcgaccccaaccagcaccugaccaucauccaagacccggaauaccggagauucggaugcaccguggacaugaacaucgcccugaccaccuucaucccacacgacaaggggcccgcagccaucgaggagugcugcaacugguuccacaagagaauggaggaacugaacagcgaaaagcaccgccucaucaacuaccaccaggaacaggccgugaacugccuccucggaaacguguucuacgagcggcuggccggccacgggcccaagcugggccccgugacccgcaagcacccgcucgugacgcgguacuucaccuucccguucgaagaaaucgacuucagcauggaggagagcaugauccaccucccgaacaaggccugcuuccucauggcccacaacggcugggucaugggcgacgacccgcugcggaacuucgcagagcccggaagcgaaguguaccucagaagggagcugaucugcuggggagacagcgugaagcugcgcuacggaaacaagcccgaggacugcccguaccugugggcgcacaugaagaaguacaccgagaucaccgccaccuacuuccaaggagugcggcuggacaacugccacagcaccccgcugcacguggccgaguacaugcuggacgccgccagaaaccuccagcccaaccucuacgugguggcagagcuguucaccgggagcgaggaccucgacaacguguucgugacccgacucggcaucagcagccugauccgggaagcaaugagcgccuacaacagccacgaggaagggaggcugguguacagauacggaggagaacccgugggcagcuucgugcagccgugccugaggccccugaugccagccaucgcgcacgcgcuguucauggacaucacccacgacaacgaaugcccgaucgugcaccggagcgcauacgacgcccugccgagcaccacgaucgucagcauggccugcugcgccagcggcagcacccgaggauacgacgagcuggugccccaccaaaucagcgucgucagcgaagaacgcuucuacaccaaguggaacccggaagcacugccgagcaacaccggagaagugaacuuccagagcggaaucaucgccgcgcgcugcgcgaucagcaaacugcaccaggaacugggagccaagggguucauccaggucuacgucgaccaaguggacgaggacaucguggcagugacccgccacagccccagcauccaccaaagcgugguggccgugagccggacagcguuccggaaccccaagacgagcuucuacagcaaagaggugccccagaugugcaucccgggaaagaucgaggaaguggugcucgaagcgcgcaccaucgaacgcaacaccaaaccguaccgcaaggacgaaaacagcauaaacgggacccccgacaucaccguggagaucagggaacacauccagcugaacgagagcaagaucgugaagcaggccggggucgccaccaagggcccgaacgaguacauccaggagaucgaguucgagaaccucagccccgggagcgugaucaucuucagagucagccuggacccacacgcccaaguggccgugggcauccuccggaaccaccugacccaguucagcccgcacuucaagagcgggagccucgccguggacaacgccgacccgauccugaagaucccguucgcgagccuggccagccggcucacccuggccgaacugaaccagauccuguaccgcugcgagagcgaagaaaaggaggacggaggagggugcuacgacaucccaaacuggagcgcgcugaaauacgcgggccugcagggccugaugagcgugcuggccgaaauccgccccaagaacgaccugggacacccauucugcaacaaccugaggagcggagacuggaugaucgacuacgucagcaacagacugaucagccgcagcggcaccaucgccgaagucggaaaauggcuccaggccauguucuucuaccugaagcagaucccgcgguaccugaucccgugcuacuucgacgccauccugaucggcgccuacaccacccugcucgacaccgccuggaagcagaugagcagcuucguccaaaacgggagcaccuucgugaagcaccucagccugggcagcgugcagcugugcggggucggaaaauucccgagccugcccauccugagcccggcgcugauggacgugccguacagacugaacgagaucaccaaggaaaaggaacagugcugcgugagccuggccgccggacugccgcacuucagcagcggcaucuuccggugcugggggcgcgacaccuucaucgcccugcggggaauccugcugaucacgggccgcuacguggaggcccggaacaucauccuggccuucgccggcacccugcggcacggacugaucccgaaccuccugggagaggggaucuacgcccgguacaacugccgggacgccguguggugguggcugcagugcauccaggacuacugcaagauggugcccaacggccuggacauccugaagugccccgucagccggauguacccgaccgacgacagcgccccgcuccccgccggaacccucgaccagccacuguucgaagugauccaggaggccaugcaaaagcacaugcagggaauccaguucagagaacggaacgccggaccccagaucgaccggaacaugaaggacgagggauucaacaucaccgccggagucgacgaggaaaccggcuucgucuacggagggaaccgguucaacugcggaacauggauggacaagaugggagagagcgaccgcgccaggaaccgcggaaucccagcaaccccgcgggacgggagcgcaguggaaaucguggggcugagcaaaagcgccgugcgguggcugcucgaacucagcaagaagaacaucuuccccuaccacgaagucaccgugaagagacacggaaaggccaucaaagucagcuacgacgaauggaacaggaagauacaggacaacuucgagaagcuguuccacgucagcgaggacccgagcgaccugaacgagaagcaccccaaccuggugcacaagcgcgggaucuacaaggacagcuacggcgcgagcagcccguggugcgacuaccaacugcgccccaacuucaccaucgccauggucguggcccccgaacucuucacgaccgagaaagcguggaaggcgcuggagaucgcggaaaagaagcuccucggaccccuggggaugaaaacccuggaccccgacgacaugguguacugcggcaucuacgacaacgcgcuggacaacgacaacuacaaccuggccaagggcuucaacuaccaccagggccccgaauggcuauggccgaucggcuacuuccugcgggccaagcuguacuucagccgccucaugggcccagaaaccaccgcaaagaccaucgugcuggucaagaacguccugagccgccacuacgugcaccucgagagaagcccauggaagggacugcccgagcugaccaacgaaaacgcgcaguacugcccguucagcugcgaaacccaggccuggagcaucgccaccauccuggaaacacuguacgaccucuag

SEQ ID NO: 20 - RNA, 4599 nt, Artificial Sequence
  Codon-Optimized AGL Coding Sequence
augggccacagcaaacagauccggauccuccuacucaacgaaauggaaaagcucgaaaagacucuguuccggcuggagcaaggauacgagcuucaguuccgguugggcccgacgcugcaggggaaggccgugacagucuacacuaacuacccauuccccggcgaaaccuucaacagagagaaguucaggucccuggacugggagaaccccacugaacgggaagaugauuccgacaaguacugcaagcugaaccuccagcaauccgguucauuccaguacuauuuccugcaaggaaacgaaaagagcggaggaggcuacauugugguugauccaauccuucgcgugggagccgauaaucaugugcugccgcuggauugcgucacccugcaaaccuuccuggcgaagugccugggcccguucgacgaaugggaaucccgccugcgggucgccaaagaguccggguauaacaugauccacuucaccccacuccaaacucuuggccuguccagauccugcuacucguuggccaaccaguuggagcugaacccggacuucucacggccuaaccggaaguacacuuggaacgacgucggacaacucguggagaagcugaagaaggaauggaaugucaucugcauuacugaugucguguacaaccacacggcggcgaauucaaaguggauccaggagcacccagaaugcgccuacaaccuggucaauuccccucaccugaagccggccugggugcucgaccgggcccuguggcgguuuucgugcgauguggcggagggaaaguacaaggagaaggggauuccggcucucaucgaaaacgaccaccacaugaacuccauccggaaaauuaucugggaggacaucuucccgaaacuuaagcugugggaauucuuccaaguggacgucaacaaggcuguggagcaguuccggagauugcugacacaagaaaaccgccgcgugaccaaauccgauccgaaccagcaccugacuaucauucaagacccggaauaccggagguuuggcugcacuguggacaugaauaucgcgcugaccaccuucaucccgcacgacaagggaccggcagccaucgaagagugcuguaacugguuccauaagaggauggaagaauugaacucugaaaagcaccggcugauuaacuaccaucaggaacaggccgugaacugucuccugggaaacguguucuacgagcggcuggcgggacacggacccaagcucggccccgugacccgcaagcauccucucgugacuagauacuuuacuuucccauucgaggagaucgacuucuccauggaagaaucaaugauccaccucccuaacaaggcuugcuuucugauggcacacaacggcugggugaugggcgaugacccccugaggaacuuugccgagcccggcuccgaaguguaccugaggagagagcugauuugcuggggggacagcgucaagcugcgcuauggaaacaagccggaagauugcccuuaccucugggcccacaugaagaaguacacugagauuacugccaccuacuuucaaggagugcgccuggauaacugccacucaaccccgcugcaugucgcugaguacauguuggacgcagcccggaaucugcaaccgaaccucuacgugguggcggagcuguucaccggcucggaggaucucgacaacguguucgugacucgccugggcaucucaucgcugauccgggaagcaauguccgccuacaacucccaugaggagggucggcugguguaccgcuacggcggagaacccgugggguccuucgugcaaccgugccugcgaccccugaugcccgccaucgcccaugcccucuuuauggauauuacccacgauaacgaaugcccuaucgugcaccgcucagccuaugaugcccuccccuccaccaccaucguguccauggccugcugcgccucggggagcacccgggguuaugacgagcuggugccgcaccagauuucggugguguccgaggagagauucuacaccaaguggaacccagaagcucugccgucaaacacuggagagguuaacuuucaguccgguauuaucgccgcuagaugugcuauuagcaaacugcaccaagagcugggcgccaaggguuucauccaagucuacgucgaucaggucgacgaggacaucguggcugucacuaggcacucaccuagcauccaccagagcgugguggccgugagccgcacugccuuccgcaacccaaagaccagcuuuuacuccaaggaggucccucagaugugcauuccuggaaagaucgaagaagugguccuggaagcccggaccaucgaacgcaacaccaagccuuaccggaaggacgaaaacucgaucaacgguaccccggauauuacuguggagauucgcgaacacauccagcucaaugaguccaagaucgugaagcaggccggaguggcaaccaaggggccgaacgaguacauccaggagaucgaauucgagaaucucagcccuggcagcgugaucaucuuccgagugucguuggacccacaugcucaggucgccgugggcauccugaggaaccaccugacccaguuuuccccgcauuucaaguccgguucgcuggccguggacaacgcagauccgauccugaagauccccuucgccuccuuggcuucgcgccucacgcuggccgagcugaaccagauccuguauagaugcgaauccgaagaaaaggaagauggaggcgguuguuacgacaucccgaacugguccgccuugaaauacgccggacugcagggauugauguccgugcuggccgaaauuagaccgaagaacgaccuggggcacccguucugcaacaaccuccggucgggggacuggaugauugauuacgugucgaaccgccucaucucccgguccgguacuauugcggaggucggcaaauggcuccaggccauguucuucuacuugaagcaaaucccccgcuaccugauccccugcuacuucgacgccauccugaucggagccuacaccacccugcuggacaccgcguggaagcagaugucuagcuucguccagaacggcuccaccuucgugaagcaccugucacugggcucagugcagcugugcggaguuggaaaguuccccagccugccuauccuguccccggccuugauggacgugccguacagacugaacgaaaucacuaaggagaaggagcaguguugcgugucguuggcggccgggcugccccacuuuucaagcgggauuuuccggugcuggggaagggacaccuucaucgcgcugcggggaauccugcugauuaccggacgcuacguggaggcucggaacaucauucucgcguucgccggcacccugcgccauggacugaucccuaaucugcuuggagagggcaucuacgcucgguacaacugcagagaugccguguggugguggcuccaaugcauccaggauuacugcaagauggugccuaacggucuggacauucugaagugcccugugucccgcauguaccccaccgacgacuccgccccccugccugccggaacccucgaccagccucuguucgaagucauccaagaggccaugcagaagcauaugcagggcauucaguuccgcgaacggaacgcagggccccagaucgaccggaacaugaaggaugaaggguucaacaucaccgccggaguggaugaagagacuggauuugucuacggaggaaaccgcuuuaacugcgggaccuggauggacaagaugggagagucagacagggccagaaauagaggaauccccgcgaccccgcgcgacggauccgccguggagauugugggccugucaaagagcgccguccgcuggcugcuggaacuuagcaagaagaacaucuucccuuaccacgaagugaccgugaaaagacauggcaaagccaucaaagucuccuacgacgaguggaaccgcaagauucaggacaacuucgaaaagcuguuccacguguccgaagaucccuccgaucugaacgagaagcauccgaaccugguccauaagcggggaaucuacaaggauagcuacggugccagcucgccguggugugacuaccagcugcggccaaauuucacgauugcgauggucgucgccccugaguuguucaccacugagaaggccuggaaagcccuggaaauagccgagaagaaauuacuggggccacugggcaugaaaacucucgacccugacgacaugguguacuguggaaucuacgacaacgcacuggacaacgauaacuacaauuuggccaagggauucaacuaccaccaggggcccgaauggcuguggccuaucggauacuuccuucgggcaaagcuuuacuucucccgccugaugggaccugaaacuacugccaagaccauugugcuugugaagaacgugcucucacggcacuacgugcaccuggagagauccccguggaaggggcucccggagcugaccaacgagaacgcccaguacugcccuuucuccugcgaaacccaagccugguccaucgccaccauacuugaaacucuguacgaccuguag

SEQ ID NO: 21 - RNA, 4599 nt, Artificial Sequence
  Codon-Optimized AGL Coding Sequence
augggacacuccaagcagauccgcauucuccuccugaacgaaauggaaaagcuggaaaagaccuuauuucgccuugaacaaggauacgagcugcaguuccggcuuggaccgacccuccaagggaaagcugucaccgucuacaccaacuaccccuucccgggggagacuuucaacagagagaaguucagauccuuggacugggaaaaucccacggaacgggaggacgacuccgauaaguacuguaaacugaaccuccagcagucgggaucguuccaguacuacuuccuacaagggaacgaaaaguccgguggugguuacaucgugguggacccgauccugcgcgugggggccgacaaccacgugcugccgcuggacugcgugacucugcaaaccuuccuggccaagugccucggcccguucgaugaaugggagucgagacugcggguggccaaggaaagcggauacaauaugauucacuuuacuccgcugcaaacccuggggcugucgcgcuccugcuacucgcucgcuaaccagcuggaacugaauccggauuuuagccggccgaaccggaaguauacguggaacgacgucggucagcuggucgagaagcucaagaaggaguggaacgucauuugcaucaccgacguggucuacaaccacaccgcggccaauuccaaguggauccaggaacacccggagugcgccuauaacuuggugaacuccccucauuugaaacccgcaugggugcucgaccgggcccuguggcgcuuuucaugcgacguggcggaagggaaguacaaggaaaaggggauucccgcccugaucgagaacgaucaccacaugaacucaauucgcaaaaucaucugggaggauaucuucccuaagcucaagcugugggaauucuuccaagucgacgucaacaaggccguggaacaauucagaaggcugcugacccaagagaaccgcagagugaccaagucggacccgaaccagcaccugacuauaauccaggacccggaauaccggagguucgguugcaccguggacaugaacauugcacucaccaccuucaucccgcacgauaaggguccggcggcgauugaggagugcugcaacugguuccacaagcggauggaggaacugaacuccgagaagcaccggcugauuaacuaccaccaggaacaggcugugaauugccugcuggggaacguguucuacgaacggcucgccggccacggccccaagcuggggcccgucacccgcaagcacccgcucgugacucgauauuucaccuucccguucgaggaaauugauuucuccauggaggaaucaaugauccaucugccgaacaaggccuguuucuugauggcccacaacggcugggugaugggagaugacccgcugagaaauuucgccgagccgggguccgagguguaccugaggagagaacucaucugcuggggggauuccgugaaacugcgcuacgggaacaagcccgaggacugccccuaccugugggcacauaugaagaaguacaccgaaaucaccgccaccuacuuccaagggguccggcuggauaacugccauucaacuccgcuccauguggccgaauacaugcuggacgccgcacggaacuugcagcccaaccucuacgugguggccgaacucuucacugggagcgaagaucucgauaacguguucgugacccggcucggaauuucgagccugauccgggaagcgaugucugcuuacaacucgcacgaagagggaaggcugguguacagauacgggggggagcccgugggauccuucgugcaaccgugccugaggccgcuuaugcccgcgaucgcccacgcucuguucauggacaucacccacgacaacgaauguccgauuguccaccggagugccuacgaugcccuuccgagcacuaccaucgugucgauggcgugcugugcguccgggucuacccgcggcuacgacgaacucgucccgcaccaaaucagcgugguguccgaagaacgguuuuacacuaaguggaacccggaggccuugcccucgaacaccggggaggucaacuuccagucgggaaucauugccgcccgaugugccaucucaaaguugcaccaagaacucggggcaaagggguucauccaaguguacguggaccaaguggacgaggauauuguggccgugaccaggcacuccccgucgauccaccaguccgugguggcagucucaagaacugccuuccggaaccccaagaccuccuuuuacucgaaggaagugccccagaugugcaucccgggcaaaaucgaagaagucgugcuggaagccagaacuaucgagcggaacaccaagcccuaccggaaggaugagaacagcaucaacggcacgcccgacaucaccgucgagaucagagagcacauccagcugaacgaauccaagauugucaagcaggccggcguagcgacuaagggacccaacgaauacauccaggagaucgaauucgaaaaccugucgccgggauccgugauuaucuuccgggugucccuggacccgcacgcccaaguggccgugggaauccugcggaaccaccugacccaguucuccccgcauuucaaguccggcucccuggcgguggacaaugcagacccgauucucaagaucccguucgccuccuuggccucccgccugacccucgccgaacucaaccagauccuguaccgcugcgagucugaggaaaaggaggacgggggaggaugcuacgauauuccgaacuggucugcccuuaaauacgcgggacugcagggucugaugucggugcucgccgagaucagaccgaagaacgaccuggggcacccguuuugcaacaaccugagaucgggggauuggaugaucgacuacgugucgaaccggcuuaucucucgcuccggcaccaucgccgaggucgggaaguggcugcaggccauguucuucuaccugaagcaaauuccgcgcuaccugaucccgugcuacuuugaugccauccugaucggcgccuacacgaccuugcuggacaccgccuggaagcagaugagcagcuucgugcagaacggcuccacguucgugaagcaucugucccugggauccgugcagcuuugcggugucggaaaguucccuucgcugccuauucuguccccggcgcugauggacgugccguaccggcugaacgagaucacuaaggagaaggaacaaugcugcgugucacuggcggcgggacucccccacuucuccuccgggauuuuccgguguuggggaagagauaccuucauugcccugagggggauacugcugaucaccggaagauacguggaggcuagaaacaucauccucgccuucgccggcacucuccgccacgggcugauccccaaccucuugggcgaaggaaucuacgcccgguauaacugccgcgacgcggucuggugguggcuucagugcauccaggauuacugcaaaauggugccgaauggacuggauauucugaagugccccguuagccgcauguaccccaccgaugacuccgcacccuugccggcgggcaccuuggaccagccgcucuuugaagugauccaggaggccaugcagaagcacaugcaggguauccaguucagagagcggaacgcugggccgcagauugaccggaacaugaaggacgaagguuucaacauuacugccgggguggacgaagagacuggguuuguguacggggggaaccgcuucaacugugggaccuggauggauaagaugggggagucggaucgggcucggaacagggggauccccgcuaccccccgggacgggucggcuguggagauugucgggcugagcaagagcgcagugcgcuggcugcuggagcucagcaaaaagaacaucuuccccuaccacgaagucacugugaagagacacggaaaggccaucaagguguccuacgaugaguggaacagaaagauccaagacaacuucgagaagcuguuccauguguccgaggauccgagcgaucugaacgaaaagcauccgaaccucgugcacaagcgcgggaucuacaaggacucguacggcgcauccucgccguggugcgacuaccagcugcgccccaauuucaccauugccauggugguggcgcccgagcuguucacuaccgagaaggccuggaaggcccuggagauugcugagaagaagcugcugggaccgcucgggaugaaaacuuuggacccugacgacaugguguacuguggaaucuacgacaaugcgcucgacaacgacaacuacaaucuugcgaagggauucaacuaccaucaggggcccgaauggcuguggccgaucggguacuuccugcgcgccaagcuguacuucucccggcugauggggcccgagacaaccgccaagaccauugugcucgucaagaacguucucucccggcacuacgugcaccucgaaagauccccguggaaggggcugcccgagcucaccaacgagaacgcacaguacugcccguucuccugugaaacccaggccuggagcaucgccaccauauuggaaacucuguaugaccucuag

SEQ ID NO: 22 - RNA, 4599 nt, Artificial Sequence
  Codon-Optimized AGL Coding Sequence
augggacacucgaaacagaucagaauccuguugcugaacgaaauggagaagcuggaaaagacccucuuucggcucgaacagggcuacgagcugcaguuccgccuggguccgacucuacaaggaaaggcagugacuguguacaccaacuacccauuucccggagaaaccuucaaccgggagaaguuccggucccuggacugggaaaacccaaccgaacgagaggaugauuccgacaaguacugcaagcugaaccuccaacaguccggaucauuccaguacuacuuuuugcaaggaaacgagaaguccggaggaggcuacaucguggucgacccgauucugagagugggagcugacaaucauguccugccucuggacugcguaacccugcaaaccuucuuggccaaaugccugggcccguucgaugagugggaaagccgccuccgggucgcaaaggaaagcggcuacaauaugauucacuucacuccucugcaaacccucggucugucccgguccuguuauucccuggcgaaccagcuggagcuuaaccccgacuucucgcgcccaaaccggaaguacaccuggaacgacgucgggcagcuuguggaaaagcugaagaaggaguggaacgugaucugcaucacugacgugguguacaaccacaccgcggccaacuccaaguggauccaagaacaucccgaaugcgcguacaaccucgugaacagcccgcaucugaagccugccugggugcuggauagggcccucuggagauucagcugcgacguggccgaggggaaguacaaagaaaagggaauucccgcccugauugagaacgaccaucacaugaacucaauccgcaagaucaucugggaggauaucuucccuaagcuuaaguugugggaguucuuccaaguggacgugaacaaggcaguggagcaguucagaaggcugcugacucaagaaaacagacgggucacuaaguccgacccuaaccagcaccuuaccaucauucaagacccggaguaccgccgguuuggcugcacugucgacaugaacaucgcccugaccacuuucaucccgcaugacaagggcccggcggcaaucgaggaaugcuguaacugguuucauaagaggauggaggaacugaauuccgagaagcaccggcugauuaacuaccaccaggaacaggcagugaauugccuccugggaaacguguucuacgaacggcuggcuggacacggaccgaagcugggucccgugacucgcaagcauccgcucgugacucgcuacuucaccuucccguuugaggagauugacuuuuccauggaagaauccaugauccaccucccgaacaaggcuugcuuccugauggcgcacaacggaugggucaugggcgacgacccacugcgcaacuucgcugagccuggcagcgaggucuaccugagaagggaacugauuugcuggggagacuccgucaagcugcgcuauggaaacaagcccgaagauugccccuaccugugggcucacaugaagaaguacacugaaaucacugccacguacuuccagggaguccggcuggacaauugccacuccaccccccuccauguggccgaguacaugcucgaugcagcgaggaaucugcagcccaaucuguacgugguugccgaacuguucaccggcuccgaggaccucgacaacguguucgugaccagacuugggauuuccagccugauccgggaagccaugucggccuacaacucccaugaagagggccgccugguguaccgcuacggcggagaacccgugggaagcuucgugcagccuugccuccggccgcugaugccugcgaucgcccacgcccuguucauggauauuacccacgacaacgaaugccccaucgugcaucgcucggccuacgacgcacugccuucgaccaccaucguguccauggccugcugcgccuccgguagcacccgcggauacgaugaacucgugccgcaccagaucagcgugguguccgaagaaagauucuacaccaaguggaacccugaggcacugccgagcaacaccggagaagugaacuuccagucggguauuaucgccgcucgcugugccaucuccaaacuccaccaagagcucggugccaagggauucauucaagucuacguggaucaggucgacgaagauauuguggccgugaccaggcacucaccuuccauccaccaauccgucgucgccgugucacggacugccuuccggaaccccaagacuucguucuacucgaaagaggugccacagauguguauccccggaaagaucgaagaggucguccuggaagcccggaccauugagaggaacaccaagccuuaccggaaggacgagaacagcaucaacgguaccccugauauuacuguggagauccgcgaacacauccagcucaacgaaucaaagauugucaagcaggccggaguggccaccaagggacccaacgaguacauccaggagaucgaauuugaaaaccucuccccuggcuccgugauuaucuuccgggugucccuggacccucacgcccaaguggccgucggcauccucagaaaccaccugacccaguucucaccccauuucaaguccgguucccuggcgguggacaacgccgauccgaucuugaagauccccuuugcaucccuggccucccgccugacucucgcggaacugaaccagauccuguaccgcugcgaaucagaggaaaaggaggacggcggcggcuguuacgauaucccgaauugguccgcucugaaauaugcgggacuucaggggcugaugagcgugcuggcggagauccggccgaagaaugaccugggacacccauucugcaacaacuugcggagcggagacuggaugaucgauuacgucagcaacagauugaucucccggagcggcacuaucgcggaggucggaaaguggcuccaggccauguucuucuaccugaagcagaucccccgauaccucaucccguguuacuucgacgccauucugaucggggccuacaccacccugcuggacaccgccuggaagcagaugagcuccuuugugcaaaacggguccaccuucgugaagcaccuuucacugggaucagugcagcucugcggcgugggaaaauuccccucgcugcccauucugagcccggcccucauggacgucccuuaccggcugaacgagaucaccaaggagaaggagcagugcuguguuucccuggcugccggacuuccacacuucucguccggcaucuuccggugcuggggccgggauaccuucauugcccugcggggcaucuuguugaucaccggucgcuacguggaggcucggaacauuauucuggcauucgccggcacucugagacacggucugauuccgaaucuuuugggcgaaggaaucuacgcccgcuacaacugucgggacgccguguggugguggcuccagugcauucaggacuauugcaagauggugccgaacggccuggacauccugaagugcccagugucgaggauguauccaaccgacgacagcgcgccucugccggccgggacccucgaccaaccccuguucgaagucauucaagaggcuaugcagaagcacaugcaggguauucaguuccgggagagaaacgcggggccccagauugauaggaacaugaaagacgagggcuucaacaucacugccggcguggacgaagaaaccgguuuuguguacggaggaaaccgguucaacugcgguaccuggauggacaagaugggagaguccgaucgcgcgcgcaacagagggaucccggcaaccccgcgggacggaucagcgguggaaauugugggacugagcaagagcgccgugcgcuggcuccuggaacugagcaaaaagaacaucuuccccuaccacgaagugaccgugaagcggcacggaaaggccaucaaagucucauacgaugaauggaauaggaagauccaggauaacuucgagaagcuguuucacguguccgaggaucccuccgaucugaacgaaaagcauccgaaucucgugcacaagcgcggcaucuacaaggacucguacggagccuccuccccuuggugcgauuaucagcugcggccuaacuucaccauugccauggucguggcuccggagcuguucacuacugagaaggccuggaaggcacuugaaauugccgagaagaagcugcuugggccuuuggggaugaaaacccuggauccggacgacaugguguacugcggaaucuacgacaacgcccuggacaacgacaacuacaaucuggcgaagggcuucaauuaccaccagggcccggaauggcuguggccuauuggguacuuccugcgcgccaagcuguacuucucacggcugaugggaccagagacuaccgccaagacuaucguccucgugaagaacgugcugucccggcacuacgugcaucuggagaggagcccuuggaagggccuuccugagcugaccaacgaaaacgcccaguacugccccuucuccugcgaaacccaggcuugguccauugccacuauacuggaaaccuuauaugaccuguag

SEQ ID NO: 23 - RNA, 4599 nt, Artificial Sequence
  Codon-Optimized AGL Coding Sequence
augggacacucaaagcagauccggauccuccugcugaacgaaauggaaaagcucgaaaagacucuguuccggcuggaacagggcuaugagcugcaguuccggcucggaccgacgcugcaaggaaaggccgugacuguguacaccaacuaccccuucccgggagaaacuuuuaacagagaaaaguuuaggucccuggacugggagaacccgaccgagcgggaagaugacuccgauaaguacugcaagcugaaccuccagcagucgggaucguuccaguacuacuuccuucaaggaaaugagaagucugguggaggauacaucgugguggaccccauccugagagugggagccgacaaucacguccugccgcuugacugcgugacucugcaaaccuuccuggcuaagugucucgggccguucgacgaaugggaguccaggcugcgcguggcuaaggagagcggcuacaauaugauccacuucaccccgcuccaaacucucggacucucgcgcuccuguuacucccucgccaaccaacuggagcugaacccggacuucucccgcccgaaccggaaguacaccuggaacgacgucggucagcucguggagaaauugaagaaggaguggaacgugaucugcauuacggacgucguguacaaccauacugcggccaacuccaaguggauucaagagcacccggaaugcgcuuacaaccuugucaacuccccgcaccugaagccggccugggugcuggacagagcccuguggcgguucucgugcgacguggcagagggaaaguacaaggagaagggcauccccgcccuuauugagaaugaccaucacaugaacuccauccggaagaucaucugggaggauaucuucccgaagcucaagcugugggaauucuuccaaguggacgugaacaaggccguggaacaguuccggagacuccugacccaagaaaaccggagagugaccaagagcgacccgaaccagcaucugacuaucauucaggauccggaguaucggcgguuuggcugcacuguggacaugaacaucgcccucaccaccuucaucccgcacgacaagggccccgccgcgaucgaggaaugcugcaacugguuccacaagcgcauggaggagcugaauuccgaaaagcaccgccugaucaacuaccaucaggagcaggcagugaacugucuccugggaaacguguuuuacgaacggcuggccggacacggcccgaagcugggucccgugacccgcaagcauccccucgugacgcgguacuucaccuucccguucgaggagaucgacuucagcauggaagaguccaugauccaucugccgaacaaggccugcuuccucauggcgcauaaugguugggucaugggagaugauccccuccgaaacuuugcggagccggguucggaaguguaucugaggagggagcucaucugcuggggagauagcgugaaacugagauacgggaacaagccggaagauuguccguaccugugggcacacaugaagaaguacaccgaaaucacugccacuuacuuccaaggaguucgccuggauaacugccauucaaccccucugcaugucgccgaguacaugcuggacgccgcucgcaaccuucagccgaaucucuacguggucgccgagcuguucaccgguuccgaagaucuggacaacguguucgugacuagacugggaaucagcagccugauccgggaagcgaugagcgccuacaacucccacgaagagggccggcucguguauagauacggcggagagccggucgggagcuucgugcaacccugccugcggccgcugaugcccgccauugcccacgccuuguucauggauaucacccacgacaacgaguguccgaucgugcaccggagcgcguacgacgcguuaccguccaccacgauugugucgauggccugcugcgccuccggaucgacccgcggcuacgaugagcuggucccgcaucaaaucagcgucgucagcgaagaacgguucuacacuaaguggaaccccgaggcgcuccccuccaacaccggagaagugaacuuccaauccggcauuaucgcugcacgcugcgcgauuagcaagcugcaucaggagcuuggcgcuaagggguucauacaggucuacguggaucaggucgacgaggacauuguggccgugacucgccacucaccguccauucaccaaagcgugguggcugugucccggaccgcuuuccggaaucccaagaccucauucuacuccaaggagguuccgcagauguguaucccgggaaagauugaggaagugguccuagaggcucgcacuauugaacgcaacaccaagccguacagaaaggacgagaauuccauuaacgggaccccggauauuaccguagaaauuagagaacauauucagcugaacgagucgaagaucgugaagcaggccgggguggcuaccaagggcccgaacgaauacauccaggagauugaguucgaaaaccucucccccggcucggugaucaucuuccgggugucccucgauccccacgcccaaguggccgugggaaucuugagaaaccaccugacucaguucagcccgcauuucaaguccggaucacucgccguggacaacgccgacccgauccuuaagauccccuucgcaucacuggccagccgccugacccuugccgaacugaaccaaauccucuaucggugcgaauccgaggagaaggaagauggggguggaugcuaugacauuccuaacuggucugcccugaaauacgcaggccugcagggacugauguccguccuggccgaaauccgcccgaagaaugaccuggggcaccccuuuugcaacaaucugagguccggagauuggaugauugauuacguguccaaccgccugauuucgcggagcggcaccaucgcggaagugggaaaguggcugcaagccauguuuuucuaccugaaacagaucccccgguaccucaucccgugcuauuucgaugcgauuuugauuggcgcguacaccacccuccucgacacugccuggaagcaaaugagcuccuucgugcaaaacgguucaaccuucgucaagcacuugucgcuggggucgguccaacuguguggagucggaaaguucccgagccugcccauccugucgccugcccugauggacgugcccuaccggcugaacgagaucaccaaagaaaaggagcagugcugcgugucccuggcggccggacucccccauuucucguccgggaucuuuagauguuggggacgggauacuuucauugcgcugcgcggcaucuuguugauuaccggacgcuacguggaagcgcggaacaucauacucgccuucgccggcacccucagacacggccugaucccgaaccuccugggagaaggcaucuacgcacgauacaacugucgggacgccgucuggugguggcugcagugcauucaggacuacugcaagauggugccgaacggucuggacauccugaagugccccgugucaaggauguacccgaccgacgauagcgcaccgcugcccgcggggacccuggaucagccgcuguucgaagugauccaagaagccaugcaaaagcacaugcagggaauucaguucagagaaaggaacgcaggcccccagauugaccggaacaugaaggacgaggguuucaacaucaccgccggcgucgacgaagaaacgggguuuguguacgggggcaaccgcuucaacugcgguacuuggauggacaagaugggggaaucagaccgcgcccgcaaccgcggaauuccggcgaccccgcgcgauggauccgcaguggaaaucgugggacuguccaagucggcugugcgguggcugcuggagcuguccaagaagaacaucuucccguaccacgaggucaccgugaagagacacgggaaggccaucaagguguccuacgacgaauggaaccggaaaauccaggauaacuucgaaaaacuguuucacguguccgaggacccgucugaccugaacgaaaaacacccgaacuuggugcauaagcggggaaucuacaaggacaguuacggagccucaagcccguggugcgacuaccagcugcggcccaacuucacaaucgcgauggugguggcgcccgagcuuuucaccacggagaaagccuggaaggcacuggagaucgcugaaaagaagcugcucgguccccucggcaugaaaacccuggacccggacgauaugguguacugcggaaucuacgacaacgcccuggacaaugauaacuacaaccuggccaagggauucaauuaccaccaggggccggaauggcuguggccgaucggcuacuuucugcgggcuaagcucuacuucucgcggcugaugggaccggaaaccacagccaagaccauuguccucgucaagaacgugcugucccgccacuacgugcaucuggagcggucaccuuggaagggccugcccgagcugaccaacgaaaacgcccaguacugccccuucuccugugaaacucaagccuggucaaucgccacuauucucgaaacucuguacgaucuguag

SEQ ID NO: 24 - RNA, 4599 nt, Artificial Sequence
  Codon-Optimized AGL Coding Sequence
augggucacagcaaacaaauccggauccugcugcucaacgaaauggaaaagcuggaaaagacucuguuucgccuggagcagggcuacgaacuccaauuccggcugggaccaacgcugcaagggaaggccgucaccguguacaccaacuaccccuuucccggagagacuuuuaaccgcgaaaaguucagaagccuggacugggaaaaccccaccgaacgggaagaugauucggacaaguacugcaagcugaaccuccagcaguccggcagcuuccaguacuacuuccuccaagggaacgaaaagagcggaggaggcuacaucgugguggauccgauccuucggguuggagcggacaaccaugugcugccucuggacugcgugacucugcaaaccuuccuagccaagugccucggcccguucgaugagugggaaucccggcugcgaguggcgaaggagucagguuacaacaugauccacuucacaccgcugcagacccugggacucucccgguccugcuacucauuggccaaccagcucgaacugaacccggacuucucaaggccgaaccgcaaguacacuuggaaugacgugggacaguugguggagaagcugaagaaagaguggaacgugaucugcauuaccgacgugguguacaaccacacugcggcgaauucgaaguggauucaggaacauccggaaugcgccuacaacuuggugaacucaccucaccugaagccugccugggugcuggacagagcccuguggcgcuuuagcugugacgucgcggaggggaaguacaaggaaaagggaauccccgcccugaucgagaacgaccaccauaugaauagcauucgcaagaucaucugggaggacauuuucccgaagcugaagcugugggaguucuuccaagucgacgucaacaaggccgucgaacaguuccggcgguugcugacccaagaaaaccggagagugacgaaaagcgacccuaaccagcaccugacaaucauucaggacccugaauaccggagauucggcuguaccgucgauaugaacaucgcccugaccaccuuuauuccccacgauaagggcccggcggccaucgaggaguguugcaacugguuccacaagagaauggaggaacucaacuccgaaaaacaccgguugauuaauuaccaccaggagcaggcggucaacugccugcugggcaacguguucuacgaaaggcucgcugggcacggcccuaagcugggaccugucacucggaaacacccccuggugacccgguacuuuacuuucccguucgaagagaucgacuucuccauggaggaaagcaugauccaccucccuaacaaggccugcuuccugauggcccacaacggaugggucaugggcgacgacccuuugcggaacuuugccgagccgggcucagagguguaccuuagacgcgaacugaucugcuggggagacuccgugaagcugcgcuacgggaacaagcccgaagauuguccuuaccugugggcacacaugaagaaguacaccgaaaucacugccaccuacuuccaaggagugcgcuuggauaacugucauagcacuccucugcacgucgccgaguacaugcuggacgcagccaggaaucuccagccuaaucuguacgugguggccgaacuguucaccgggagcgaggaccuggacaacguguucgugacccggcugggcaucagcucccuuauccgggaggccauguccgcauacaacucgcacgaggagggucgccugguguaccgcuacggaggagagccggucggaucauuuguccaaccaugccuccggccccugaugccagcgaucgcgcacgcucucuucauggacaucacccacgauaacgaaugcccuaucgugcaccggagcgcuuacgacgcccucccuucgaccaccauuguguccauggccugcugcgccuccgguuccacucggggcuacgaugaacuggugccacaccagauuuccguggugucagaggagcgguucuacaccaaguggaacccagaggcgcugccgagcaacacuggggaagugaacuuccaguccggaaucauagcggcuagaugugcaauuuccaagcuucaucaggagcugggcgccaaaggauucauccaggucuacguggaccaaguggaugaggacauuguggccgugacuagacauucaccgucaauccaccaaucggucguggcuguguccagaaccgcauuccgcaaccccaagacuuccuucuacuccaaggaggucccucagaugugcaucccgggaaagaucgaggagguggugcuggaggccaggaccaucgaaagaaacacuaagccuuaccggaaagacgaaaacuccaucaaugggacucccgauauuaccguggagauuagggagcacauucagcugaacgaaucaaagauugugaaacaggccggggucgcaacuaaagggccuaaugaguacauccaagagaucgaguucgaaaaccugucgccggguuccgugaucauuuuccgcguguccuuggacccucacgcccaaguggccgugggcauccugaggaaccaccugacccaguucagcccacacuucaaguccggauccuuggcuguggacaacgccgauccaauccucaagaucccuuuugcgucgcuggccucacggcuuacccuggccgagcugaaccagauccuguaccgcugcgagagcgaagaaaaggaggacgguggagguugcuacgacauuccaaacugguccgcgcuuaaguacgccggacuccagggucugauguccgugcuugccgagaucagaccgaaaaacgaccuggggcaccccuuuugcaacaaccugagaagcggagacuggaugaucgacuauguguccaaccggcugauuucgagaagcgguacuauugccgaggucggaaaguggcuccaagcaauguuuuucuaccugaagcaaauuccccgcuaccugaucccgugcuacuuugacgccauucugaucggugcauacacuacccugcuggacaccgcguggaagcagauguccagcuucgugcagaauggcuccaccuucgucaagcaucugucccucggaagcgugcagcugugcggagugggaaaguuuccgucgcugccaauccugucccccgcgcugauggaugucccguaccggcugaacgaaaucacgaaggaaaaagaacagugcugcgugucccuugccgccggacugccgcacuucuccuccggcauuuuccggugcuggggacgggauaccuucaucgcgcugagagguauucugcugauuaccggcagauauguggaagcccgcaacaucauccuggccuuugccggcacucugcggcacgggcucaucccuaaccucuugggagaaggcaucuacgcgcgcuacaacugccgggaugcuguguggugguggcugcagugcauccaggacuacuguaaaauggugcccaauggccuugacauccucaagugcccagugucccggauguacccgaccgaugacuccgcgccccugcccgccggcacccuugaucaaccucuguucgaagucauccaagaggccaugcagaagcacaugcagggaauccaguucagggaaagaaacgccgggccucagaucgaccggaacaugaaggacgagggauucaacauuaccgccggaguggacgaggaaacuggcuucguguacgguggaaaccgcuucaacugcggcaccuggauggauaagaugggcgaauccgaucgcgcccgcaaccggggaaucccagcaacuccuagggacggaagcgcagucgagaucguggggcuguccaaguccgccgugcgguggcucuuagaacuguccaagaagaauauuuuccccuaccacgaggucaccgugaagcgccauggaaaggccaucaaaguguccuaugacgaauggaaccgcaagauccaggacaacuucgaaaaguuguuccacguguccgaggaccccagcgaucugaacgaaaagcaccccaaccucgugcacaagaggggcaucuacaaggacuccuacggagcuagcuccccuuggugcgauuaccaacugcggccuaauuucaccaucgccauggucgucgcacccgaacucuucaccaccgagaaggccuggaaggcucuggaaaucgccgaaaagaagcuucugggcccgcugggcaugaaaacucucgauccugacgauauggucuacuguggcaucuacgacaacgcccuugacaacgacaacuacaaccuggccaagggcuuuaacuaccaccagggcccagaguggcucuggcccaucggauauuuccugcgggccaaacuguacuucucgcgguugauggguccggaaaccacagcuaagaccaucgugcucgugaagaaugugcugucgcggcacuauguccaucuggagcgcucccccuggaagggacucccugagcugacuaaugagaacgcccaguacugcccuuucuccugcgaaacccaggccuggagcaucgcuaccauucucgaaacgcucuacgaucuguag

SEQ ID NO: 25 - RNA, 4599 nt, Artificial Sequence
  Codon-Optimized AGL Coding Sequence
augggacauucuaaacagauucggauccuccugcucaacgaaauggagaagcucgaaaagacccuguuccggcucgaacagggauacgaacugcaauuccggcugggucccaccuuacaaggaaaggccgugacugucuacaccaacuacccguuccccggcgaaaccuucaauagggagaaguuccggucccucgauugggagaacccuacagagcgcgaagaugauucagacaaguauugcaagcugaauuugcagcagagcggcucauuccaauacuacuuccugcaaggaaacgaaaagucgggcggcggcuacaucgugguggacccuauucugagagugggcgccgacaaccauguccugccgcuggacugcgucacccugcaaacuuuccuggccaagugccuggguccuuucgaugagugggaaucgagacuucgcguggcaaaggaaucggguuauaauaugauucacuucaccccgcugcaaacccugggccugucgcggucuugcuacucacuggccaaccagcuggaacugaacccagauuucucacgccccaaccggaaguacaccuggaacgaugugggccagcuuguggaaaagcucaaaaaggaguggaacgugaucugcauuacugacgugguguacaaccauacugcugcuaauuccaaguggauccaggaacauccugagugugcuuacaaccuggucaacuccccacaccugaagcccgccugggugcuggaucgggcucucuggcgguucuccugcgaugucgccgaaggaaaguacaaggagaaggggaucccugcgcugaucgaaaacgaccaucacaugaauuccaucaggaaaaucaucugggaggacaucuucccuaagcucaagcugugggaguucuuucaagucgacgugaacaaggccguggagcaguucagacggcugcugacacaagagaaccgccgcgucaccaagagcgacccgaaucagcaccugacgauuauccaggacccugaguacagaagauucggcugcaccguggauaugaacauugcucugaccaccuucaucccccacgauaagggucccgcagccauugaggagugcugcaacugguuccacaagaggauggaagaacugaauuccgagaagcaccggcugaucaauuaucaccaagaacaagccgugaacugccuucugggaaacgucuuuuacgagcgccuggcgggacaugggccaaagcucgggcccgugaccagaaagcacccacuggucacccgcuacuucaccuucccguucgaggaaaucgacuucagcauggaagagucgaugauccacuugccgaacaaggccugcuuccucauggcccauaacgguugggucaugggcgaugacccucuucgcaacuucgcggagcccgguucugaagucuaucuucggcgggaacugauuugcuggggagacuccgucaagcugcgcuacggaaacaagcccgaggauugcccguacuugugggcccauaugaagaaguacacugagaucacugccacuuacuuccaaggagugcgccucgacaauugucacagcacuccgcugcacguggcggaguacaugcuggacgccgcucgcaacuugcagccuaaucuguaugucguggccgaguuguucaccggcucggaagaucuggacaacguguucgucacucgccugggaaucuccucccugauccgggaagcgaugagcgccuacaacucccacgaagaggggcgguugguguaccgcuacggcggagagccugucggaaguuucgugcagcccugucugaggccccugaugcccgcuaucgcccaugcgcuguuuauggacaucacccacgacaacgaaugcccuauugugcaccgcuccgccuaugaugcccugcccuccaccacuauugucagcauggccugcugcgccucgggguccacccggggauacgacgaacuggugccccaccaaauuuccgugguguccgaggaacgguucuacaccaaguggaacccugaagcgcugccaucgaacacuggagaagugaacuuucagucgggaauuaucgcagcccgaugcgccaucagcaagcugcaccaggaacucggcgcaaaggguuuuauccaagucuacguggaccaggucgacgaggacauugucgccgugacccggcacuccccauccauccaccagucugugguggcugugucaaggacggcuuuccggaacccaaagaccagcuucuacagcaaggaagugccucagaugugcaucccggggaagaucgaagaaguggugcuggaggccagaaccaucgaaagaaacaccaagcccuaucggaaggacgagaacucgaucaacgguacuccggacauuaccgucgagauacgcgagcacauucagcugaacgaguccaaaaucgugaagcaggccgggguggccacgaagggucccaacgaguacauucaggagaucgaguucgagaaccugagccccggguccgugaucaucuuccgcgugucccuggacccccacgcccaaguggccgugggcauccugcggaaccaucugacccaguucuccccgcacuucaagagcggcucgcucgccguggacaacgcggacccgauccucaagaucccuuucgcaucgcuggccucccgccugacccuggccgaacugaaucagaucuuguaccgaugcgaaucagaagagaaggaggacggggggggcugcuacgauauccccaacuggagcgcguugaaguacgcaggauugcagggauugauguccguccucgcugaaauccgcccgaagaacgaccugggacacccguuuugcaacaaccugagaucaggggauuggaugaucgauuacgugucgaacagacugaucucgcgcagcggcacuauugccgaaguggggaaguggcuccaggccauguucuucuaccugaagcagaucccucgguacuugaucccuuguuacuucgacgccauccugaucggagccuacaccacccugcuugacacugcauggaagcagauguccagcuucgugcaaaacggaagcaccuucgugaagcaccugucccugggauccgugcagcucugcggcgugggaaaguuuccgucccuccccauccugagcccugcccuuauggacgugccguacaggcugaacgaaauuaccaaagagaaggagcaaugcuguguguccuuggcggccggauugccgcauuucuccuccgggauuuuccggugcuggggacgggacaccuuuaucgcacugagggguauucuccugaucaccggucgcuacguggaggcucgcaacauuauucuggccuucgcgggcacgcuuagacauggauugaucccuaaccuucugggagaagggaucuacgcgcgguacaacugccgcgaugccguguggugguggcugcagugcauccaggacuacugcaaaauggugccgaauggucuggauauccugaaguguccgguuucgcggauguacccuaccgacgacagcgccccucucccggccggcacucucgaccagccccuauuugaaguaauccaggaggccaugcaaaagcacaugcagggcauacaguucagagagaggaacgccggaccgcagauugaccggaacaugaaggacgagggauucaacauuaccgcgggaguggaugaggaaacugguuucguguacggcggaaaccgguuuaacugcggcacuuggauggacaagaugggagaauccgaccgcgcccgaaaccgcggaauucccgccacuccccgcgacggcuccgccguggaaauugugggacugucaaaguccgcaguccgcuggcugcuggaacucucaaagaagaacaucuucccguaccacgaggucaccgugaagcggcacggcaaagcgaucaaagugucguacgacgaguggaaccggaagauucaggauaacuucgagaagcuguuucacguguccgaagauccaagcgaccugaacgagaagcaucccaacuuggugcacaagcgcggcaucuacaaggauuccuacggagccagcagcccguggugcgacuaccaacuccgccccaacuucaccaucgccauggugguggcgccggagcuguucacgacggagaaagcuuggaaggcucucgaaaucgcggagaagaagcugcuggguccucuggggaugaaaacccuggacccggacgauaugguguacugugggaucuacgacaacgcccuggacaacgacaacuacaaccucgccaagggguucaacuaccaccagggacccgaauggcucuggccaaucggauacuuccugagagcgaagcuuuacuucucgcggcugauggguccugaaaccacggccaagaccaucgugcucgugaaaaaugugcugucaaggcacuacgugcaucuggagaggucgccauggaagggucugccggaacugaccaacgaaaacgcacaguacugccccuuuucgugcgagacucaggccugguccaucgccaccauucucgaaacucucuacgaccuguag

SEQ ID NO: 26 - RNA, 4599 nt, Artificial Sequence
  Codon-Optimized AGL Coding Sequence
augggacacucgaaacagaucagaauccuguugcucaacgaaauggagaagcuggaaaagacccucuuucggcucgaacagggcuacgagcugcaguuccgccuggguccgacacuacaaggaaaggcagucacuguguacaccaacuacccauuucccggagaaaccuucaaccgggagaaguuccggucccuggacugggaaaacccaaccgaacgagaggaugacuccgacaaguacugcaagcugaaccuccaacaguccggaucauuccaguacuacuuucugcaagggaacgagaaguccggaggcggcuacaucguggucgacccaauacuuagagugggagccgacaaucauguccugccucuggacugcgugacccugcaaaccuucuuggcgaaaugucugggcccguucgaugagugggaaagccgccucagagucgcaaaggaguccggauacaacaugauucacuucacuccgcugcaaacccucggucugucccggucgugcuauucucuggcgaaccagcuggagcuuaaccccgacuucucgcgcccaaaccggaaguacaccuggaacgacgucgggcagcuuguggaaaagcugaagaaggaguggaacgugaucugcaucacugacgugguguacaaccauacggccgccaacucgaaguggauccaagagcaucccgagugcgcguacaaccucgugaauagcccgcaucugaagccugcuugggugcuggauagagcccucuggagauucagcugcgacguggccgaggggaaguacaaagaaaagggaauuccggccuugauugagaacgaccaucacaugaacucaauccgcaagaucaucugggaggauaucuucccuaagcuuaaguugugggaguucuuccaaguggacguaaacaaggcaguggagcaguucagaagguugcugacucaagaaaacagacgggucacuaaguccgauccuaaccagcaccuuaccaucauucaagacccugaguaccgccgguuuggcugcaccgucgacaugaacaucgcccugaccacuuucaucccgcaugacaagggcccggcggcaaucgaggaaugcuguaacugguuucauaagaggauggaggaacugaauuccgagaagcaccggcugauuaacuaccaccaggaacaggcagucaacugccuccugggcaacguguucuacgaacggcuggcuggacacggaccgaagcugggucccgugacucgcaagcauccgcucgugacucgcuacuucaccuucccguuugaggagauugacuucuccauggaagaauccaugauccaccucccgaacaaggcuugcuuccugauggcgcacaacggaugggucaugggcgacgacccacugcgcaauuucgcugagccuggcucggaggucuaccugagaagggaauugauuugcuggggagacuccgugaagcugcgcuauggcaacaagccugaagauugccccuaccugugggcucacaugaagaaguacacggaaaucacugccacguacuuccagggaguccggcuggacaauugccacucgaccccgcuccauguggccgaguacaugcuggaugcagcgaggaaucugcagcccaaucuguacgugguugcagaacuguucacuggcuccgaggaccucgacaacguguucgugaccagacuggggauuuccucacugauccgggaagccaugucggccuacaacucccaugaagagggccgccugguguaccgcuaugggggagaacccgugggaagcuucgugcagccuugccuccggccgcugaugccugcgaucgcccacgcccuguucauggauaucacucacgacaacgaaugccccauugugcaucgcucggccuacgacgcacugccuucgaccacuaucguguccauggccugcugcgccuccgggagcacccgcggauacgaugaacucgugccgcaccagaucagcgugguguccgaagaacgguucuacaccaaguggaaccccgaagcccugccuagcaauaccggggaagugaacuuccaguccgguauuaucgccgcucgcugcgccaucuccaaacuccaccaagagcucggugccaagggauucauucaagucuacguggaucaggucgacgaagauauuguggccgugaccaggcacucaccuuccauccaccaauccgucgucgccgugucccggacugcguuucggaaccccaagacuucguucuacucgaaagaagugccacagauguguaucccgggaaaaaucgaggaggucgugcucgaagcccggaccauugagaggaacaccaagccuuaccggaaagacgagaacucuaucaacgguaccccugauauuacuguggagauccgcgaacacauccagcugaacgaaucaaagaucgucaagcaggcuggaguggccaccaagggacccaacgaguacauccaggagaucgaauuugaaaaccucuccccuggcuccgugauuaucuuccgggugucccuggacccucacgcccaaguggccgugggaauucucagaaaccaccugacccaguucucaccacacuuuaaguccgguucccuggcgguggacaacgccgauccgaucuugaagauccccuucgcaucgcucgccucccgccugacucucgcggaacugaaccagauccuguaccgcugugaauccgaggaaaaggaggacggcggcggcuguuacgauauccccaauuggucggcuuugaaauacgcgggacuucaggggcugaugucugugcuggcggaaauccggccgaagaacgaccugggacacccauucugcaacaacuugcggagcggagacuggaugaucgauuacgucagcaacagauugaucagccggagcggcacuaucgccgaggucggaaaguggcuccaggccauguucuucuaccugaagcagaucccccgauaccucauccccuguuacuucgacgccauucugaucggggccuacaccacccugcuggacaccgccuggaagcagaugagcaguuuugugcaaaacggguccaccuucgugaagcaccuuucacugggcucagugcagcucugcggcgugggaaaguuccccucgcugcccauucugagccccgcccugauggacgucccuuaccggcugaacgagaucaccaaggagaaggagcagugcuguguuucccuggcugccgggcugccacacuucucguccggcaucuuccgguguuggggccgggauaccuucauugcccugcggggaauccugcuuaucaccggucgcuacguggaggcucggaacauuauucucgcguucgccggcacccugagacacggucugauuccgaaucuguugggcgaaggaaucuacgccagauacaacugucgggacgccguguggugguggcuccagugcauucaggacuauugcaagauggugccgaacggccuggacauccugaagugcccagugucgaggauguauccaacugacgacagcgcaccucugccggccgggacccucgaccaaccccuguucgaagucauucaagaggcuaugcagaagcacaugcaggguauucaguuccgggagcggaacgcggggccccagauugauaggaacaugaaagacgagggcuucaacaucacugccggcguggacgaagaaaccgguuuuguguacggaggaaaccgcuucaacugcgguaccuggauggacaagaugggagaauccgaucgcgcgcgcaacagagggaucccggcaaccccucgggacggauccgcgguggaaauugugggacugagcaagagcgccgugcgguggcuccuggaacuguccaaaaagaacaucuuccccuaccacgaagugaccgugaagagacacggaaaggccaucaaagucucauacgaugaauggaacaggaagauccaggauaacuucgagaagcuguuucacguguccgaggaucccuccgaucugaacgagaagcauccgaaucuggugcacaagcgcgggaucuacaaggacucguacggagcguccuccccuuggugcgacuaucagcugcggccuaacuucaccauugccauggucguggccccggagcuguucacaacugagaaggccuggaaggcccuugaaauugccgagaagaagcugcuggggccuuuggggaugaaaacccuggauccggacgacaugguguacugcggaaucuacgacaacgcccuggacaacgauaacuacaaucucgcgaagggcuucaauuaccaccaaggccccgaauggcucuggccuauuggguacuuccugcgcgccaagcuguacuucucacggcugaugggaccagagacuaccgccaagacuaucguccucgugaagaacgugcugucccggcacuacgugcaucuggagaggagcccuuggaagggacuuccugagcugacgaacgaaaacgcgcaguacugccccuucuccugcgaaacccaggcuugguccauugccacuauacuggaaaccuuauaugaccuguag

SEQ ID NO: 27 - RNA, 4599 nt, Artificial Sequence
  Codon-Optimized AGL Coding Sequence
augggacacucgaaacagauccggauccuguugcugaacgaaauggagaagcuugaaaagacccuguuucggcuggagcagggcuacgagcugcaguuccgccuggguccgacacuacaaggaaaggccgugacuguguacaccaacuacccauuucccggagaaacuuucaaccgggagaaguuccggucccuggacugggaaaacccaaccgaacgagaggacgacucggacaaguacugcaagcugaaccuccaacaguccggaucauuccaguacuacuuucugcaagggaacgagaaguccggaggcggcuacaucguggucgacccgauacuuagagugggcgccgacaaucauguccugccucuggauugcgugacccugcaaaccuucuuggccaaaugucugggcccguucgaugagugggaaagccgccucagagucgcaaaggaguccggauacaacaugauucauuucaccccgcugcaaacccugggucugucccggucgugcuauucucuggcgaaccagcuggagcuuaaccccgacuucucgcgcccaaaccggaaguacaccuggaacgacgucgggcagcuuguggaaaagcugaagaaggaguggaacgugaucugcaucacugacgugguguacaaccauacggccgccaacucgaaguggauccaggagcaucccgagugcgcauacaaccucgugaacagcccgcaccuuaagccugcuugggugcuggacagagcccucuggagauucaguugcgacguggccgaggggaaguacaaggaaaagggaauuccggccuugaucgagaacgaccaucacaugaacucaaucaggaagaucaucugggaggacaucuucccuaagcuuaaguugugggaguucuuccaaguggacguaaacaaggcaguggagcaguucagaagguugcugacccaagaaaacagacgcgucacuaaguccgauccuaaccaacaccuuaccaucauucaagacccugaauaccgccgguuuggcugcaccgucgauaugaacaucgcccugaccacuuucaucccgcaugacaagggcccggcggcaaucgaggaaugcuguaacugguuucauaagagaauggaagaacugaauuccgagaagcaccggcugauuaacuaccaccaggaacaggcagugaacugccugcugggcaauguguucuacgaacggcuggcuggacacggaccgaagcugggucccgugacuaggaagcauccgcucgugacucgcuacuucaccuucccguuugaggagauugacuucucgauggaagaauccaugauccaucugccuaacaaggcuugcuuccugauggcgcacaacggaugggucaugggcgacgacccccugcgcaacuucgccgagccuggcucggaggucuaccugagaagggaacuuaucuguuggggagacuccgucaagcugcgcuacggaaacaagcccgaagauugccccuaccugugggcucacaugaagaaguacacggaaaucacugcaacguacuuccagggaguccggcuggacaauugccacuccaccccccuucauguggccgaguacaugcucgaugcagcgaggaaucugcagccgaaucuguacgugguugccgaacuguucacuggcuccgaggacuuggacaacguguucgugaccagacuggggaucuccucccugauccgggaagccaugucggccuacaacucccaugaagagggccgccugguguaccgcuacgggggagaacccgugggaagcuucgugcaaccuugccugcggccgcugaugccugcgaucgcccacgcccuguucauggacaucacucacgauaacgaaugcccgauugugcaucgcucggccuacgacgcacugccgagcaccacuaucguguccauggccugcugcgccuccgggagcacucgcggauacgaugaacucgugccgcaccagaucagcgugguguccgaagaacgcuucuauaccaaguggaaccccgaagcgcugccaucgaauacuggcgaagugaacuuccaguccgguauuaucgccgcucgcugugccaucagcaaacugcaccaagagcuuggugccaagggauucauucaagucuacguggaucaggucgacgaagauauuguggccgugaccaggcacucaccuuccauccaccaaucagucguggccgugucccggaccgcguuccggaaccccaagaccagcuucuacucgaaagaagugccucagauguguaucccgggaaaaaucgaagaggucgugcuggaagcccggaccauugagaggaacaccaagccuuaccggaaagacgagaacucuaucaacgguaccccugauauuacuguggagauccgcgaacacauccagcugaacgaaucaaagaucgucaagcaggcuggaguggccaccaagggacccaacgaguacauccaggagaucgaauuugaaaaccucuccccuggcuccgugauuaucuuucgggugucccuggacccucacgcccaaguggccgugggaauucucagaaaccaccugacccaguucucaccccacuucaaguccgguucccuggcgguggauaacgccgacccgauuuugaagauccccuucgccucgcuggccucccgccugacucucgcggaacugaaccagauccuguaccgcugugaaucagaggaaaaagaggacggcggcggcuguuacgauauucccaauuggucggcuuugaaauacgcgggacuucaggggcugaugucugugcuggcggaaauccggccgaagaacgaccugggacacccauucugcaacaacuugcgguccggagacuggaugaucgauuacgucagcaacagauugaucagccggagcggcacuaucgcugaggucggaaaguggcugcaggccauguucuucuaucugaagcagaucccccgauaccucauccccuguuacuucgacgccauucugaucggggccuacaccacccugcuggacaccgccuggaagcagaugagcaguuuugugcaaaacggguccaccuucgugaagcaccuuucacugggcucagugcagcucugcggcgugggaaaguuccccucucugcccauucugagcccggcccugauggacgucccuuaccggcugaacgagaucaccaaggagaaggagcagugcugcguuucccuggcugccgggcugccacacuucucguccggcaucuuccggugcuggggccgggauaccuucaucgcccugcgggguauccugcuuaucaccggucgcuacguggaggcucggaacauuauucuggcguucgccggcacccuuagacacggacugauuccgaaccuuuugggcgaaggaaucuacgccagauacaacugucgggacgccguguggugguggcuucagugcauucaggacuauugcaagauggugccgaacggccuggacauccugaagugcccagugucgaggauguauccaaccgacgacagcgcaccucugccggccgggacccucgaccaaccccuguucgaagucauucaggaggcuaugcagaagcacaugcaggguauucaguuccgggagcggaacgcggggccgcagauugauaggaacaugaaagacgagggcuucaacaucacugccggcguggacgaagaaaccgguuuuguguacggaggaaacagauucaacugcgguaccuggauggacaagaugggagaguccgaucgcgcgcgcaacagagggaucccggcaaccccgcgggacggauccgcgguggaaauugugggacugagcaagagcgccgugcgguggcugcuggaacugagcaaaaagaacaucuuccccuaccacgaagugaccgugaagcggcacggaaaggccaucaaagucucauacgaugaauggaauaggaagauccaggauaacuucgagaagcuguuucacguguccgaggaucccuccgaucugaacgaaaagcacccgaaucucgugcacaagcgcgggaucuauaaggacucguacggagcguccuccccuuggugcgacuaucagcugcggccuaacuucaccauugccauggucguggccccggagcuguucacaacugagaaggccuggaaggcccuugaaauugccgagaagaagcugcuggggccuuuggggaugaaaacccuggauccggacgacaugguguacugcggaaucuacgacaacgcccuggacaacgauaacuacaaucuggccaagggcuucaauuaccaccagggcccggaauggcuguggcccauuggguacuuccugcgcgccaagcuguacuucucacggcugaugggaccagagacuaccgccaagacuaucguccucgugaagaacgugcugucccggcacuacgugcaucuggagaggagcccuuggaagggacuuccugaacugacuaacgagaacgcgcaguacugccccuucuccugcgaaacccaggcuugguccauugccaccauacuggaaacccuuuaugaccuguag

SEQ ID NO: 28 - RNA, 4599 nt, Artificial Sequence
  Codon-Optimized AGL Coding Sequence
augggacacucgaaacagauuagaauccuguugcucaacgaaauggagaagcuggaaaagacccucuuucggcuggagcagggcuacgagcuccaguuccgccuggguccgacacuacaagggaaggcagugaccguguacaccaacuacccauuucccggagaaaccuucaaccgggagaaguuccggucccuggacugggaaaacccaaccgaacgagaggaugacagcgacaaguacugcaagcugaaccuccaacagucgggaucguuccaguacuacuuucugcaagggaacgagaaguccggaggaggcuacaucguggucgacccgauacuuagagugggagccgacaaccauguccugccucuggacugcgugacccugcaaaccuucuuggccaaaugucugggcccguucgaugagugggaaagccgccucagaguggccaaggaguccggguacaacaugauucacuucacuccgcugcaaacccucggucugucccggucgugcuauucucuggcgaaccagcuggagcugaaccccgacuucucccgcccaaaccggaaguacaccuggaacgacgucgggcagcuuguggaaaagcugaagaaggaguggaacgugaucugcauuacugacgugguguacaaccacaccgccgccaacucgaaguggauccaagaacaucccgagugcgcguacaaccucgugaacagcccgcaucugaagccggcuugggugcucgauagagcccucuggagauucuccugugacgucgccgaggggaaguacaaagagaaggguauuccggcccucauugagaacgaccaucacaugaacucaauccggaagaucaucugggaggauaucuucccuaagcuuaaguugugggaguucuuccaaguggacguaaacaaggccguggaacaguucagaaggcugcugacucaagaaaaccgccgcgucacuaaguccgauccuaaccagcaucuuaccaucauccaagacccugaguaucgccgguuugggugcaccgucgacaugaacaucgcacugaccacuuucaucccgcaugacaaggggccggcggccaucgaggaaugcuguaacugguuucauaagaggauggaggaacugaauuccgagaagcaccggcugauuaacuaccaccaggaacaggcagugaauugccuccuggggaacguguucuacgaaaggcuggcuggacacggaccgaagcuggggcccgugacucgcaagcauccgcucgugacucgcuacuucaccuucccguuugaggagauugacuucucaauggaagaauccaugauccaccucccgaacaaggcuugcuucuugauggcgcacaauggaugggucaugggcgacgacccacugcgcaacuucgcugagccuggcucggaggucuaccugagaagggaauugauuugcuggggggacuccgucaagcugcgcuauggaaacaagccggaagauugccccuaccugugggcucacaugaagaaguacacggaaauuacugccacguacuuccagggcguccggcuggacaacugccacuccacuccccuccauguggccgaguacaugcucgacgcagcgaggaaucugcagcccaaucuguacgugguugcagaacuguucacuggguccgaggaccucgacaauguguucgugaccagacuggggaucuccucccugauccgggaagccaugucggccuacaacucccaugaagagggccgccugguguaccgcuacgggggagaacccguggggagcuucgugcagccuugccuccgcccgcugaugccugccaucgcccacgcccuguucauggauaucacucaugacaacgaaugucccauugugcaucgcucggccuacgacgcacugccuucgaccacuaucguguccauggccugcugcgccuccgggagcaccaggggauacgacgaacucgugccgcaccagaucagcgugguguccgaagagagauucuauaccaaguggaaccccgaagcgcugcccagcaauaccggggaagugaacuuccaguccgguauuaucgccgcucgcugugcgaucagcaagcuccaccaggagcucggugccaagggauucauucaagucuacguggaccaggucgacgaagauaucguggccgugaccaggcacucaccuuccauucaccaauccguggucgccgugucccggacugcuuuucggaaccccaagacuucguucuacucgaaagaagugccacagauguguaucccggggaaaaucgaagaggucguccucgaagcccggaccauugagaggaacaccaagccuuaccggaaagacgagaacucuaucaacgggaccccugauauuacuguggagauccgcgaacacauccagcugaacgaaucaaagaucgucaagcaggcuggaguggcgaccaagggacccaacgaguacauccaggagaucgaauuugaaaaccucuccccuggcuccgugauuaucuuccgggugucccuggacccucacgcccaaguggccgugggaauucucagaaaccaccugacucaguucucaccccacuuuaagucugggucccuggcgguggacaacgccgauccgaucuugaaaaucccuuucgcaagccuggccucccgccugacuuuggccgagcugaaccagauccuguaccgcugugaaucagaggaaaaggaggacggggguggcuguuacgauauccccaacugguccgcuuugaaauacgcgggacugcaggggcugauguccgugcuggcggaaaucagaccgaagaacgaucuggggcaccccuucugcaacaacuugcgguccggagacuggaugaucgauuacgucagcaaccgguugaucagcagaagcgguacuaucgccgaggucggaaaguggcugcaggccauguucuucuaccugaagcagaucccucgauaccucauccccuguuacuucgacgccauuuugaucggggccuacaccacccugcuggacacugccuggaagcagaugagcaguuuugugcaaaaugggucgaccuucgugaagcaccuuuccuugggcucagugcagcucugcggcguggggaaguuccccucgcugcccauucuguccccggcccugauggacgucccuuaccggcugaacgagauuaccaaggagaaggagcagugcuguguuucccuggcugccgggcugccacacuucucguccgggaucuuccggugcuggggccgcgauaccuucauugcgcugcgggguauccugcuuaucaccggucgcuacguggaggcucggaacauuauccuugcauucgccgguacccugagacacggucugaucccgaaucuucucggggaaggaaucuacgcaagauacaacugccgggacgccguguggugguggcuccagugcauucaggacuauugcaagauggugccgaacggacuugacauccugaagugcccagugucgaggauguacccuaccgacgacagcgcuccucugccggccgggacccuggaccaaccccuguucgaagucauccaagaggcuaugcagaagcacaugcaggguauucaguuccgggaacggaacgcggggccccagauugauaggaacaugaaggacgaggguuucaacaucacugccggcguggacgaagaaacuggguuuguguacggaggaaacagauucaacugcgguaccuggauggacaagaugggagaauccgaucgcgcgcgcaacagagggaucccggcaaccccgcgggacggauccgcgguggaaauugugggacugagcaagagcgccgugcgguggcuccuggaacuguccaaaaagaacaucuuccccuaccacgaagugaccgugaagcggcacggaaaggccaucaaagucucauacgaugaauggaaucggaagauccaggauaacuucgagaagcuguuucacguguccgaggaucccuccgaucucaacgaaaagcauccgaaucucgugcacaagcgcgggaucuacaaggacucguacggggcguccucaccuuggugcgacuaucagcugcggccuaacuucacuauugcgauggucguggccccggaguuauucacaacggagaaggccuggaaggcccuugaaauugcggagaagaagcugcuggggccucucgggaugaaaacccuggauccggacgacaugguguacugcggaaucuacgacaacgcccuugacaacgauaacuacaaucuggccaagggguucaauuaccaccaggggccggaauggcucuggcccauuggguacuuccugcgcgccaagcuguacuucucacggcugauggggccagagacuaccgccaagacuaucguccucgugaaaaacgugcugucccggcacuacgugcaucuggagaggagcccuuggaagggacugccagagcugacgaacgagaacgcgcaguacugccccuucuccugcgaaacccaggcuuggucgauugccacuauacuggaaaccuuauaugaccuguag

SEQ ID NO: 29 - RNA, 4599 nt, Artificial Sequence
  Codon-Optimized AGL Coding Sequence
augggacacucaaagcaaauccgcauucugcugcugaacgagauggaaaagcuggaaaagacucuguuccggcuggaacaggguuacgagcugcaguuucggcucggcccaaccuugcaagggaaggccgucacugucuacaccaacuacccuuuuccgggggagacuuucaaccgcgaaaaguuccgcucccuggauugggaaaaccccacugaacgggaggaugacagcgacaaguacugcaaacugaaccuucagcaguccggcagcuuccaauacuacuuccugcaaggaaacgaaaaguccggcggcgguuacaucguggucgaccccauucugagagugggagccgauaaucaugugcugccccuggacugcgucacccugcaaacuuuccuggcuaagugccugggaccguucgaugagugggaauccaggcuccgcguggcgaaggagucgggcuacaacaugauucauuucacuccccuucaaacucuggggcugagucgcagcuguuacucccuggccaaccagcuugaacugaacccagacuuuucccggccaaacagaaaguacaccuggaacgacgugggacaauugguggagaagcuuaagaaggaauggaacgugaucugcaucaccgaugugguguauaaccacacugccgcgaauuccaaguggauccaggaacaccccgagugugcuuacaaccuugugaacagcccucaccuuaagccggccugggugcuggaucgggcgcuguggagauucuccugcgacguggccgaagggaaguacaaagaaaagggaauccccgcccugauugaaaaugaccaccauaugaacuccauucggaaaaucauuugggaagauaucuuucccaagcugaagcucugggaguucuuucaaguggaugugaacaaggcuguggagcaguuccggcggcugcugacccaggagaaccgccgcgugaccaaguccgacccuaaccagcacuugaccaucauacaggacccggaauaccggagauucggcugcacugucgacaugaacauugcccucacuaccuucaucccgcaugacaagggacccgcugccaucgaagagugcugcaacugguuccacaagcggauggaagaacugaacucugaaaagcacaggcugaucaacuaccaccaggaacaggcugugaacugccugcugggcaacguguucuacgagagacucgcaggacacggaccgaagcugggcccugugacccggaagcauccucuggucacccgcuacuucaccuucccguucgaagagaucgacuuuucgauggaagaaucgaugauccaccucccuaacaaggccugcuuccucauggcgcacaacggcugggucaugggcgacgacccgcugagaaacuucgccgagcccgggagcgaaguguaccuccggcgggaacuuauuugcuggggagauagcgugaagcuuagauauggcaacaagccugaggacugcccauaccugugggcgcacaugaagaaguacacugaaauuaccgcgaccuacuuccaaggaguccgacucgacaacugccacagcaccccacuucacgucgcggaguacauguuggaugccgcacggaaucuccagcccaaucuguaugucguggcugaacuguucacuggauccgaggaccuugacaauguguucgugacuagacuggggaucuccagccugauccgggaagcuauguccgcguacaacucccacgaagagggacggcugguguaccgcuacggcggagagcccgugggaagcuucgugcagcccugccugcggccucugaugccggccaucgcucacgcccuguucauggauaucacucacgacaaugaguguccuaucgugcacaggagcgcguacgacgcccugcccuccacuacuaucgugucgauggccugcugcgcaagcgguucuacccgcgguuacgacgagcuugucccgcaccaaauauccguggugucagaggaacgguucuacaccaaguggaacccggaggcccugccuucaaacaccggcgaagugaacuuccaguccggaaucauugccgcccgcugugccauuucaaaguugcaccaggagcugggcgccaagggauucauucaggucuacguugaccaggucgacgaagauaucguggccguuacuagacauucaccgagcauccaucagagcguggucgcagucagcaggacugccuuccgcaacccgaaaaccucguucuacuccaaggaagugccccagauguguaucccgggaaaaauugaggaaguggugcuggaggcccggaccaucgagcggaacacuaagcccuaccggaaggacgagaauucaaucaacggaaccccugacaucaccguggagauccgcgagcauauccaacugaacgagucgaagaucgucaagcaggcugggguggcaacuaagggcccuaacgaguacauucaggagauugaauucgagaaccugucccccggguccgugaucauuuuccgcgugucccuggacccacaugcucaaguagcaguggggauccugagaaaccaccugacccaguuuagcccgcacuucaaguccggaucccuggccguggauaacgccgacccgauccugaagauccccuuugcaucccuggcuucccggcugaccuuggccgaacugaaccagauucuguaccgcugcgaaucagaggaaaaggaggacggaggcggaugcuacgauauccccaauuggucggcgcugaaguacgccggccuucaaggacugauguccgugcuggccgagaucaggccgaagaaugaccugggacacccguucugcaacaacuugagaagcggggacuggaugauugauuacgugucgaaccggcugaucucccggagcggcaccaucgcggaagucggaaaguggcuccaggccauguucuucuaccugaagcagaucccccgcuaccugauccccugcuacuucgacgcgaucuugauuggggcauacaccacucugcuugacaccgcuuggaagcagauguccuccuucgugcaaaacggauccaccuucgugaagcaccugucccuuggaucagugcagcugugcggcgugggaaaguucccuucccuucccauccuguccccugcgcugauggacgugccguaccggcucaacgagaucaccaaggaaaaggaacagugcugcgugucacuggcagccggccuuccgcauuuuucgagcggaauuuucagauguuggggcagagacaccuucauugcgcugcgcgguauccugcugauuaccggcagauacguggaagccagaaacauuauccuggcguuugcugguacucugcggcacggacugauuccuaaccuguugggagaggggaucuacgcccgguacaauugcagagaugccguguggugguggcugcagugcauccaggacuacugcaagauggugcccaacggacuugacauucugaagugcccggugucgcgcauguaccccaccgacgacucugcgccccugccggccgguacccuggaucagccgcuguucgaagugauccaggaagccaugcaaaagcacaugcagggaauucaguucagggaacggaacgcaggcccgcaaaucgaccggaacaugaaggacgaaggcuucaacauuaccgccggcguggacgaggaaaccggcuucguguacggcggcaaccgguucaauugcgguacuuggauggacaagaugggagaaagcgaccgcgccaggaaucggggcauuccugccaccccgcgggacgguagcgcgguggagaucgugggccuuucgaaguccgcgguccgcuggcuucuggagcugucuaagaaaaacaucuucccuuaccacgaggucaccgugaaacgccacggaaaggccaucaagguguccuacgacgaauggaacaggaagauccaggacaacuuugagaagcuguuucacgugucggaagauccguccgaccugaacgaaaagcaccccaaccuuguccauaagcgcgguaucuacaaagauucguauggugcauccuccccuuggugcgacuaccaacuccggccgaacuucaccaucgcaauggugguggccccggagcuguucaccacugaaaaggccuggaaggcccuggaaaucgccgaaaagaagcugcugggaccgcuggggaugaaaacccuggaccccgaugauaugguguacugcgggaucuacgacaacgcccuggauaacgacaacuacaaccuggccaagggcuucaacuaccaucaggguccggaguggcuguggccaaucggauacuuccugagggccaagcuguacuucucccgcuugaugggccccgaaacuaccgcaaagacuaucgugcucgugaagaacguccugucccggcacuacgugcaucuggaacggucgccguggaaaggccugccagaguugaccaacgagaaugcccaguauugcccguucucaugcgaaacccaagccuggagcauugccacuauucuggaaacccucuacgaccuguag

SEQ ID NO: 30 - RNA, 4599 nt, Artificial Sequence
  Codon-Optimized AGL Coding Sequence
augggacacucgaaacagaucagaauccuguugcucaacgaaauggagaagcucgaaaagacccuguuccggcuggagcaggguuacgagcugcaguuccgccuggguccgacucuacaagggaaagcagugacggucuacaccaacuacccguuucccggagaaaccuucaaccgggagaaguuccggucccuggacugggagaacccgaccgaacgagaggaugacucagauaaguacugcaagcugaacuugcaacaguccgggucauuccaguacuacuuucugcaagggaacgagaagucaggagggggcuacaucguggucgacccgauacugcgcgugggagccgacaaucacguccugccgcuggacugcgugacccugcaaaccuuccucgccaaaugucuggggccguucgaugagugggaaagccgccucagagucgcaaaggaguccggauacaacaugauucacuucacuccgcugcaaacacucggucugucccggucgugcuauucucuggcgaaccagcuggagcuuaaucccgacuuuucccgcccgaaccggaaguacaccuggaacgacgucgggcagcuuguggaaaagcugaagaaggaguggaacgugaucugcaucacugaugugguguacaaccacacggcugccaacucgaaguggauccaagagcaucccgagugcgcguacaacuuggugaacagcccgcaucugaagccugcuugggugcuggacagagcccucuggagauucagcugcgacguggccgaggggaaguacaaagaaaaggggauuccggccuugauugagaacgaccaucacaugaacucaauccgcaagaucauuugggaggauaucuucccuaagcuuaaguugugggaguucuuccaaguggacguaaacaaggcaguggagcaguucagaaggcugcugacucaagaaaacagacgcgucacuaaguccgacccgaaccagcaccuuaccaucauccaagacccggaguaccgccgguucggcugcaccgucgauaugaacauagcccugaccacuuucaucccccaugacaaggggccggcggcaaucgaggaaugcuguaacugguuucauaagcggauggaggaacugaauuccgagaagcaccggcugauuaacuaccaccaggaacaggcagugaacugccugcugggcaacguguucuacgaacggcuggcuggacacggaccgaagcugggucccgugacuagaaagcauccgcucgucacucgcuacuucaccuucccguuugaggagauugacuucuccauggaagaauccaugauccacuugccgaacaaggcuugcuuccugauggcgcacaacggaugggucaugggcgacgacccgcugaggaauuucgcggagccggguucggaaguguaccugagaagggaacucauuugcuggggagacuccgucaagcugcgcuaugggaacaagcccgaggauugccccuaccugugggcucacaugaagaaguacacggaaaucaccgccacguacuuccagggaguccggcuggacaauugccacuccaccccccuccauguggccgaguacaugcuggaugcagcgcgcaaucugcagccgaaucuguacgugguugcagagcuguucacuggguccgaggaccucgacaacguguucgugacuagauuggggaucuccucccucauccgggaagccaugucggccuacaacucccaugaggaggggaggcugguguacagauacggcggcgaacccgugggaagcuucgugcagccgugccuccggccgcugaugccggccaucgcccacgcccuguucauggauaucacucacgacaacgaaugcccgaucgugcaucgcucggccuacgacgcacugccguccaccacuaucguguccauggcaugcugcgccuccgggagcacccgcggauacgaugagcucgugccgcaccagauuagcgugguguccgaagaacgcuucuauaccaaguggaaccccgaagcccugccguccaauaccggggaagugaacuuccaguccgguauuaucgccgcucgcugugcgaucucgaaacuccaccaagagcucggugccaagggguucauucaggucuacguggaucaggucgacgaggauauuguggcagugaccaggcacucaccuagcauccaccaauccguggucgccgugucacgcacugcguuucggaaccccaagaccucguucuacucgaaagaagugccgcagauguguaucccgggaaagaucgaagaggucgugcuggaagcacggaccauugagaggaacaccaagccuuaccggaaagacgagaacucuaucaacgggaccccggauaucacuguggagauucgcgaacacauccagcugaacgaaucaaagaucgucaagcaggcuggaguggccaccaagggacccaacgaguacauccaggagaucgaauuugaaaaccucuccccgggguccgugaucaucuuccgggugucccuggacccccacgcccaaguggccgugggaauucucagaaaccaccugacccaguucucaccccacuuuaagucggguucccuggccguggacaacgccgauccgauccucaagaucccguucgcgucgcuggccucccgccucacucucgcggaacugaaccagauccuguaccgcugugaaucagaggaaaaggaggacggcggcggcuguuacgauauuccgaauuggucggcuuugaaauacgcgggacuucaggggcugaugucuguccuggcggaaauccggccgaagaacgaccuggggcacccguucugcaacaacuugcggagcggagauuggaugaucgacuacgucagcaacagacugaucagccggagcggcacuaucgccgaggucggaaagugguugcaggccauguucuucuaccugaagcagaucccccgauaccucaucccguguuacuucgacgccauccugaucggggccuacaccacccuccuggacaccgccuggaagcagaugagcaguuuugugcaaaacggguccaccuucgugaagcaccuuucccugggcucagugcagcugugcggcgugggaaaguuccccucgcugcccauucugagcccggcccugauggacguccccuaccggcugaacgagaucaccaaggagaaggagcagugcugugugucccuggcugccgggcugccgcacuuuucguccggcaucuuccggugcugggggcgggauaccuucauugcccugcggggaauccuucuuaucaccggucgcuauguggaggcucggaacauuauucuggcguucgccggaacccugagacacgggcugauuccgaaccucuugggggaagggaucuacgcccgcuacaacugucgggacgccguguggugguggcuccagugcauucaggacuauugcaagauggugcccaacgggcuggacauccugaagugcccggugucgaggauguauccgaccgacgacagcgcaccccugccggccgggacccucgaccaaccccuguucgaagucauucaagaggcuaugcagaagcacaugcaggguauucaguuccgggaacggaacgcggggccccagauugauaggaacaugaaagacgaggguuucaacaucacugccggcguggacgaagaaaccgguuuuguguacggaggaaaccgguucaacugcgguaccuggauggauaagaugggagaaucagaucgcgcgcgcaacagagggaucccggcaaccccgcgggacggaucggcuguggaaauugugggacugagcaagagcgccgugcgguggcugcuggaacugagcaaaaagaacaucuuccccuaccacgaagugaccgugaagcggcacggaaaggccaucaaagucuccuacgaugaauggaauaggaagauccaggauaacuucgagaagcuuuuucacguguccgaggaucccuccgaucugaacgagaagcauccgaaucucgugcauaagagggggaucuacaaggacuccuacggagcguccuccccuuggugcgacuaucagcugcggccuaacuucaccauugccauggucguggccccggagcucuuuacaaccgagaaggccuggaaggcccucgaaauugccgaaaagaagcugcuggggcccuuggggaugaaaacccuggauccggacgacaugguguacugcggaaucuacgacaacgcccuggacaacgacaacuacaaucuggcgaagggcuucaauuaccaccaggggccggaauggcucuggccgauuggguacuuccugcgcgccaagcuguacuucucacggcugaugggaccggagacuaccgccaagaccaucguccucgugaagaacgugcugucgcggcacuacgugcaccuggagaggagccccuggaaggggcuucccgagcugacgaacgagaacgcgcaguacugucccuucuccugcgaaacccaagccugguccauugccacuauacuggaaaccuuauaugaccuguag

SEQ ID NO: 31 - RNA, 4599 nt, Artificial Sequence
  Codon-Optimized AGL Coding Sequence
augggccacagcaagcagauccggaucuugcugcugaacgagauggagaagcuggagaagacccuguucaggcuggagcagggcuacgagcugcaguuccgguugggccccaccuugcagggcaaggccgugaccguguacaccaacuaccccuuccccggcgaaaccuucaacagggagaaguuccggucccuggacugggagaaccccaccgagagggaggacgacuccgacaaguacugcaagcugaaccugcagcaguccggcuccuuccaguacuacuuccugcagggcaacgagaaaagcggcggcggcuacaucgugguggaccccaucuugcgggugggcgccgacaaccacgugcugcccuuggacugcgugacccugcagaccuucuuggccaagugcuugggccccuucgacgagugggagagcaggcugaggguggccaaggaguccggcuacaacaugauccacuucacccccuugcagacccugggccuguccagguccugcuacucccuggccaaccaguuggaguugaaccccgacuucuccaggcccaacaggaaguacaccuggaacgacgugggccagcugguggagaaguugaagaaggaguggaacgugaucugcaucaccgacgugguguacaaccacaccgccgccaacagcaaguggauccaggagcaccccgagugcgccuacaaccuggugaacuccccccacuugaagcccgccuggguguuggacagggcccuguggcgguucuccugcgacguggccgagggcaaguacaaggagaagggcauccccgccuugaucgagaacgaccaccacaugaacuccauccggaagaucaucugggaggacaucuuccccaagcugaagcugugggaguucuuccagguggacgugaacaaggccguggagcaguucaggaggcugcugacccaggagaacaggcgggugaccaaguccgaccccaaccagcaccugaccaucauccaggaccccgaguacaggcgguucggcugcaccguggacaugaacaucgcccugaccaccuucaucccccacgacaagggccccgccgccaucgaggagugcugcaacugguuccacaagaggauggaggaguugaacuccgagaagcaccggcugaucaacuaccaccaggagcaggccgugaacugccuguugggcaacguguucuacgagcggcuggccggccacggccccaagcugggccccgugaccaggaagcaccccuuggugaccagguacuucaccuuccccuucgaggagaucgacuucuccauggaggaguccaugauccaccugcccaacaaggccugcuuccugauggcccacaacggcugggugaugggcgacgacccccugcggaacuucgccgagcccggcuccgagguguaccugaggagggagcugaucugcuggggcgacagcgugaaguugcgguacggcaacaagcccgaggacugccccuaccugugggcccacaugaagaaguacaccgagaucaccgccaccuacuuccagggcgugcggcuggacaacugccacuccaccccccugcacguggccgaguacauguuggacgccgccaggaacuugcagcccaacuuguacgugguggccgagcuguucaccggcagcgaggaccuggacaacguguucgugaccaggcugggcaucagcuccuugaucagggaggccaugagcgccuacaacagccacgaggagggcagguugguguaccgguacggcggcgagcccgugggcuccuucgugcagcccugcuugaggcccuugaugcccgccaucgcccacgcccuguucauggacaucacccacgacaacgagugccccaucgugcacagguccgccuacgacgcccugcccagcaccaccaucguguccauggccugcugcgccagcggcagcaccaggggcuacgacgaguuggugccccaccagaucuccgugguguccgaggagcgguucuacaccaaguggaaccccgaggccuugcccuccaacaccggcgaggugaacuuccagagcggcaucaucgccgccaggugcgccaucagcaagcugcaccaggagcugggcgccaagggcuucauccagguguacguggaccagguggacgaggacaucguggccgugaccaggcacucccccagcauccaccaguccgugguggccguguccaggaccgccuucaggaaccccaagaccuccuucuacagcaaggaggugccccagaugugcauccccggcaagaucgaggagguggugcuggaggccaggaccaucgagaggaacaccaagcccuacaggaaggacgagaacuccaucaacggcacccccgacaucaccguggagaucagggagcacauccagcugaacgagagcaagaucgugaagcaggccggcguggccaccaagggccccaacgaguacauccaggagaucgaguucgagaacuugucccccggcagcgugaucaucuucagggugagccuggacccccacgcccagguggccgugggcauccugcggaaccaccugacccaguucagcccccacuucaaguccggcagccuggccguggacaacgccgaccccaucuugaagauccccuucgccucccuggccuccagguugaccuuggccgagcugaaccagauccuguaccggugcgaguccgaggagaaggaggacggcggcggcugcuacgacauccccaacugguccgcccugaaguacgccggccugcagggcuugauguccguguuggccgagaucaggcccaagaacgacuugggccaccccuucugcaacaacuugagguccggcgacuggaugaucgacuacgugagcaaccggcugaucucccgguccggcaccaucgccgaggugggcaagugguugcaggccauguucuucuaccugaagcagaucccccgguaccugauccccugcuacuucgacgccaucuugaucggcgccuacaccacccugcuggacaccgccuggaagcagauguccagcuucgugcagaacggcuccaccuucgugaagcaccuguccuugggcuccgugcagcugugcggcgugggcaaguuccccucccugcccauccugucccccgcccugauggacgugcccuacagguugaacgagaucaccaaggagaaggagcagugcugcgugucccuggccgccggcuugccccacuucuccuccggcaucuuccggugcuggggcagggacaccuucaucgcccugaggggcauccugcugaucaccggccgguacguggaggccaggaacaucaucuuggccuucgccggcacccugaggcacggccugauccccaaccugcugggcgagggcaucuacgccagguacaacugccgggacgccguguggugguggcugcagugcauccaggacuacugcaagauggugcccaacggccuggacauccugaagugccccguguccaggauguaccccaccgacgacuccgcccccuugcccgccggcacccuggaccagcccuuguucgaggugauccaggaggccaugcagaagcacaugcagggcauccaguuccgggagaggaacgccggcccccagaucgaccggaacaugaaggacgagggcuucaacaucaccgccggcguggacgaggaaaccggcuucguguacggcggcaaccgguucaacugcggcaccuggauggacaagaugggcgagagcgacagggccaggaacaggggcauccccgccacccccagggacggcuccgccguggagaucgugggccugagcaaguccgccgugcggugguugcuggaguuguccaagaagaacaucuuccccuaccacgaggugaccgugaagaggcacggcaaggccaucaagguguccuacgacgaguggaacaggaagauccaggacaacuucgagaagcuguuccacguguccgaggaccccuccgacuugaacgagaagcaccccaaccuggugcacaagcggggcaucuacaaggacagcuacggcgccuccagccccuggugcgacuaccagcugaggcccaacuucaccaucgccauggugguggcccccgagcuguucaccaccgagaaggccuggaaggccuuggagaucgccgagaagaaguugcugggcccccugggcaugaagaccuuggaccccgacgacaugguguacugcggcaucuacgacaacgccuuggacaacgacaacuacaaccuggccaagggcuucaacuaccaccagggccccgaguggcuguggcccaucggcuacuuccugcgggccaaguuguacuucuccagguugaugggccccgaaaccaccgccaagaccaucguguuggugaagaacgugcugucccggcacuacgugcaccuggagaggucccccuggaagggccugcccgagcugaccaacgagaacgcccaguacugccccuucagcugcgaaacccaggccugguccaucgccaccauccuggaaacccuguacgacuuguag

SEQ ID NO: 32 - RNA, 4599 nt, Artificial Sequence
  Codon-Optimized AGL Coding Sequence
augggacauagcaagcagauccggaucuugcugcugaaugaaauggaaaagcuggaaaagacccuguucagacuggaacagggauacgaacugcaguuccgguugggaccuaccuugcagggaaaggcugugaccguguacaccaauuacccuuucccuggagaaaccuucaauagagaaaaguucagaucucuagauugggaaaauccuaccgaaagagaagaugauucugauaaguacugcaagcugaaucugcagcagucuggaucuuuccaguacuacuuccugcagggaaaugaaaagagcggaggaggauacaucgugguggauccuaucuugcgggugggagcugauaaucaugugcugccuuuggauugcgugacccugcagaccuucuuggcuaagugcuugggaccuuucgaugaaugggaaagcagacugagaguggcuaaggaaucuggauacaauaugauccauuucaccccuuugcagacccugggacugucuagaucuugcuacucucuggcuaaucaguuggaauugaauccugauuucucuagaccuaauagaaaguacaccuggaaugaugugggacagcugguggaaaaguugaagaaggaauggaaugugaucugcaucaccgaugugguguacaaucauaccgcugcuaauagcaaguggauccaggaacauccugaaugcgcuuacaaucuggugaauucuccucauuugaagccugcuuggguguuggauagagcucuguggcgguucucuugcgauguggcugaaggaaaguacaaggaaaagggaaucccugcuuugaucgaaaaugaucaucauaugaauucuauccggaagaucaucugggaagauaucuucccuaagcugaagcugugggaauucuuccagguggaugugaauaaggcuguggaacaguucagaagacugcugacccaggaaaauagacgggugaccaagucugauccuaaucagcaucugaccaucauccaggauccugaauacagacgguucggaugcaccguggauaugaauaucgcucugaccaccuucaucccucaugauaagggaccugcugcuaucgaagaaugcugcaauugguuccauaagagaauggaagaauugaauucugaaaagcaucggcugaucaauuaccaucaggaacaggcugugaauugccuguugggaaauguguucuacgaacggcuggcuggacauggaccuaagcugggaccugugaccagaaagcauccuuuggugaccagauacuucaccuucccuuucgaagaaaucgauuucucuauggaagaaucuaugauccaucugccuaauaaggcuugcuuccugauggcucauaauggaugggugaugggagaugauccucugcggaauuucgcugaaccuggaucugaaguguaccugagaagagaacugaucugcuggggagauagcgugaaguugcgguacggaaauaagccugaagauugcccuuaccugugggcucauaugaagaaguacaccgaaaucaccgcuaccuacuuccagggagugcggcuggauaauugccauucuaccccucugcauguggcugaauacauguuggaugcugcuagaaauuugcagccuaauuuguacgugguggcugaacuguucaccggaagcgaagaucuggauaauguguucgugaccagacugggaaucagcucuuugaucagagaagcuaugagcgcuuacaauagccaugaagaaggaagauugguguaccgguacggaggagaaccugugggaucuuucgugcagccuugcuugaggccuuugaugccugcuaucgcucaugcucuguucauggauaucacccaugauaaugaaugcccuaucgugcauagaucugcuuacgaugcucugccuagcaccaccaucgugucuauggcuugcugcgcuagcggaagcaccagaggauacgaugaauuggugccucaucagaucucuguggugucugaagaacgguucuacaccaaguggaauccugaagcuuugccuucuaauaccggagaagugaauuuccagagcggaaucaucgcugcuagaugcgcuaucagcaagcugcaucaggaacugggagcuaagggauucauccagguguacguggaucagguggaugaagauaucguggcugugaccagacauucuccuagcauccaucagucugugguggcugugucuagaaccgcuuucagaaauccuaagaccucuuucuacagcaaggaagugccucagaugugcaucccuggaaagaucgaagaaguggugcuggaagcuagaaccaucgaaagaaauaccaagccuuacagaaaggaugaaaauucuaucaauggaaccccugauaucaccguggaaaucagagaacauauccagcugaaugaaagcaagaucgugaagcaggcuggaguggcuaccaagggaccuaaugaauacauccaggaaaucgaauucgaaaauuugucuccuggaagcgugaucaucuucagagugagccuggauccucaugcucagguggcugugggaauccugcggaaucaucugacccaguucagcccucauuucaagucuggaagccuggcuguggauaaugcugauccuaucuugaagaucccuuucgcuucucuggcuucuagauugaccuuggcugaacugaaucagauccuguaccggugcgaaucugaagaaaaggaagauggaggaggaugcuacgauaucccuaauuggucugcucugaaguacgcuggacugcagggauugaugucuguguuggcugaaaucagaccuaagaaugauuugggacauccuuucugcaauaauuugagaucuggagauuggaugaucgauuacgugagcaaucggcugaucucucggucuggaaccaucgcugaagugggaaagugguugcaggcuauguucuucuaccugaagcagaucccucgguaccugaucccuugcuacuucgaugcuaucuugaucggagcuuacaccacccugcuggauaccgcuuggaagcagaugucuagcuucgugcagaauggaucuaccuucgugaagcaucugucuuugggaucugugcagcugugcggagugggaaaguucccuucucugccuauccugucuccugcucugauggaugugccuuacagauugaaugaaaucaccaaggaaaaggaacagugcugcgugucucuggcugcuggauugccucauuucucuucuggaaucuuccggugcuggggaagagauaccuucaucgcucugagaggaauccugcugaucaccggacgguacguggaagcuagaaauaucaucuuggcuuucgcuggaacccugagacauggacugaucccuaaucugcugggagaaggaaucuacgcuagauacaauugccgggaugcuguguggugguggcugcagugcauccaggauuacugcaagauggugccuaauggacuggauauccugaagugcccugugucuagaauguacccuaccgaugauucugcuccuuugccugcuggaacccuggaucagccuuuguucgaagugauccaggaagcuaugcagaagcauaugcagggaauccaguuccgggaaagaaaugcuggaccucagaucgaucggaauaugaaggaugaaggauucaauaucaccgcuggaguggaugaagaaaccggauucguguacggaggaaaucgguucaauugcggaaccuggauggauaagaugggagaaagcgauagagcuagaaauagaggaaucccugcuaccccuagagauggaucugcuguggaaaucgugggacugagcaagucugcugugcggugguugcuggaauugucuaagaagaauaucuucccuuaccaugaagugaccgugaagagacauggaaaggcuaucaaggugucuuacgaugaauggaauagaaagauccaggauaauuucgaaaagcuguuccaugugucugaagauccuucugauuugaaugaaaagcauccuaaucuggugcauaagcggggaaucuacaaggauagcuacggagcuucuagcccuuggugcgauuaccagcugaggccuaauuucaccaucgcuauggugguggcuccugaacuguucaccaccgaaaaggcuuggaaggcuuuggaaaucgcugaaaagaaguugcugggaccucugggaaugaagaccuuggauccugaugauaugguguacugcggaaucuacgauaaugcuuuggauaaugauaauuacaaucuggcuaagggauucaauuaccaucagggaccugaauggcuguggccuaucggauacuuccugcgggcuaaguuguacuucucuagauugaugggaccugaaaccaccgcuaagaccaucguguuggugaagaaugugcugucucggcauuacgugcaucuggaaagaucuccuuggaagggacugccugaacugaccaaugaaaaugcucaguacugcccuuucagcugcgaaacccaggcuuggucuaucgcuaccauccuggaaacccuguacgauuuguag

SEQ ID NO: 33 - RNA, 158 nt, Artificial Sequence
  Modified Xenopus beta-globin 3'UTR
  misc_feature (2)..(2): n is unlocked nucleomonomer UNA-U
  misc_feature (157)..(157): n is unlocked nucleomonomer UNA-A
cnagugacugacuaggaucugguuaccacuaaaccagccucaagaacacccgaauggagucucuaagcuacauaauaccaacuuacacuuacaaaauguugucccccaaaauguagccauucguaucugcuccuaauaaaaagaaaguuucuucacnu

SEQ ID NO: 34 - RNA, 158 nt, Artificial Sequence
  Modified Xenopus beta-globin 3'UTR
  misc_feature (2)..(2): n is unlocked nucleomonomer UNA-U
  misc_feature (3)..(3): n is unlocked nucleomonomer UNA-A
  misc_feature (4)..(4): n is unlocked nucleomonomer UNA-G
  misc_feature (155)..(155): n is unlocked nucleomonomer UNA-A
  misc_feature (156)..(156): n is unlocked nucleomonomer UNA-C
  misc_feature (157)..(157): n is unlocked nucleomonomer UNA-A
cnnnugacugacuaggaucugguuaccacuaaaccagccucaagaacacccgaauggagucucuaagcuacauaauaccaacuuacacuuacaaaauguugucccccaaaauguagccauucguaucugcuccuaauaaaaagaaaguuucuucnnnu

SEQ ID NO: 35 - RNA, 158 nt, Artificial Sequence
  Modified Xenopus beta-globin 3'UTR
  misc_feature (2)..(2): n is unlocked nucleomonomer UNA-U
  misc_feature (8)..(8): n is unlocked nucleomonomer UNA-C
  misc_feature (14)..(14): n is unlocked nucleomonomer UNA-A
  misc_feature (20)..(20): n is unlocked nucleomonomer UNA-U
  misc_feature (26)..(26): n is unlocked nucleomonomer UNA-C
  misc_feature (32)..(32): n is unlocked nucleomonomer UNA-A
  misc_feature (38)..(38): n is unlocked nucleomonomer UNA-C
  misc_feature (44)..(44): n is unlocked nucleomonomer UNA-G
  misc_feature (50)..(50): n is unlocked nucleomonomer UNA-C
  misc_feature (56)..(56): n is unlocked nucleomonomer UNA-G
  misc_feature (62)..(62): n is unlocked nucleomonomer UNA-U
  misc_feature (68)..(68): n is unlocked nucleomonomer UNA-C
  misc_feature (74)..(74): n is unlocked nucleomonomer UNA-A
  misc_feature (80)..(80): n is unlocked nucleomonomer UNA-A
  misc_feature (86)..(86): n is unlocked nucleomonomer UNA-C
  misc_feature (92)..(92): n is unlocked nucleomonomer UNA-C
  misc_feature (98)..(98): n is unlocked nucleomonomer UNA-G
  misc_feature (104)..(104): n is unlocked nucleomonomer UNA-C
  misc_feature (110)..(110): n is unlocked nucleomonomer UNA-A
  misc_feature (116)..(116): n is unlocked nucleomonomer UNA-G
  misc_feature (122)..(122): n is unlocked nucleomonomer UNA-C
  misc_feature (128)..(128): n is unlocked nucleomonomer UNA-U
  misc_feature (134)..(134): n is unlocked nucleomonomer UNA-U
  misc_feature (140)..(140): n is unlocked nucleomonomer UNA-A
  misc_feature (146)..(146): n is unlocked nucleomonomer UNA-A
  misc_feature (152)..(152): n is unlocked nucleomonomer UNA-U
  misc_feature (157)..(157): n is unlocked nucleomonomer UNA-A
cnaguganugacunggaucngguuancacuanaccagncucaanaacacncgaaungagucncuaagnuacaunauaccnacuuanacuuanaaaaunuugucncccaanauguanccauunguaucngcuccnaauaanaagaanguuucnucacnu

SEQ ID NO: 36 - RNA, 158 nt, Artificial Sequence
  Modified Xenopus beta-globin 3'UTR
  misc_feature (2)..(2): n is unlocked nucleomonomer UNA-U
  misc_feature (3)..(3): n is unlocked nucleomonomer UNA-A
  misc_feature (8)..(8): n is unlocked nucleomonomer UNA-C
  misc_feature (9)..(9): n is unlocked nucleomonomer UNA-U
  misc_feature (14)..(14): n is unlocked nucleomonomer UNA-A
  misc_feature (15)..(15): n is unlocked nucleomonomer UNA-G
  misc_feature (20)..(20): n is unlocked nucleomonomer UNA-U
  misc_feature (21)..(21): n is unlocked nucleomonomer UNA-G
  misc_feature (26)..(27): n is unlocked nucleomonomer UNA-C
  misc_feature (32)..(33): n is unlocked nucleomonomer UNA-A
  misc_feature (38)..(39): n is unlocked nucleomonomer UNA-C
  misc_feature (44)..(44): n is unlocked nucleomonomer UNA-G
  misc_feature (45)..(45): n is unlocked nucleomonomer UNA-A
  misc_feature (50)..(51): n is unlocked nucleomonomer UNA-C
  misc_feature (56)..(57): n is unlocked nucleomonomer UNA-G
  misc_feature (62)..(62): n is unlocked nucleomonomer UNA-U
  misc_feature (63)..(63): n is unlocked nucleomonomer UNA-C
  misc_feature (68)..(68): n is unlocked nucleomonomer UNA-C
  misc_feature (69)..(69): n is unlocked nucleomonomer UNA-U
  misc_feature (74)..(75): n is unlocked nucleomonomer UNA-A
  misc_feature (80)..(81): n is unlocked nucleomonomer UNA-A
  misc_feature (86)..(86): n is unlocked nucleomonomer UNA-C
  misc_feature (87)..(87): n is unlocked nucleomonomer UNA-A
  misc_feature (92)..(92): n is unlocked nucleomonomer UNA-C
  misc_feature (93)..(93): n is unlocked nucleomonomer UNA-A
  misc_feature (98)..(98): n is unlocked nucleomonomer UNA-G
  misc_feature (99)..(99): n is unlocked nucleomonomer UNA-U
  misc_feature (104)..(105): n is unlocked nucleomonomer UNA-C
  misc_feature (110)..(111): n is unlocked nucleomonomer UNA-A
  misc_feature (116)..(116): n is unlocked nucleomonomer UNA-G
  misc_feature (117)..(117): n is unlocked nucleomonomer UNA-C
  misc_feature (122)..(122): n is unlocked nucleomonomer UNA-C
  misc_feature (123)..(123): n is unlocked nucleomonomer UNA-G
  misc_feature (128)..(128): n is unlocked nucleomonomer UNA-U
  misc_feature (129)..(129): n is unlocked nucleomonomer UNA-G
  misc_feature (134)..(134): n is unlocked nucleomonomer UNA-U
  misc_feature (135)..(135): n is unlocked nucleomonomer UNA-A
  misc_feature (140)..(141): n is unlocked nucleomonomer UNA-A
  misc_feature (146)..(146): n is unlocked nucleomonomer UNA-A
  misc_feature (147)..(147): n is unlocked nucleomonomer UNA-G
  misc_feature (152)..(153): n is unlocked nucleomonomer UNA-U
  misc_feature (157)..(157): n is unlocked nucleomonomer UNA-A
cnnguganngacunngaucnnguuannacuannccagnnucaannacacnngaaunnagucnnuaagnnacaunnuaccnncuuanncuuannaaaunnugucnnccaannuguanncauunnuaucnncuccnnauaannagaannuuucnncacnu

SEQ ID NO: 37 - RNA, 158 nt, Artificial Sequence
  Modified Xenopus beta-globin 3'UTR
  misc_feature (1)..(1): n is unlocked nucleomonomer UNA-C
  misc_feature (2)..(2): n is unlocked nucleomonomer UNA-U
  misc_feature (3)..(3): n is unlocked nucleomonomer UNA-A
  misc_feature (4)..(4): n is unlocked nucleomonomer UNA-G
  misc_feature (5)..(5): n is unlocked nucleomonomer UNA-U
  misc_feature (6)..(6): n is unlocked nucleomonomer UNA-G
  misc_feature (7)..(7): n is unlocked nucleomonomer UNA-A
  misc_feature (8)..(8): n is unlocked nucleomonomer UNA-C
  misc_feature (9)..(9): n is unlocked nucleomonomer UNA-U
  misc_feature (10)..(10): n is unlocked nucleomonomer UNA-G
  misc_feature (11)..(11): n is unlocked nucleomonomer UNA-A
  misc_feature (12)..(12): n is unlocked nucleomonomer UNA-C
  misc_feature (13)..(13): n is unlocked nucleomonomer UNA-U
  misc_feature (14)..(14): n is unlocked nucleomonomer UNA-A
  misc_feature (15)..(16): n is unlocked nucleomonomer UNA-G
  misc_feature (17)..(17): n is unlocked nucleomonomer UNA-A
  misc_feature (18)..(18): n is unlocked nucleomonomer UNA-U
  misc_feature (19)..(19): n is unlocked nucleomonomer UNA-C
  misc_feature (20)..(20): n is unlocked nucleomonomer UNA-U
  misc_feature (21)..(22): n is unlocked nucleomonomer UNA-G
  misc_feature (23)..(24): n is unlocked nucleomonomer UNA-U
  misc_feature (25)..(25): n is unlocked nucleomonomer UNA-A
  misc_feature (26)..(27): n is unlocked nucleomonomer UNA-C
  misc_feature (28)..(28): n is unlocked nucleomonomer UNA-A
  misc_feature (29)..(29): n is unlocked nucleomonomer UNA-C
  misc_feature (30)..(30): n is unlocked nucleomonomer UNA-U
  misc_feature (31)..(33): n is unlocked nucleomonomer UNA-A
  misc_feature (34)..(35): n is unlocked nucleomonomer UNA-C
  misc_feature (36)..(36): n is unlocked nucleomonomer UNA-A
  misc_feature (37)..(37): n is unlocked nucleomonomer UNA-G
  misc_feature (38)..(39): n is unlocked nucleomonomer UNA-C
  misc_feature (40)..(40): n is unlocked nucleomonomer UNA-U
  misc_feature (41)..(41): n is unlocked nucleomonomer UNA-C
  misc_feature (42)..(43): n is unlocked nucleomonomer UNA-A
  misc_feature (44)..(44): n is unlocked nucleomonomer UNA-G
  misc_feature (45)..(46): n is unlocked nucleomonomer UNA-A
  misc_feature (47)..(47): n is unlocked nucleomonomer UNA-C
  misc_feature (48)..(48): n is unlocked nucleomonomer UNA-A
  misc_feature (49)..(51): n is unlocked nucleomonomer UNA-C
  misc_feature (52)..(52): n is unlocked nucleomonomer UNA-G
  misc_feature (53)..(54): n is unlocked nucleomonomer UNA-A
  misc_feature (55)..(55): n is unlocked nucleomonomer UNA-U
  misc_feature (56)..(57): n is unlocked nucleomonomer UNA-G
  misc_feature (58)..(58): n is unlocked nucleomonomer UNA-A
  misc_feature (59)..(59): n is unlocked nucleomonomer UNA-G
  misc_feature (60)..(60): n is unlocked nucleomonomer UNA-U
  misc_feature (61)..(61): n is unlocked nucleomonomer UNA-C
  misc_feature (62)..(62): n is unlocked nucleomonomer UNA-U
  misc_feature (63)..(63): n is unlocked nucleomonomer UNA-C
  misc_feature (64)..(64): n is unlocked nucleomonomer UNA-U
  misc_feature (65)..(66): n is unlocked nucleomonomer UNA-A
  misc_feature (67)..(67): n is unlocked nucleomonomer UNA-G
  misc_feature (68)..(68): n is unlocked nucleomonomer UNA-C
  misc_feature (69)..(69): n is unlocked nucleomonomer UNA-U
  misc_feature (70)..(70): n is unlocked nucleomonomer UNA-A
  misc_feature (71)..(71): n is unlocked nucleomonomer UNA-C
  misc_feature (72)..(72): n is unlocked nucleomonomer UNA-A
  misc_feature (73)..(73): n is unlocked nucleomonomer UNA-U
  misc_feature (74)..(75): n is unlocked nucleomonomer UNA-A
  misc_feature (76)..(76): n is unlocked nucleomonomer UNA-U
  misc_feature (77)..(77): n is unlocked nucleomonomer UNA-A
  misc_feature (78)..(79): n is unlocked nucleomonomer UNA-C
  misc_feature (80)..(81): n is unlocked nucleomonomer UNA-A
  misc_feature (82)..(82): n is unlocked nucleomonomer UNA-C
  misc_feature (83)..(84): n is unlocked nucleomonomer UNA-U
  misc_feature (85)..(85): n is unlocked nucleomonomer UNA-A
  misc_feature (86)..(86): n is unlocked nucleomonomer UNA-C
  misc_feature (87)..(87): n is unlocked nucleomonomer UNA-A
  misc_feature (88)..(88): n is unlocked nucleomonomer UNA-C
  misc_feature (89)..(90): n is unlocked nucleomonomer UNA-U
  misc_feature (91)..(91): n is unlocked nucleomonomer UNA-A
  misc_feature (92)..(92): n is unlocked nucleomonomer UNA-C
  misc_feature (93)..(96): n is unlocked nucleomonomer UNA-A
  misc_feature (97)..(97): n is unlocked nucleomonomer UNA-U
  misc_feature (98)..(98): n is unlocked nucleomonomer UNA-G
  misc_feature (99)..(100): n is unlocked nucleomonomer UNA-U
  misc_feature (101)..(101): n is unlocked nucleomonomer UNA-G
  misc_feature (102)..(102): n is unlocked nucleomonomer UNA-U
  misc_feature (103)..(107): n is unlocked nucleomonomer UNA-C
  misc_feature (108)..(111): n is unlocked nucleomonomer UNA-A
  misc_feature (112)..(112): n is unlocked nucleomonomer UNA-U
  misc_feature (113)..(113): n is unlocked nucleomonomer UNA-G
  misc_feature (114)..(114): n is unlocked nucleomonomer UNA-U
  misc_feature (115)..(115): n is unlocked nucleomonomer UNA-A
  misc_feature (116)..(116): n is unlocked nucleomonomer UNA-G
  misc_feature (117)..(118): n is unlocked nucleomonomer UNA-C
  misc_feature (119)..(119): n is unlocked nucleomonomer UNA-A
  misc_feature (120)..(121): n is unlocked nucleomonomer UNA-U
  misc_feature (122)..(122): n is unlocked nucleomonomer UNA-C
  misc_feature (123)..(123): n is unlocked nucleomonomer UNA-G
  misc_feature (124)..(124): n is unlocked nucleomonomer UNA-U
  misc_feature (125)..(125): n is unlocked nucleomonomer UNA-A
  misc_feature (126)..(126): n is unlocked nucleomonomer UNA-U
  misc_feature (127)..(127): n is unlocked nucleomonomer UNA-C
  misc_feature (128)..(128): n is unlocked nucleomonomer UNA-U
  misc_feature (129)..(129): n is unlocked nucleomonomer UNA-G
  misc_feature (130)..(130): n is unlocked nucleomonomer UNA-C
  misc_feature (131)..(131): n is unlocked nucleomonomer UNA-U
  misc_feature (132)..(133): n is unlocked nucleomonomer UNA-C
  misc_feature (134)..(134): n is unlocked nucleomonomer UNA-U
  misc_feature (135)..(136): n is unlocked nucleomonomer UNA-A
  misc_feature (137)..(137): n is unlocked nucleomonomer UNA-U
  misc_feature (138)..(142): n is unlocked nucleomonomer UNA-A
  misc_feature (143)..(143): n is unlocked nucleomonomer UNA-G
  misc_feature (144)..(146): n is unlocked nucleomonomer UNA-A
  misc_feature (147)..(147): n is unlocked nucleomonomer UNA-G
  misc_feature (148)..(149): n is unlocked nucleomonomer UNA-U
  misc_feature (150)..(150): n is unlocked nucleomonomer UNA-U
  misc_feature (151)..(151): n is unlocked nucleomonomer UNA-C
  misc_feature (152)..(153): n is unlocked nucleomonomer UNA-U
  misc_feature (154)..(154): n is unlocked nucleomonomer UNA-C
  misc_feature (155)..(155): n is unlocked nucleomonomer UNA-A
  misc_feature (156)..(156): n is unlocked nucleomonomer UNA-C
  misc_feature (157)..(157): n is unlocked nucleomonomer UNA-A
  misc_feature (158)..(158): n is unlocked nucleomonomer UNA-U
nnnnnnnnnnnnnnnnnnnnnnnnnnnnnnnnnnnnnnnnnnnnnnnnnnnnnnnnnnnnnnnnnnnnnnnnnnnnnnnnnnnnnnnnnnnnnnnnnnnnnnnnnnnnnnnnnnnnnnnnnnnnnnnnnnnnnnnnnnnnnnnnnnnnnnnnnnnnnn

SEQ ID NO: 38 - RNA, 100 nt, Unknown
  Poly(A) 100 Tail
aaaaaaaaaaaaaaaaaaaaaaaaaaaaaaaaaaaaaaaaaaaaaaaaaaaaaaaaaaaaaaaaaaaaaaaaaaaaaaaaaaaaaaaaaaaaaaaaaaaa

SEQ ID NO: 39 - RNA, 110 nt, Unknown
  Poly(A) 110 Tail
aaaaaaaaaaaaaaaaaaaaaaaaaaaaaaaaaaaaaaaaaaaaaaaaaaaaaaaaaaaaaaaaaaaaaaaaaaaaaaaaaaaaaaaaaaaaaaaaaaaaaaaaaaaaaa

SEQ ID NO: 40 - RNA, 9 nt, Unknown
  Triple Stop Codon
auaagugaa

SEQ ID NO: 41 - RNA, 4599 nt, Artificial Sequence
  Codon-Optimized AGL Coding Sequence
augggccacagcaagcagauccggauccugcugcugaacgagauggagaagcuggagaagacccuguuccggcuggagcagggcuacgagcugcaguuccggcugggccccacccugcagggcaaggccgugaccguguacaccaacuaccccuuccccggcgagaccuucaaccgggagaaguuccggagccuggacugggagaaccccaccgagcgggaggacgacagcgacaaguacugcaagcugaaccugcagcagagcggcagcuuccaguacuacuuccugcagggcaacgagaagagcggcggcggcuacaucgugguggaccccauccugcgggugggcgccgacaaccacgugcugccccuggacugcgugacccugcagaccuuccuggccaagugccugggccccuucgacgagugggagagccggcugcggguggccaaggagagcggcuacaacaugauccacuucaccccccugcagacccugggccugagccggagcugcuacagccuggccaaccagcuggagcugaaccccgacuucagccggcccaaccggaaguacaccuggaacgacgugggccagcugguggagaagcugaagaaggaguggaacgugaucugcaucaccgacgugguguacaaccacaccgccgccaacagcaaguggauccaggagcaccccgagugcgccuacaaccuggugaacagcccccaccugaagcccgccugggugcuggaccgggcccuguggcgguucagcugcgacguggccgagggcaaguacaaggagaagggcauccccgcccugaucgagaacgaccaccacaugaacagcauccggaagaucaucugggaggacaucuuccccaagcugaagcugugggaguucuuccagguggacgugaacaaggccguggagcaguuccggcggcugcugacccaggagaaccggcgggugaccaagagcgaccccaaccagcaccugaccaucauccaggaccccgaguaccggcgguucggcugcaccguggacaugaacaucgcccugaccaccuucaucccccacgacaagggccccgccgccaucgaggagugcugcaacugguuccacaagcggauggaggagcugaacagcgagaagcaccggcugaucaacuaccaccaggagcaggccgugaacugccugcugggcaacguguucuacgagcggcuggccggccacggccccaagcugggccccgugacccggaagcacccccuggugacccgguacuucaccuuccccuucgaggagaucgacuucagcauggaggagagcaugauccaccugcccaacaaggccugcuuccugauggcccacaacggcugggugaugggcgacgacccccugcggaacuucgccgagcccggcagcgagguguaccugcggcgggagcugaucugcuggggcgacagcgugaagcugcgguacggcaacaagcccgaggacugccccuaccugugggcccacaugaagaaguacaccgagaucaccgccaccuacuuccagggcgugcggcuggacaacugccacagcaccccccugcacguggccgaguacaugcuggacgccgcccggaaccugcagcccaaccuguacgugguggccgagcuguucaccggcagcgaggaccuggacaacguguucgugacccggcugggcaucagcagccugauccgggaggccaugagcgccuacaacagccacgaggagggccggcugguguaccgguacggcggcgagcccgugggcagcuucgugcagcccugccugcggccccugaugcccgccaucgcccacgcccuguucauggacaucacccacgacaacgagugccccaucgugcaccggagcgccuacgacgcccugcccagcaccaccaucgugagcauggccugcugcgccagcggcagcacccggggcuacgacgagcuggugccccaccagaucagcguggugagcgaggagcgguucuacaccaaguggaaccccgaggcccugcccagcaacaccggcgaggugaacuuccagagcggcaucaucgccgcccggugcgccaucagcaagcugcaccaggagcugggcgccaagggcuucauccagguguacguggaccagguggacgaggacaucguggccgugacccggcacagccccagcauccaccagagcgugguggccgugagccggaccgccuuccggaaccccaagaccagcuucuacagcaaggaggugccccagaugugcauccccggcaagaucgaggagguggugcuggaggcccggaccaucgagcggaacaccaagcccuaccggaaggacgagaacagcaucaacggcacccccgacaucaccguggagauccgggagcacauccagcugaacgagagcaagaucgugaagcaggccggcguggccaccaagggccccaacgaguacauccaggagaucgaguucgagaaccugagccccggcagcgugaucaucuuccgggugagccuggacccccacgcccagguggccgugggcauccugcggaaccaccugacccaguucagcccccacuucaagagcggcagccuggccguggacaacgccgaccccauccugaagauccccuucgccagccuggccagccggcugacccuggccgagcugaaccagauccuguaccggugcgagagcgaggagaaggaggacggcggcggcugcuacgacauccccaacuggagcgcccugaaguacgccggccugcagggccugaugagcgugcuggccgagauccggcccaagaacgaccugggccaccccuucugcaacaaccugcggagcggcgacuggaugaucgacuacgugagcaaccggcugaucagccggagcggcaccaucgccgaggugggcaaguggcugcaggccauguucuucuaccugaagcagaucccccgguaccugauccccugcuacuucgacgccauccugaucggcgccuacaccacccugcuggacaccgccuggaagcagaugagcagcuucgugcagaacggcagcaccuucgugaagcaccugagccugggcagcgugcagcugugcggcgugggcaaguuccccagccugcccauccugagccccgcccugauggacgugcccuaccggcugaacgagaucaccaaggagaaggagcagugcugcgugagccuggccgccggccugccccacuucagcagcggcaucuuccggugcuggggccgggacaccuucaucgcccugcggggcauccugcugaucaccggccgguacguggaggcccggaacaucauccuggccuucgccggcacccugcggcacggccugauccccaaccugcugggcgagggcaucuacgcccgguacaacugccgggacgccguguggugguggcugcagugcauccaggacuacugcaagauggugcccaacggccuggacauccugaagugccccgugagccggauguaccccaccgacgacagcgccccccugcccgccggcacccuggaccagccccuguucgaggugauccaggaggccaugcagaagcacaugcagggcauccaguuccgggagcggaacgccggcccccagaucgaccggaacaugaaggacgagggcuucaacaucaccgccggcguggacgaggagaccggcuucguguacggcggcaaccgguucaacugcggcaccuggauggacaagaugggcgagagcgaccgggcccggaaccggggcauccccgccaccccccgggacggcagcgccguggagaucgugggccugagcaagagcgccgugcgguggcugcuggagcugagcaagaagaacaucuuccccuaccacgaggugaccgugaagcggcacggcaaggccaucaaggugagcuacgacgaguggaaccggaagauccaggacaacuucgagaagcuguuccacgugagcgaggaccccagcgaccugaacgagaagcaccccaaccuggugcacaagcggggcaucuacaaggacagcuacggcgccagcagccccuggugcgacuaccagcugcggcccaacuucaccaucgccauggugguggcccccgagcuguucaccaccgagaaggccuggaaggcccuggagaucgccgagaagaagcugcugggcccccugggcaugaagacccuggaccccgacgacaugguguacugcggcaucuacgacaacgcccuggacaacgacaacuacaaccuggccaagggcuucaacuaccaccagggccccgaguggcuguggcccaucggcuacuuccugcgggccaagcuguacuucagccggcugaugggccccgagaccaccgccaagaccaucgugcuggugaagaacgugcugagccggcacuacgugcaccuggagcggagccccuggaagggccugcccgagcugaccaacgagaacgcccaguacugccccuucagcugcgagacccaggccuggagcaucgccaccauccuggagacccuguacgaccuguag

SEQ ID NO: 42 - RNA, 4599 nt, Artificial Sequence
  Codon-Optimized AGL Coding Sequence
augggccauagcaagcagauccggauccuccugcucaaugagauggaaaagcucgagaaaacccucuuuaggcuggagcaaggcuacgaacuccaguuucggcucgggcccacucuccagggcaaggccgugaccgucuacaccaacuaucccuucccuggcgagaccuucaacagggagaaguuucggucccucgacugggagaaccccaccgagagggaggacgacuccgacaaguauugcaagcugaaccuccaacaauccggguccuuccaguacuacuuucugcaaggcaacgaaaagagcgggggcggguauauuguggucgaucccauccuccgggugggggcugacaaccacguccucccccuggauugcgugacucugcagaccuuccucgcuaaaugccugggcccuuucgacgagugggagagcaggcugcggguggccaaggaguccggguauaauaugauccacuucaccccccugcagacucugggccucucccgguccuguuauagccuggccaaccagcucgagcucaacccugauuucuccaggccuaacaggaaauacaccuggaacgacgugggccagcucgucgagaagcucaagaaagaguggaacgugaucugcaucacugacguggucuauaaccacacugcugcuaacagcaaguggauucaggagcaccccgagugcgccuacaaccuggucaacuccccccaucucaagccugccuggguccucgauagggcccuguggcgguuuagcugcgacguggccgagggcaaguauaaggagaaaggcauuccugcucugaucgagaacgaccaucacaugaacagcauucggaagauuaucugggaagacaucuuccccaaacugaagcucugggaguucuuucaagucgacgucaauaaggcuguggaacaauucaggaggcugcugacccaagagaaccggcgggucaccaaauccgaccccaaucaacaucugacuaucauccaagacccugaguauaggcgguucgggugcacugucgacaugaauaucgcccucacuacuuuuauuccccacgauaaaggccccgccgccaucgaggaguguugcaacugguuccacaagaggauggaagagcucaacuccgaaaaacaccggcucaucaauuaccaccaggagcaggccgugaacugucugcugggcaacgucuucuacgagcggcucgcugggcacgggcccaagcucggcccugucacuaggaaacacccucucgugacccgguacuucacuuuucccuucgaggaaauugauuuuagcauggaggaguccaugauccaccuccccaacaaggcuugcuuccucauggcccauaacggcugggucaugggcgacgacccucugcggaauuucgcugagcccggguccgagguguaucuccggagggagcugaucuguuggggcgauagcgugaagcuccgguacggcaacaagcccgaagauugcccuuaccucugggcccauaugaagaaguauacugagauuacugccacuuacuuucagggcguccggcuggacaauugucauuccaccccucugcaugucgcugaauauaugcuggacgcugcucggaaccugcaacccaaccucuacgucgucgcugagcucuuuaccggcagcgaggaccucgauaacgucuucgugacuaggcucgggaucagcagccucauuagggaagccaugagcgccuacaacagccacgaggaagggaggcucguguaucgguacggcggcgagccugugggcagcuucgugcagcccugccugcggccucucaugcccgcuaucgcccacgcccucuucauggacaucacucacgacaacgaaugcccuaucguccacagguccgcuuacgacgcucugcccagcacuaccaucguguccauggccugcugcgcuagcggcagcaccaggggguacgacgagcucgucccucaccagaucuccgucguguccgaggagcgguucuauacuaaauggaacccugaggcccugccuuccaauaccggggaggugaacuuucaaagcgggaucaucgccgcccggugcgcuauuagcaagcugcaccaggaacugggcgccaaaggguucauccaggucuacgucgaccaaguggacgaggauauugucgccgucaccaggcauuccccuagcauucaccaguccguggucgcugucuccaggacugcuuuucggaaccccaaaacuuccuucuauagcaaagaggucccucaaauguguauuccugggaagaucgaggaggucgugcuggaggcuaggacuaucgaaaggaauacuaagccuuaccggaaagacgaaaacuccauuaacggcacccccgacauuaccgucgagaucagggagcacauccagcugaacgagagcaagaucgugaagcaagcuggcguggccaccaagggccccaacgaguacauccaagagauugaguucgagaaucugucccccggcagcgugaucauuuuuagggugagccuggacccccacgcccaagucgcugugggcauccugcggaaccaccucacccaauuuagcccucauuucaaguccgggagccucgcuguggauaacgccgacccuauucucaagaucccuuucgcuucccuggccagcaggcucacucuggcugaacucaaccagauucuguaucggugcgaguccgaggagaaagaggacgggggcggcuguuacgauauucccaauugguccgcccugaaguacgccgggcugcaagggcucauguccguccuggccgagauuaggcccaaaaacgaucugggccacccuuucugcaacaaccugagguccggcgacuggaugaucgauuacgucagcaaucggcugaucucccgguccggcacuaucgcugagguggggaaguggcugcaggcuauguuuuuuuaucucaaacagauuccccgguaucugauucccugcuauuucgacgcuauucucaucggggccuacaccacucugcucgacaccgccuggaaacagauguccagcuucgugcagaacggguccaccuucgucaagcaucugucccugggguccgugcaacucugcggcgucggcaaguuuccuagccuccccauccuguccccugcccucauggacgucccuuaccggcucaacgaaauuaccaaggagaaagaacaaugcugcgugucccucgcugccgggcucccucacuucuccuccgggaucuuucgguguuggggccgggacacuuucaucgcccugagggggauucuccucaucacuggccgguacgucgaggcccggaacaucauccucgccuucgcugggacccuccggcacgggcucaucccuaaccuccucggggagggcaucuacgccagguauaacugccgggacgcugucuggugguggcuccagugcauucaggacuauugcaagauggugcccaacgggcucgauauccucaaaugucccgugagcaggauguacccuaccgacgacuccgcuccucugccugcugggacccucgaccagccccuguucgaggucauucaggaggccaugcaaaagcauaugcaggggauucaguuucgggagcggaacgcugggccccagauugaccggaauaugaaagaugagggguucaacauuacugccggcguggacgaggagaccggcuucguguacggcggcaaccgguuuaacugcgggaccuggauggacaagaugggcgagagcgauagggcuaggaauaggggcauucccgccacccccagggacggcuccgcugucgagaucgucgggcucagcaaguccgcugugcgguggcugcucgagcucagcaagaagaacaucuuuccuuaccacgaggucaccgucaagaggcacggcaaagcuauuaaagucuccuacgacgaauggaauaggaagauucaagauaauuucgagaaacucuuccacgugagcgaggauccuuccgaccucaacgagaaacaccccaaccucgugcauaagcgggggauuuauaaggacagcuacggcgcuuccagcccuuggugcgauuaccagcuccggccuaacuucaccauugccaugguggucgccccugaacucuucacuaccgagaaggccuggaaggcucuggaaaucgccgagaagaagcugcuggggccccuggggaugaagacucucgaccccgacgacaugguguauugcggcaucuacgauaacgcccucgauaacgauaauuauaaccuggcuaagggguuuaacuaccaucaaggcccugaauggcucuggccuaucggcuacuuccugcgggccaagcucuacuucagcaggcugauggggcccgaaacuacugccaaaacuauugugcuggugaagaacgugcugagccggcacuacgugcaccuggaaaggagcccuuggaagggccugcccgagcucaccaacgaaaacgcccaguauugcccuuuuagcugcgagacccaagccugguccaucgcuacuauccuggaaacccuguacgaccucuag

SEQ ID NO: 43 - RNA, 4599 nt, Artificial Sequence
  Codon-Optimized AGL Coding Sequence
auggggcacagcaaacaaaucaggauccuccuccucaacgaaauggaaaaacucgaaaaaacccucuucaggcucgaacaaggguacgaacuccaauucaggcucgggccgacgcuccaagggaaagcggugacgguguacacgaacuacccguucccgggggaaacguucaacagggaaaaauucaggagccucgacugggaaaacccgacggaaagggaagacgacagcgacaaauacugcaaacucaaccuccaacaaagcgggagcuuccaauacuacuuccuccaagggaacgaaaaaagcggggggggguacaucgugguggacccgauccucagggugggggcggacaaccacgugcucccgcucgacugcgugacgcuccaaacguuccucgcgaaaugccucgggccguucgacgaaugggaaagcaggcucaggguggcgaaagaaagcggguacaacaugauccacuucacgccgcuccaaacgcucgggcucagcaggagcugcuacagccucgcgaaccaacucgaacucaacccggacuucagcaggccgaacaggaaauacacguggaacgacguggggcaacucguggaaaaacucaaaaaagaauggaacgugaucugcaucacggacgugguguacaaccacacggcggcgaacagcaaauggauccaagaacacccggaaugcgcguacaaccucgugaacagcccgcaccucaaaccggcgugggugcucgacagggcgcucuggagguucagcugcgacguggcggaagggaaauacaaagaaaaagggaucccggcgcucaucgaaaacgaccaccacaugaacagcaucaggaaaaucaucugggaagacaucuucccgaaacucaaacucugggaauucuuccaaguggacgugaacaaagcgguggaacaauucaggaggcuccucacgcaagaaaacaggagggugacgaaaagcgacccgaaccaacaccucacgaucauccaagacccggaauacaggagguucgggugcacgguggacaugaacaucgcgcucacgacguucaucccgcacgacaaagggccggcggcgaucgaagaaugcugcaacugguuccacaaaaggauggaagaacucaacagcgaaaaacacaggcucaucaacuaccaccaagaacaagcggugaacugccuccucgggaacguguucuacgaaaggcucgcggggcacgggccgaaacucgggccggugacgaggaaacacccgcucgugacgagguacuucacguucccguucgaagaaaucgacuucagcauggaagaaagcaugauccaccucccgaacaaagcgugcuuccucauggcgcacaacgggugggugaugggggacgacccgcucaggaacuucgcggaaccggggagcgaaguguaccucaggagggaacucaucugcuggggggacagcgugaaacucagguacgggaacaaaccggaagacugcccguaccucugggcgcacaugaaaaaauacacggaaaucacggcgacguacuuccaaggggugaggcucgacaacugccacagcacgccgcuccacguggcggaauacaugcucgacgcggcgaggaaccuccaaccgaaccucuacgugguggcggaacucuucacggggagcgaagaccucgacaacguguucgugacgaggcucgggaucagcagccucaucagggaagcgaugagcgcguacaacagccacgaagaagggaggcucguguacagguacgggggggaaccgguggggagcuucgugcaaccgugccucaggccgcucaugccggcgaucgcgcacgcgcuguucauggacaucacgcacgacaacgaaugcccgaucgugcacaggagcgcguacgacgcgcucccgagcacgacgaucgugagcauggcgugcugcgcgagcgggagcacgaggggguacgacgaacucgugccgcaccaaaucagcguggugagcgaagaaagguucuacacgaaauggaacccggaagcgcucccgagcaacacgggggaagugaacuuccaaagcgggaucaucgcggcgaggugcgcgaucagcaaacuccaccaagaacucggggcgaaaggguucauccaaguguacguggaccaaguggacgaagacaucguggcggugacgaggcacagcccgagcauccaccaaagcgugguggcggugagcaggacggcguucaggaacccgaaaacgagcuucuacagcaaagaagugccgcaaaugugcaucccggggaaaaucgaagaaguggugcucgaagcgaggacgaucgaaaggaacacgaaaccguacaggaaagacgaaaacagcaucaacgggacgccggacaucacgguggaaaucagggaacacauccaacucaacgaaagcaaaaucgugaaacaagcggggguggcgacgaaagggccgaacgaauacauccaagaaaucgaauucgaaaaccucagcccggggagcgugaucaucuucagggugagccucgacccgcacgcgcaaguggcgguggggauccucaggaaccaccucacgcaauucagcccgcacuucaaaagcgggagccucgcgguggacaacgcggacccgauccucaaaaucccguucgcgagccucgcgagcaggcucacgcucgcggaacucaaccaaauccucuacaggugcgaaagcgaagaaaaagaagacgggggggggugcuacgacaucccgaacuggagcgcgcucaaauacgcggggcuccaagggcucaugagcgugcucgcggaaaucaggccgaaaaacgaccucgggcacccguucugcaacaaccucaggagcggggacuggaugaucgacuacgugagcaacaggcucaucagcaggagcgggacgaucgcggaaguggggaaauggcuccaagcgauguucuucuaccucaaacaaaucccgagguaccucaucccgugcuacuucgacgcgauccucaucggggcguacacgacgcuccucgacacggcguggaaacaaaugagcagcuucgugcaaaacgggagcacguucgugaaacaccucagccucgggagcgugcaacucugcgggguggggaaauucccgagccucccgauccucagcccggcgcucauggacgugccguacaggcucaacgaaaucacgaaagaaaaagaacaaugcugcgugagccucgcggcggggcucccgcacuucagcagcgggaucuucaggugcugggggagggacacguucaucgcgcucagggggauccuccucaucacggggagguacguggaagcgaggaacaucauccucgcguucgcggggacgcucaggcacgggcucaucccgaaccuccucggggaagggaucuacgcgagguacaacugcagggacgcgguguggugguggcuccaaugcauccaagacuacugcaaaauggugccgaacgggcucgacauccucaaaugcccggugagcaggauguacccgacggacgacagcgcgccgcucccggcggggacgcucgaccaaccgcuguucgaagugauccaagaagcgaugcaaaaacacaugcaagggauccaauucagggaaaggaacgcggggccgcaaaucgacaggaacaugaaagacgaaggguucaacaucacggcggggguggacgaagaaacgggguucguguacggggggaacagguucaacugcgggacguggauggacaaaaugggggaaagcgacagggcgaggaacagggggaucccggcgacgccgagggacgggagcgcgguggaaaucguggggcucagcaaaagcgcggugagguggcuccucgaacucagcaaaaaaaacaucuucccguaccacgaagugacggugaaaaggcacgggaaagcgaucaaagugagcuacgacgaauggaacaggaaaauccaagacaacuucgaaaaacucuuccacgugagcgaagacccgagcgaccucaacgaaaaacacccgaaccucgugcacaaaagggggaucuacaaagacagcuacggggcgagcagcccguggugcgacuaccaacucaggccgaacuucacgaucgcgauggugguggcgccggaacucuucacgacggaaaaagcguggaaagcgcucgaaaucgcggaaaaaaaacuccucgggccgcucgggaugaaaacgcucgacccggacgacaugguguacugcgggaucuacgacaacgcgcucgacaacgacaacuacaaccucgcgaaaggguucaacuaccaccaagggccggaauggcucuggccgaucggguacuuccucagggcgaaacucuacuucagcaggcucauggggccggaaacgacggcgaaaacgaucgugcucgugaaaaacgugcucagcaggcacuacgugcaccucgaaaggagcccguggaaagggcucccggaacucacgaacgaaaacgcgcaauacugcccguucagcugcgaaacgcaagcguggagcaucgcgacgauccucgaaacgcucuacgaccucuga

SEQ ID NO: 44 - RNA, 4599 nt, Artificial Sequence
  Codon-Optimized AGL Coding Sequence
augggccacagcaagcagaucaggauccuccuccucaacgaaauggaaaagcucgaaaagacacucuucaggcucgaacagggcuacgaacuccaguucaggcucggcccaacacuccagggcaaggccgugacaguguacacaaacuacccauucccaggcgaaacauucaacagggaaaaguucaggagccucgacugggaaaacccaacagaaagggaagacgacagcgacaaguacugcaagcucaaccuccagcagagcggcagcuuccaguacuacuuccuccagggcaacgaaaagagcggcggcggcuacaucgugguggacccaauccucagggugggcgccgacaaccacgugcucccacucgacugcgugacacuccagacauuccucgccaagugccucggcccauucgacgaaugggaaagcaggcucaggguggccaaggaaagcggcuacaacaugauccacuucacaccacuccagacacucggccucagcaggagcugcuacagccucgccaaccagcucgaacucaacccagacuucagcaggccaaacaggaaguacacauggaacgacgugggccagcucguggaaaagcucaagaaggaauggaacgugaucugcaucacagacgugguguacaaccacacagccgccaacagcaaguggauccaggaacacccagaaugcgccuacaaccucgugaacagcccacaccucaagccagccugggugcucgacagggcccucuggagguucagcugcgacguggccgaaggcaaguacaaggaaaagggcaucccagcccucaucgaaaacgaccaccacaugaacagcaucaggaagaucaucugggaagacaucuucccaaagcucaagcucugggaauucuuccagguggacgugaacaaggccguggaacaguucaggaggcuccucacacaggaaaacaggagggugacaaagagcgacccaaaccagcaccucacaaucauccaggacccagaauacaggagguucggcugcacaguggacaugaacaucgcccucacaacauucaucccacacgacaagggcccagccgccaucgaagaaugcugcaacugguuccacaagaggauggaagaacucaacagcgaaaagcacaggcucaucaacuaccaccaggaacaggccgugaacugccuccucggcaacguguucuacgaaaggcucgccggccacggcccaaagcucggcccagugacaaggaagcacccacucgugacaagguacuucacauucccauucgaagaaaucgacuucagcauggaagaaagcaugauccaccucccaaacaaggccugcuuccucauggcccacaacggcugggugaugggcgacgacccacucaggaacuucgccgaaccaggcagcgaaguguaccucaggagggaacucaucugcuggggcgacagcgugaagcucagguacggcaacaagccagaagacugcccauaccucugggcccacaugaagaaguacacagaaaucacagccacauacuuccagggcgugaggcucgacaacugccacagcacaccacuccacguggccgaauacaugcucgacgccgccaggaaccuccagccaaaccucuacgugguggccgaacucuucacaggcagcgaagaccucgacaacguguucgugacaaggcucggcaucagcagccucaucagggaagccaugagcgccuacaacagccacgaagaaggcaggcucguguacagguacggcggcgaaccagugggcagcuucgugcagccaugccucaggccacucaugccagccaucgcccacgcccucuucauggacaucacacacgacaacgaaugcccaaucgugcacaggagcgccuacgacgcccucccaagcacaacaaucgugagcauggccugcugcgccagcggcagcacaaggggcuacgacgaacucgugccacaccagaucagcguggugagcgaagaaagguucuacacaaaguggaacccagaagcccucccaagcaacacaggcgaagugaacuuccagagcggcaucaucgccgccaggugcgccaucagcaagcuccaccaggaacucggcgccaagggcuucauccagguguacguggaccagguggacgaagacaucguggccgugacaaggcacagcccaagcauccaccagagcgugguggccgugagcaggacagccuucaggaacccaaagacaagcuucuacagcaaggaagugccacagaugugcaucccaggcaagaucgaagaaguggugcucgaagccaggacaaucgaaaggaacacaaagccauacaggaaggacgaaaacagcaucaacggcacaccagacaucacaguggaaaucagggaacacauccagcucaacgaaagcaagaucgugaagcaggccggcguggccacaaagggcccaaacgaauacauccaggaaaucgaauucgaaaaccucagcccaggcagcgugaucaucuucagggugagccucgacccacacgcccagguggccgugggcauccucaggaaccaccucacacaguucagcccacacuucaagagcggcagccucgccguggacaacgccgacccaauccucaagaucccauucgccagccucgccagcaggcucacacucgccgaacucaaccagauccucuacaggugcgaaagcgaagaaaaggaagacggcggcggcugcuacgacaucccaaacuggagcgcccucaaguacgccggccuccagggccucaugagcgugcucgccgaaaucaggccaaagaacgaccucggccacccauucugcaacaaccucaggagcggcgacuggaugaucgacuacgugagcaacaggcucaucagcaggagcggcacaaucgccgaagugggcaaguggcuccaggccauguucuucuaccucaagcagaucccaagguaccucaucccaugcuacuucgacgccauccucaucggcgccuacacaacacuccucgacacagccuggaagcagaugagcagcuucgugcagaacggcagcacauucgugaagcaccucagccucggcagcgugcagcucugcggcgugggcaaguucccaagccucccaauccucagcccagcccucauggacgugccauacaggcucaacgaaaucacaaaggaaaaggaacagugcugcgugagccucgccgccggccucccacacuucagcagcggcaucuucaggugcuggggcagggacacauucaucgcccucaggggcauccuccucaucacaggcagguacguggaagccaggaacaucauccucgccuucgccggcacacucaggcacggccucaucccaaaccuccucggcgaaggcaucuacgccagguacaacugcagggacgccguguggugguggcuccagugcauccaggacuacugcaagauggugccaaacggccucgacauccucaagugcccagugagcaggauguacccaacagacgacagcgccccacucccagccggcacacucgaccagccacucuucgaagugauccaggaagccaugcagaagcacaugcagggcauccaguucagggaaaggaacgccggcccacagaucgacaggaacaugaaggacgaaggcuucaacaucacagccggcguggacgaagaaacaggcuucguguacggcggcaacagguucaacugcggcacauggauggacaagaugggcgaaagcgacagggccaggaacaggggcaucccagccacaccaagggacggcagcgccguggaaaucgugggccucagcaagagcgccgugagguggcuccucgaacucagcaagaagaacaucuucccauaccacgaagugacagugaagaggcacggcaaggccaucaaggugagcuacgacgaauggaacaggaagauccaggacaacuucgaaaagcuguuccacgugagcgaagacccaagcgaccucaacgaaaagcacccaaaccucgugcacaagaggggcaucuacaaggacagcuacggcgccagcagcccauggugcgacuaccagcucaggccaaacuucacaaucgccauggugguggccccagaacucuucacaacagaaaaggccuggaaggcccucgaaaucgccgaaaagaagcuccucggcccacucggcaugaagacacucgacccagacgacaugguguacugcggcaucuacgacaacgcccucgacaacgacaacuacaaccucgccaagggcuucaacuaccaccagggcccagaauggcucuggccaaucggcuacuuccucagggccaagcucuacuucagcaggcucaugggcccagaaacaacagccaagacaaucgugcucgugaagaacgugcucagcaggcacuacgugcaccucgaaaggagcccauggaagggccucccagaacucacaaacgaaaacgcccaguacugcccauucagcugcgaaacacaggccuggagcaucgccacaauccucgaaacacucuacgaccucuga

SEQ ID NO: 45 - RNA, 4599 nt, Artificial Sequence
  Codon-Optimized AGL Coding Sequence
augggccacagcaagcagauccggaucuugcugcugaacgagauggagaagcuggagaagacccuguucaggcuggagcagggcuacgagcugcaguuccgguugggccccaccuugcagggcaaggccgugaccguguacaccaacuaccccuuccccggcgagacguucaacagggagaaguuccggucccuggacugggagaaccccaccgagagggaggacgacuccgacaaguacugcaagcugaaccugcagcaguccggcuccuuccaguacuacuuccugcagggcaacgagaagaguggcggcggcuacaucgugguggaccccaucuugcgggugggcgccgacaaccacgugcugcccuuggacugcgugacccugcagaccuucuuggccaagugcuugggccccuucgacgagugggagagcaggcugaggguggccaaggaguccggcuacaacaugauccacuucacccccuugcagacccugggccuguccagguccugcuacucccuggccaaccaguuggaguugaaccccgacuucuccaggcccaacaggaaguacaccuggaacgacgugggccagcugguggagaaguugaagaaggaguggaacgugaucugcaucaccgacgugguguacaaccacaccgccgccaacagcaaguggauccaggagcaccccgagugcgccuacaaccuggugaacuccccccacuugaagcccgccuggguguuggacagggcccuguggcgguucuccugcgacguggccgagggcaaguacaaggagaagggcauccccgccuugaucgagaacgaccaccacaugaacuccauccggaagaucaucugggaggacaucuuccccaagcugaagcugugggaguucuuccagguggacgugaacaaggccguggagcaguucaggaggcugcugacccaggagaacaggcgggugaccaaguccgaccccaaccagcaccugaccaucauccaggaccccgaguacaggcgguucggcugcaccguggacaugaacaucgcccugaccaccuucaucccccacgacaagggccccgccgccaucgaggagugcugcaacugguuccacaagaggauggaggaguugaacuccgagaagcaccggcugaucaacuaccaccaggagcaggccgugaacugccuguugggcaacguguucuacgagcggcuggccggccacggccccaagcugggccccgugaccaggaagcaccccuuggugaccagguacuucaccuuccccuucgaggagaucgacuucuccauggaggaguccaugauccaccugcccaacaaggccugcuuccugauggcccacaacggcugggugaugggcgacgacccccugcggaacuucgccgagcccggcuccgagguguaccugaggagggagcugaucugcuggggcgacagcgugaaguugcgguacggcaacaagcccgaggacugccccuaccugugggcccacaugaagaaguacaccgagaucaccgccaccuacuuccagggcgugcggcuggacaacugccacuccaccccccugcacguggccgaguacauguuggacgccgccaggaacuugcagcccaacuuguacgugguggccgagcuguucaccggcagcgaggaccuggacaacguguucgugaccaggcugggcaucagcuccuugaucagggaggccaugagcgccuacaacagccacgaggagggcagguugguguaccgguacggcggcgagcccgugggcuccuucgugcagcccugcuugaggcccuugaugcccgccaucgcccacgcccuguucauggacaucacccacgacaacgagugccccaucgugcacagguccgccuacgacgcccugcccagcaccaccaucguguccauggccugcugcgccagcggcagcaccaggggcuacgacgaguuggugccccaccagaucuccgugguguccgaggagcgguucuacaccaaguggaaccccgaggccuugcccuccaacaccggcgaggugaacuuccagagcggcaucaucgccgccaggugcgccaucagcaagcugcaccaggagcugggcgccaagggcuucauccagguguacguggaccagguggacgaggacaucguggccgugaccaggcacucccccagcauccaccaguccgugguggccguguccaggaccgccuucaggaaccccaagaccuccuucuacagcaaggaggugccccagaugugcauccccggcaagaucgaggagguggugcuggaggccaggaccaucgagaggaacaccaagcccuacaggaaggacgagaacuccaucaacggcacccccgacaucaccguggagaucagggagcacauccagcugaacgagagcaagaucgugaagcaggccggcguggccaccaagggccccaacgaguacauccaggagaucgaguucgagaacuugucccccggcagcgugaucaucuucagggugagccuggacccccacgcccagguggccgugggcauccugcggaaccaccugacccaguucagcccccacuucaaguccggcagccuggccguggacaacgccgaccccaucuugaagauccccuucgccucccuggccuccagguugaccuuggccgagcugaaccagauccuguaccggugcgaguccgaggagaaggaggacggcggcggcugcuacgacauccccaacugguccgcccugaaguacgccggccugcagggcuugauguccguguuggccgagaucaggcccaagaacgacuugggccaccccuucugcaacaacuugagguccggcgacuggaugaucgacuacgugagcaaccggcugaucucccgguccggcaccaucgccgaggugggcaagugguugcaggccauguucuucuaccugaagcagaucccccgguaccugauccccugcuacuucgacgccaucuugaucggcgccuacaccacccugcuggacaccgccuggaagcagauguccagcuucgugcagaacggcuccaccuucgugaagcaccuguccuugggcuccgugcagcugugcggcgugggcaaguuccccucccugcccauccugucccccgcccugauggacgugcccuacagguugaacgagaucaccaaggagaaggagcagugcugcgugucccuggccgccggcuugccccacuucuccuccggcaucuuccggugcuggggcagggacaccuucaucgcccugaggggcauccugcugaucaccggccgguacguggaggccaggaacaucaucuuggccuucgccggcacccugaggcacggccugauccccaaccugcugggcgagggcaucuacgccagguacaacugccgggacgccguguggugguggcugcagugcauccaggacuacugcaagauggugcccaacggccuggacauccugaagugccccguguccaggauguaccccaccgacgacuccgcccccuugcccgccggcacccuggaccagcccuuguucgaggugauccaggaggccaugcagaagcacaugcagggcauccaguuccgggagaggaacgccggcccccagaucgaccggaacaugaaggacgagggcuucaacaucaccgccggcguggacgaggagacuggcuucguguacggcggcaaccgguucaacugcggcaccuggauggacaagaugggcgagagcgacagggccaggaacaggggcauccccgccacccccagggacggcuccgccguggagaucgugggccugagcaaguccgccgugcggugguugcuggaguuguccaagaagaacaucuuccccuaccacgaggugaccgugaagaggcacggcaaggccaucaagguguccuacgacgaguggaacaggaagauccaggacaacuucgagaagcuguuccacguguccgaggaccccuccgacuugaacgagaagcaccccaaccuggugcacaagcggggcaucuacaaggacagcuacggcgccuccagccccuggugcgacuaccagcugaggcccaacuucaccaucgccauggugguggcccccgagcuguucaccaccgagaaggccuggaaggccuuggagaucgccgagaagaaguugcugggcccccugggcaugaagaccuuggaccccgacgacaugguguacugcggcaucuacgacaacgccuuggacaacgacaacuacaaccuggccaagggcuucaacuaccaccagggccccgaguggcuguggcccaucggcuacuuccugcgggccaaguuguacuucuccagguugaugggccccgagacgaccgccaagaccaucguguuggugaagaacgugcugucccggcacuacgugcaccuggagaggucccccuggaagggccugcccgagcugaccaacgagaacgcccaguacugccccuucagcugcgagacgcaggccugguccaucgccaccauccuggagacgcuguacgacuuguag